European Patent Application EP 4 477 665 A1, published December 18, 2024. Title: Stefin A protein variants specifically binding to CD40L, and uses thereof. Applicant: AffyXell Therapeutics Co., Ltd. Application KR. The sequence listing filed with the application follows.

SEQUENCE LISTING (730 sequences)

SEQ ID NO: 1 - protein, 48 aa, Artificial Sequence
  VARIANT 48: note = X can be any amino acid
MIPGGLSEAKPATPEIQEIVDKVKPQLEEKTGETYGKLEAVQYKTQVX

SEQ ID NO: 2 - protein, 24 aa, Artificial Sequence
GTNYYIKVRAGDNKYMHLKVFKSL

SEQ ID NO: 3 - protein, 21 aa, Artificial Sequence
EDLVLTGYQVDKNKDDELTGF

SEQ ID NO: 4 - protein, 95 aa, Artificial Sequence
  source 1..95: note = X individually can be any amino acid
  VARIANT 4
  VARIANT 49: note = The amino acid 'X' at residue 49 can be repeated one or more times
  VARIANT 50
  VARIANT 71..73
  VARIANT 74: note = The amino acid 'X' at residue 74 can be repeated one or more times
  VARIANT 75
  VARIANT 77
MIPXGLSEAKPATPEIQEIVDKVKPQLEEKTGETYGKLEAVQYKTQVVXXTNYYIKVRAGDNKYMHLKVFXXXXXDXVLTGYQVDKNKDDELTGF

SEQ ID NO: 5 - protein, 95 aa, Artificial Sequence
  source 1..95: note = X individually can be any amino acid
  VARIANT 49: note = The amino acid 'X' at residue 49 can be repeated one or more times
  VARIANT 74: note = The amino acid 'X' at residue 74 can be individually repeated one or more times
MIPGGLSEAKPATPEIQEIVDKVKPQLEEKTGETYGKLEAVQYKTQVDXGTNYYIKVRAGDNKYMHLKVFKSLXEDLVLTGYQVDKNKDDELTGF

SEQ ID NO: 6 - protein, 9 aa, Artificial Sequence
HDVFYDQKA

SEQ ID NO: 7 - protein, 9 aa, Artificial Sequence
PFKIITVWH

SEQ ID NO: 8 - protein, 9 aa, Artificial Sequence
QYKIITWWS

SEQ ID NO: 9 - protein, 9 aa, Artificial Sequence
HYYVHYNDQ

SEQ ID NO: 10 - protein, 9 aa, Artificial Sequence
YYQIITWWQ

SEQ ID NO: 11 - protein, 9 aa, Artificial Sequence
VHGPHLEQA

SEQ ID NO: 12 - protein, 9 aa, Artificial Sequence
LQDQWPWRD

SEQ ID NO: 13 - skipped

SEQ ID NO: 14 - protein, 9 aa, Artificial Sequence
SWVKPDNEL

SEQ ID NO: 15 - protein, 9 aa, Artificial Sequence
NSLGVSEWV

SEQ ID NO: 16 - protein, 9 aa, Artificial Sequence
VYRIVSWWR

SEQ ID NO: 17 - protein, 9 aa, Artificial Sequence
YYRQLKFNT

SEQ ID NO: 18 - protein, 9 aa, Artificial Sequence
GWIKVDNVL

SEQ ID NO: 19 - protein, 9 aa, Artificial Sequence
TAYYIHVNA

SEQ ID NO: 20 - protein, 9 aa, Artificial Sequence
VRVEPTPND

SEQ ID NO: 21 - protein, 9 aa, Artificial Sequence
DLNSSVWYQ

SEQ ID NO: 22 - protein, 9 aa, Artificial Sequence
FTYQISYTV

SEQ ID NO: 23 - protein, 9 aa, Artificial Sequence
RENWYGEFA

SEQ ID NO: 24 - protein, 9 aa, Artificial Sequence
TALAWNTQA

SEQ ID NO: 25 - protein, 9 aa, Artificial Sequence
HIPALKVHA

SEQ ID NO: 26 - protein, 9 aa, Artificial Sequence
HHAYAAVYV

SEQ ID NO: 27 - protein, 9 aa, Artificial Sequence
YDELYHEKA

SEQ ID NO: 28 - protein, 9 aa, Artificial Sequence
SWYYPKNVL

SEQ ID NO: 29 - protein, 9 aa, Artificial Sequence
FLEWHFWEW

SEQ ID NO: 30 - protein, 9 aa, Artificial Sequence
SWVRGTNQL

SEQ ID NO: 31 - protein, 9 aa, Artificial Sequence
WRKLLSWWK

SEQ ID NO: 32 - protein, 9 aa, Artificial Sequence
PKSHQTNEQ

SEQ ID NO: 33 - protein, 9 aa, Artificial Sequence
NWNQIDNPL

SEQ ID NO: 34 - protein, 9 aa, Artificial Sequence
FWVGLHNQL

SEQ ID NO: 35 - protein, 9 aa, Artificial Sequence
FTQPFNEPI

SEQ ID NO: 36 - protein, 9 aa, Artificial Sequence
PEYQPQPKA

SEQ ID NO: 37 - protein, 9 aa, Artificial Sequence
NDPYFQSFS

SEQ ID NO: 38 - protein, 9 aa, Artificial Sequence
HQDDVAWQS

SEQ ID NO: 39 - protein, 9 aa, Artificial Sequence
KGYFHTVEA

SEQ ID NO: 40 - protein, 9 aa, Artificial Sequence
VDQVWSENA

SEQ ID NO: 41 - protein, 9 aa, Artificial Sequence
LSSIWQDVA

SEQ ID NO: 42 - protein, 9 aa, Artificial Sequence
TASLYWNYA

SEQ ID NO: 43 - protein, 9 aa, Artificial Sequence
SWKQWHNYL

SEQ ID NO: 44 - protein, 9 aa, Artificial Sequence
QVHLDNSPL

SEQ ID NO: 45 - protein, 9 aa, Artificial Sequence
QNNWYLSNY

SEQ ID NO: 46 - protein, 9 aa, Artificial Sequence
WEWALLLEY

SEQ ID NO: 47 - protein, 9 aa, Artificial Sequence
GDSYWEYVS

SEQ ID NO: 48 - protein, 9 aa, Artificial Sequence
GQKWWQHKI

SEQ ID NO: 49 - protein, 9 aa, Artificial Sequence
LDGLYHVNS

SEQ ID NO: 50 - protein, 9 aa, Artificial Sequence
HAPAPVQAI

SEQ ID NO: 51 - protein, 9 aa, Artificial Sequence
WEDHWNYQY

SEQ ID NO: 52 - protein, 9 aa, Artificial Sequence
SWRYKSNQL

SEQ ID NO: 53 - protein, 9 aa, Artificial Sequence
RVDWWLPEV

SEQ ID NO: 54 - protein, 9 aa, Artificial Sequence
SWIEISNQL

SEQ ID NO: 55 - protein, 9 aa, Artificial Sequence
SLGQAETWA

SEQ ID NO: 56 - protein, 9 aa, Artificial Sequence
KIGQLPSRV

SEQ ID NO: 57 - protein, 9 aa, Artificial Sequence
AWHTKNNSI

SEQ ID NO: 58 - protein, 9 aa, Artificial Sequence
QTKLVTWWW

SEQ ID NO: 59 - protein, 9 aa, Artificial Sequence
AVFDYADPS

SEQ ID NO: 60 - protein, 9 aa, Artificial Sequence
HVKIVTWWK

SEQ ID NO: 61 - protein, 9 aa, Artificial Sequence
HVLKVSSVS

SEQ ID NO: 62 - protein, 9 aa, Artificial Sequence
YQDYDSATH

SEQ ID NO: 63 - protein, 9 aa, Artificial Sequence
SWGKVSNEL

SEQ ID NO: 64 - protein, 9 aa, Artificial Sequence
LEDEWWSIL

SEQ ID NO: 65 - protein, 9 aa, Artificial Sequence
YYKLVTWWR

SEQ ID NO: 66 - protein, 9 aa, Artificial Sequence
AWVKEHNLI

SEQ ID NO: 67 - protein, 9 aa, Artificial Sequence
QEYLWKQYI

SEQ ID NO: 68 - protein, 9 aa, Artificial Sequence
FNKDLFLGW

SEQ ID NO: 69 - protein, 9 aa, Artificial Sequence
HFGIRYAHV

SEQ ID NO: 70 - protein, 9 aa, Artificial Sequence
WYAWQEGWQ

SEQ ID NO: 71 - protein, 9 aa, Artificial Sequence
GNAAWGSFA

SEQ ID NO: 72 - protein, 9 aa, Artificial Sequence
REDLDLFYT

SEQ ID NO: 73 - protein, 9 aa, Artificial Sequence
NENVYRVTQ

SEQ ID NO: 74 - protein, 9 aa, Artificial Sequence
WHKIVTQWP

SEQ ID NO: 75 - protein, 9 aa, Artificial Sequence
HYRIITHWE

SEQ ID NO: 76 - protein, 9 aa, Artificial Sequence
LVFDASTSA

SEQ ID NO: 77 - protein, 9 aa, Artificial Sequence
QYAEFLEHI

SEQ ID NO: 78 - protein, 9 aa, Artificial Sequence
GNVQEDWHI

SEQ ID NO: 79 - protein, 9 aa, Artificial Sequence
GWSASYPES

SEQ ID NO: 80 - protein, 9 aa, Artificial Sequence
YQFEHISYG

SEQ ID NO: 81 - protein, 9 aa, Artificial Sequence
AWITPVNVL

SEQ ID NO: 82 - protein, 9 aa, Artificial Sequence
ESYAAIFWG

SEQ ID NO: 83 - protein, 9 aa, Artificial Sequence
RVWPWTWDR

SEQ ID NO: 84 - protein, 10 aa, Artificial Sequence
QVKKWWEYFV

SEQ ID NO: 85 - protein, 9 aa, Artificial Sequence
IGQISEQQW

SEQ ID NO: 86 - protein, 9 aa, Artificial Sequence
AFHKLGWIL

SEQ ID NO: 87 - protein, 9 aa, Artificial Sequence
FKKWWWKYK

SEQ ID NO: 88 - protein, 9 aa, Artificial Sequence
ASQRLWIIY

SEQ ID NO: 89 - protein, 9 aa, Artificial Sequence
QRETHILWS

SEQ ID NO: 90 - protein, 9 aa, Artificial Sequence
GQYWFWAPG

SEQ ID NO: 91 - protein, 9 aa, Artificial Sequence
RDWAYYIYF

SEQ ID NO: 92 - protein, 9 aa, Artificial Sequence
IGYKLNYIW

SEQ ID NO: 93 - protein, 9 aa, Artificial Sequence
VSLTEQRWK

SEQ ID NO: 94 - protein, 9 aa, Artificial Sequence
WVSQQHYSH

SEQ ID NO: 95 - protein, 9 aa, Artificial Sequence
DDDNQHYGL

SEQ ID NO: 96 - protein, 9 aa, Artificial Sequence
PTRWISIYW

SEQ ID NO: 97 - protein, 9 aa, Artificial Sequence
TAFAPNKAS

SEQ ID NO: 98 - protein, 9 aa, Artificial Sequence
HYTDFKWHK

SEQ ID NO: 99 - protein, 9 aa, Artificial Sequence
NKFWSWAPG

SEQ ID NO: 100 - protein, 9 aa, Artificial Sequence
ELDEPAWDW

SEQ ID NO: 101 - protein, 9 aa, Artificial Sequence
HEKWGFWEL

SEQ ID NO: 102 - protein, 9 aa, Artificial Sequence
VATADLIKA

SEQ ID NO: 103 - protein, 9 aa, Artificial Sequence
YYKVISWWH

SEQ ID NO: 104 - protein, 9 aa, Artificial Sequence
HWHHYDNII

SEQ ID NO: 105 - protein, 9 aa, Artificial Sequence
VYKIITFWS

SEQ ID NO: 106 - protein, 9 aa, Artificial Sequence
GWIQRHNLI

SEQ ID NO: 107 - protein, 9 aa, Artificial Sequence
KTWEDTVVA

SEQ ID NO: 108 - protein, 9 aa, Artificial Sequence
LDQHHVYQV

SEQ ID NO: 109 - protein, 9 aa, Artificial Sequence
LEDVWGVWA

SEQ ID NO: 110 - protein, 9 aa, Artificial Sequence
WLPWTVELI

SEQ ID NO: 111 - protein, 9 aa, Artificial Sequence
QHFTWDWFW

SEQ ID NO: 112 - protein, 9 aa, Artificial Sequence
LFEVLQGSS

SEQ ID NO: 113 - protein, 9 aa, Artificial Sequence
PYSWQHEVV

SEQ ID NO: 114 - protein, 9 aa, Artificial Sequence
WWQENAEWI

SEQ ID NO: 115 - protein, 9 aa, Artificial Sequence
SYDPVYQDT

SEQ ID NO: 116 - protein, 9 aa, Artificial Sequence
RVFDTPLAA

SEQ ID NO: 117 - protein, 9 aa, Artificial Sequence
WWDIPWIWV

SEQ ID NO: 118 - protein, 9 aa, Artificial Sequence
YQKVITWWQ

SEQ ID NO: 119 - protein, 9 aa, Artificial Sequence
QWIKWGNIL

SEQ ID NO: 120 - protein, 9 aa, Artificial Sequence
ATPEKKYVV

SEQ ID NO: 121 - protein, 9 aa, Artificial Sequence
TSERLWILY

SEQ ID NO: 122 - protein, 9 aa, Artificial Sequence
EHHSQPLAH

SEQ ID NO: 123 - protein, 9 aa, Artificial Sequence
WTADWLWTV

SEQ ID NO: 124 - protein, 9 aa, Artificial Sequence
SFQREHYSW

SEQ ID NO: 125 - protein, 9 aa, Artificial Sequence
GKTWHKHNR

SEQ ID NO: 126 - protein, 9 aa, Artificial Sequence
KWWYRIGNP

SEQ ID NO: 127 - protein, 9 aa, Artificial Sequence
LERFNFHGE

SEQ ID NO: 128 - protein, 9 aa, Artificial Sequence
VYKNKRGGH

SEQ ID NO: 129 - protein, 9 aa, Artificial Sequence
WGENLFAKW

SEQ ID NO: 130 - protein, 9 aa, Artificial Sequence
GIRKKQQQR

SEQ ID NO: 131 - protein, 9 aa, Artificial Sequence
GHAFYFAFV

SEQ ID NO: 132 - protein, 9 aa, Artificial Sequence
TYGKKWYSW

SEQ ID NO: 133 - protein, 9 aa, Artificial Sequence
YFYRHWEDR

SEQ ID NO: 134 - protein, 9 aa, Artificial Sequence
WQVHDKQWL

SEQ ID NO: 135 - protein, 9 aa, Artificial Sequence
PYWYRKNNL

SEQ ID NO: 136 - protein, 9 aa, Artificial Sequence
ASDIYLRID

SEQ ID NO: 137 - protein, 9 aa, Artificial Sequence
FLHRKPQDR

SEQ ID NO: 138 - protein, 9 aa, Artificial Sequence
WQDHHNVKR

SEQ ID NO: 139 - protein, 9 aa, Artificial Sequence
PYGYRAKAP

SEQ ID NO: 140 - protein, 9 aa, Artificial Sequence
PLVQELWGF

SEQ ID NO: 141 - protein, 9 aa, Artificial Sequence
YWLLEIEHR

SEQ ID NO: 142 - protein, 9 aa, Artificial Sequence
RWRYPARKP

SEQ ID NO: 143 - protein, 9 aa, Artificial Sequence
LYIYRHPNY

SEQ ID NO: 144 - protein, 9 aa, Artificial Sequence
PWLYRQKSD

SEQ ID NO: 145 - protein, 9 aa, Artificial Sequence
PYWYRHDQE

SEQ ID NO: 146 - protein, 9 aa, Artificial Sequence
PYWYRKYPD

SEQ ID NO: 147 - protein, 8 aa, Artificial Sequence
EYKFRNLE

SEQ ID NO: 148 - protein, 9 aa, Artificial Sequence
EDFIAADDD

SEQ ID NO: 149 - protein, 9 aa, Artificial Sequence
DSQEFPSHL

SEQ ID NO: 150 - protein, 9 aa, Artificial Sequence
EPDWPDFLI

SEQ ID NO: 151 - protein, 9 aa, Artificial Sequence
ILNPKSWNF

SEQ ID NO: 152 - protein, 9 aa, Artificial Sequence
WNENHFSVW

SEQ ID NO: 153 - protein, 9 aa, Artificial Sequence
NKDWEDQII

SEQ ID NO: 154 - protein, 9 aa, Artificial Sequence
YYNGDNTQI

SEQ ID NO: 155 - protein, 9 aa, Artificial Sequence
YWDDKVGYY

SEQ ID NO: 156 - protein, 9 aa, Artificial Sequence
FHFRKPQDR

SEQ ID NO: 157 - protein, 9 aa, Artificial Sequence
PYWYREPEN

SEQ ID NO: 158 - protein, 9 aa, Artificial Sequence
EYGWYHLPY

SEQ ID NO: 159 - protein, 9 aa, Artificial Sequence
TYHFRTDLN

SEQ ID NO: 160 - protein, 9 aa, Artificial Sequence
PYLWRKHAV

SEQ ID NO: 161 - protein, 9 aa, Artificial Sequence
LYQFRKEPV

SEQ ID NO: 162 - protein, 9 aa, Artificial Sequence
FYYRGPQPV

SEQ ID NO: 163 - protein, 9 aa, Artificial Sequence
YPDGDLILY

SEQ ID NO: 164 - protein, 9 aa, Artificial Sequence
QFGEIIWWE

SEQ ID NO: 165 - protein, 9 aa, Artificial Sequence
VEERWGLWV

SEQ ID NO: 166 - protein, 9 aa, Artificial Sequence
HHPWQPAKQ

SEQ ID NO: 167 - protein, 9 aa, Artificial Sequence
PYRWRPDHA

SEQ ID NO: 168 - protein, 9 aa, Artificial Sequence
HSNAWNLQH

SEQ ID NO: 169 - protein, 9 aa, Artificial Sequence
FYYYRSEPT

SEQ ID NO: 170 - protein, 9 aa, Artificial Sequence
PYWYRPNRP

SEQ ID NO: 171 - protein, 9 aa, Artificial Sequence
ELYSNQIVW

SEQ ID NO: 172 - protein, 9 aa, Artificial Sequence
YKDWVVNPP

SEQ ID NO: 173 - protein, 9 aa, Artificial Sequence
PYQYRKDPK

SEQ ID NO: 174 - protein, 9 aa, Artificial Sequence
YYGNTSILI

SEQ ID NO: 175 - protein, 9 aa, Artificial Sequence
FKYRHQQDK

SEQ ID NO: 176 - protein, 9 aa, Artificial Sequence
YWYRNPADR

SEQ ID NO: 177 - protein, 9 aa, Artificial Sequence
ETKLAHEDI

SEQ ID NO: 178 - protein, 9 aa, Artificial Sequence
LGEQYIDVD

SEQ ID NO: 179 - protein, 9 aa, Artificial Sequence
PYRYRTHHK

SEQ ID NO: 180 - protein, 9 aa, Artificial Sequence
YNPKPGIDN

SEQ ID NO: 181 - protein, 9 aa, Artificial Sequence
FYYRKRYDR

SEQ ID NO: 182 - protein, 9 aa, Artificial Sequence
YQYRNPIDK

SEQ ID NO: 183 - protein, 9 aa, Artificial Sequence
IEYQSPALY

SEQ ID NO: 184 - protein, 9 aa, Artificial Sequence
PDAPAYSKS

SEQ ID NO: 185 - protein, 9 aa, Artificial Sequence
PDLNYEVTL

SEQ ID NO: 186 - protein, 9 aa, Artificial Sequence
YDQNQWSPH

SEQ ID NO: 187 - protein, 9 aa, Artificial Sequence
RWQYRHPQT

SEQ ID NO: 188 - protein, 9 aa, Artificial Sequence
RFSAGEEWE

SEQ ID NO: 189 - protein, 9 aa, Artificial Sequence
DYPRHHQDQ

SEQ ID NO: 190 - protein, 9 aa, Artificial Sequence
FRKKWAQLW

SEQ ID NO: 191 - protein, 9 aa, Artificial Sequence
PFFYRKDNP

SEQ ID NO: 192 - protein, 9 aa, Artificial Sequence
EFILQPWWY

SEQ ID NO: 193 - protein, 9 aa, Artificial Sequence
KYRHRLTYE

SEQ ID NO: 194 - protein, 9 aa, Artificial Sequence
YAQRGEVYF

SEQ ID NO: 195 - protein, 9 aa, Artificial Sequence
VRAFLYYKD

SEQ ID NO: 196 - protein, 9 aa, Artificial Sequence
PWEFRGDHK

SEQ ID NO: 197 - protein, 9 aa, Artificial Sequence
GWSHYFQYL

SEQ ID NO: 198 - protein, 9 aa, Artificial Sequence
FSEDLTLNG

SEQ ID NO: 199 - protein, 9 aa, Artificial Sequence
TQWEFIEWP

SEQ ID NO: 200 - protein, 9 aa, Artificial Sequence
FTYRLPQHR

SEQ ID NO: 201 - protein, 9 aa, Artificial Sequence
DEIFHGAYN

SEQ ID NO: 202 - protein, 9 aa, Artificial Sequence
WGEIQHWRQ

SEQ ID NO: 203 - protein, 9 aa, Artificial Sequence
EQWLPNPYF

SEQ ID NO: 204 - protein, 9 aa, Artificial Sequence
QLLSHQWTE

SEQ ID NO: 205 - protein, 9 aa, Artificial Sequence
HRYWTRDVT

SEQ ID NO: 206 - protein, 9 aa, Artificial Sequence
GDESHKWHK

SEQ ID NO: 207 - protein, 9 aa, Artificial Sequence
RVDEHYIQF

SEQ ID NO: 208 - protein, 9 aa, Artificial Sequence
SDWRHHGGW

SEQ ID NO: 209 - protein, 9 aa, Artificial Sequence
WFDNLHNNF

SEQ ID NO: 210 - protein, 9 aa, Artificial Sequence
PSSGGGPKW

SEQ ID NO: 211 - protein, 9 aa, Artificial Sequence
RSDTLHYWN

SEQ ID NO: 212 - protein, 9 aa, Artificial Sequence
IQYRWQDRV

SEQ ID NO: 213 - protein, 9 aa, Artificial Sequence
FQPIKLANA

SEQ ID NO: 214 - protein, 9 aa, Artificial Sequence
FAFRKYEDR

SEQ ID NO: 215 - protein, 9 aa, Artificial Sequence
LHNWWKGNW

SEQ ID NO: 216 - protein, 9 aa, Artificial Sequence
LNRYYHASI

SEQ ID NO: 217 - protein, 9 aa, Artificial Sequence
RYWAFRYLW

SEQ ID NO: 218 - protein, 9 aa, Artificial Sequence
PFWANEHGW

SEQ ID NO: 219 - protein, 9 aa, Artificial Sequence
ADSGFNATP

SEQ ID NO: 220 - protein, 9 aa, Artificial Sequence
RQHKKPHPN

SEQ ID NO: 221 - protein, 9 aa, Artificial Sequence
HSHRFHEAH

SEQ ID NO: 222 - protein, 9 aa, Artificial Sequence
PWHYPPNKW

SEQ ID NO: 223 - protein, 9 aa, Artificial Sequence
YKTPFPQYT

SEQ ID NO: 224 - protein, 9 aa, Artificial Sequence
YQLVDLDLD

SEQ ID NO: 225 - protein, 9 aa, Artificial Sequence
EYPPVQQVL

SEQ ID NO: 226 - protein, 9 aa, Artificial Sequence
YSEPPPVQN

SEQ ID NO: 227 - protein, 9 aa, Artificial Sequence
EYLYRPLNP

SEQ ID NO: 228 - protein, 9 aa, Artificial Sequence
ALLIHHDPW

SEQ ID NO: 229 - protein, 9 aa, Artificial Sequence
EFQHRTFNH

SEQ ID NO: 230 - protein, 9 aa, Artificial Sequence
GEIWSAKHK

SEQ ID NO: 231 - protein, 9 aa, Artificial Sequence
PEYKPVDHT

SEQ ID NO: 232 - protein, 9 aa, Artificial Sequence
GEIVWYQVE

SEQ ID NO: 233 - protein, 10 aa, Artificial Sequence
IVFYLQEYYE

SEQ ID NO: 234 - protein, 9 aa, Artificial Sequence
GYAVFHKYL

SEQ ID NO: 235 - protein, 9 aa, Artificial Sequence
FFHRTSVVY

SEQ ID NO: 236 - protein, 9 aa, Artificial Sequence
PWQYRNNPE

SEQ ID NO: 237 - protein, 9 aa, Artificial Sequence
QNDELYPYK

SEQ ID NO: 238 - protein, 9 aa, Artificial Sequence
YWENHRGHV

SEQ ID NO: 239 - protein, 9 aa, Artificial Sequence
YEAIERWHG

SEQ ID NO: 240 - protein, 9 aa, Artificial Sequence
WNANILRYW

SEQ ID NO: 241 - protein, 9 aa, Artificial Sequence
TPRYVPLNP

SEQ ID NO: 242 - protein, 9 aa, Artificial Sequence
PYHAFDWYW

SEQ ID NO: 243 - protein, 9 aa, Artificial Sequence
YDPSEWFPR

SEQ ID NO: 244 - protein, 9 aa, Artificial Sequence
FDIFYFNPI

SEQ ID NO: 245 - protein, 9 aa, Artificial Sequence
NLYFFFYQT

SEQ ID NO: 246 - protein, 111 aa, Artificial Sequence
MIPGGLSEAKPATPEIQEIVDKVKPQLEEKTGETYGKLEAVQYKTQVVHDVFYDQKAGTNYYIKVRAGDNKYMHLKVFKSLKWWYRIGNPEDLVLTGYQVDKNKDDELTGF

SEQ ID NO: 247 - protein, 111 aa, Artificial Sequence
MIPGGLSEAKPATPEIQEIVDKVKPQLEEKTGETYGKLEAVQYKTQVVPFKIITVWHGTNYYIKVRAGDNKYMHLKVFKSLLERFNFHGEEDLVLTGYQVDKNKDDELTGF

SEQ ID NO: 248 - protein, 111 aa, Artificial Sequence
MIPGGLSEAKPATPEIQEIVDKVKPQLEEKTGETYGKLEAVQYKTQVVQYKIITWWSGTNYYIKVRAGDNKYMHLKVFKSLVYKNKRGGHEDLVLTGYQVDKNKDDELTGF

SEQ ID NO: 249 - protein, 111 aa, Artificial Sequence
MIPGGLSEAKPATPEIQEIVDKVKPQLEEKTGETYGKLEAVQYKTQVVHYYVHYNDQGTNYYIKVRAGDNKYMHLKVFKSLWGENLFAKWEDLVLTGYQVDKNKDDELTGF

SEQ ID NO: 250 - protein, 111 aa, Artificial Sequence
MIPGGLSEAKPATPEIQEIVDKVKPQLEEKTGETYGKLEAVQYKTQVVYYQIITWWQGTNYYIKVRAGDNKYMHLKVFKSLGIRKKQQQREDLVLTGYQVDKNKDDELTGF

SEQ ID NO: 251 - protein, 111 aa, Artificial Sequence
MIPGGLSEAKPATPEIQEIVDKVKPQLEEKTGETYGKLEAVQYKTQVVVHGPHLEQAGTNYYIKVRAGDNKYMHLKVFKSLGHAFYFAFVEDLVLTGYQVDKNKDDELTGF

SEQ ID NO: 252 - protein, 111 aa, Artificial Sequence
MIPGGLSEAKPATPEIQEIVDKVKPQLEEKTGETYGKLEAVQYKTQVVLQDQWPWRDGTNYYIKVRAGDNKYMHLKVFKSLTYGKKWYSWEDLVLTGYQVDKNKDDELTGF

SEQ ID NO: 253 - protein, 103 aa, Artificial Sequence
MIPGGLSEAKPATPEIQEIVDKVKPQLEEKTGETYGKLEAVQYKTQVDAGTNYYIKVRAGDNKYMHLKVFKSLYFYRHWEDREDLVLTGYQVDKNKDDELTGF

SEQ ID NO: 254 - protein, 111 aa, Artificial Sequence
MIPGGLSEAKPATPEIQEIVDKVKPQLEEKTGETYGKLEAVQYKTQVVSWVKPDNELGTNYYIKVRAGDNKYMHLKVFKSLWQVHDKQWLEDLVLTGYQVDKNKDDELTGF

SEQ ID NO: 255 - protein, 111 aa, Artificial Sequence
MIPGGLSEAKPATPEIQEIVDKVKPQLEEKTGETYGKLEAVQYKTQVVNSLGVSEWVGTNYYIKVRAGDNKYMHLKVFKSLPYWYRKNNLEDLVLTGYQVDKNKDDELTGF

SEQ ID NO: 256 - protein, 111 aa, Artificial Sequence
MIPGGLSEAKPATPEIQEIVDKVKPQLEEKTGETYGKLEAVQYKTQVVVYRIVSWWRGTNYYIKVRAGDNKYMHLKVFKSLASDIYLRIDEDLVLTGYQVDKNKDDELTGF

SEQ ID NO: 257 - protein, 111 aa, Artificial Sequence
MIPGGLSEAKPATPEIQEIVDKVKPQLEEKTGETYGKLEAVQYKTQVVYYRQLKFNTGTNYYIKVRAGDNKYMHLKVFKSLFLHRKPQDREDLVLTGYQVDKNKDDELTGF

SEQ ID NO: 258 - protein, 111 aa, Artificial Sequence
MIPGGLSEAKPATPEIQEIVDKVKPQLEEKTGETYGKLEAVQYKTQVVGWIKVDNVLGTNYYIKVRAGDNKYMHLKVFKSLWQDHHNVKREDLVLTGYQVDKNKDDELTGF

SEQ ID NO: 259 - protein, 111 aa, Artificial Sequence
MIPGGLSEAKPATPEIQEIVDKVKPQLEEKTGETYGKLEAVQYKTQVVTAYYIHVNAGTNYYIKVRAGDNKYMHLKVFKSLPYGYRAKAPEDLVLTGYQVDKNKDDELTGF

SEQ ID NO: 260 - protein, 111 aa, Artificial Sequence
MIPGGLSEAKPATPEIQEIVDKVKPQLEEKTGETYGKLEAVQYKTQVVVRVEPTPNDGTNYYIKVRAGDNKYMHLKVFKSLPLVQELWGFEDLVLTGYQVDKNKDDELTGF

SEQ ID NO: 261 - protein, 111 aa, Artificial Sequence
MIPGGLSEAKPATPEIQEIVDKVKPQLEEKTGETYGKLEAVQYKTQVVDLNSSVWYQGTNYYIKVRAGDNKYMHLKVFKSLYWLLEIEHREDLVLTGYQVDKNKDDELTGF

SEQ ID NO: 262 - protein, 111 aa, Artificial Sequence
MIPGGLSEAKPATPEIQEIVDKVKPQLEEKTGETYGKLEAVQYKTQVVFTYQISYTVGTNYYIKVRAGDNKYMHLKVFKSLRWRYPARKPEDLVLTGYQVDKNKDDELTGF

SEQ ID NO: 263 - protein, 111 aa, Artificial Sequence
MIPGGLSEAKPATPEIQEIVDKVKPQLEEKTGETYGKLEAVQYKTQVVRENWYGEFAGTNYYIKVRAGDNKYMHLKVFKSLLYIYRHPNYEDLVLTGYQVDKNKDDELTGF

SEQ ID NO: 264 - protein, 111 aa, Artificial Sequence
MIPGGLSEAKPATPEIQEIVDKVKPQLEEKTGETYGKLEAVQYKTQVVTALAWNTQAGTNYYIKVRAGDNKYMHLKVFKSLPWLYRQKSDEDLVLTGYQVDKNKDDELTGF

SEQ ID NO: 265 - protein, 111 aa, Artificial Sequence
MIPGGLSEAKPATPEIQEIVDKVKPQLEEKTGETYGKLEAVQYKTQVVHIPALKVHAGTNYYIKVRAGDNKYMHLKVFKSLPYWYRHDQEEDLVLTGYQVDKNKDDELTGF

SEQ ID NO: 266 - protein, 111 aa, Artificial Sequence
MIPGGLSEAKPATPEIQEIVDKVKPQLEEKTGETYGKLEAVQYKTQVVHHAYAAVYVGTNYYIKVRAGDNKYMHLKVFKSLPYWYRKYPDEDLVLTGYQVDKNKDDELTGF

SEQ ID NO: 267 - protein, 110 aa, Artificial Sequence
MIPGGLSEAKPATPEIQEIVDKVKPQLEEKTGETYGKLEAVQYKTQVVYDELYHEKAGTNYYIKVRAGDNKYMHLKVFKSLEYKFRNLEEDLVLTGYQVDKNKDDELTGF

SEQ ID NO: 268 - protein, 111 aa, Artificial Sequence
MIPGGLSEAKPATPEIQEIVDKVKPQLEEKTGETYGKLEAVQYKTQVVSWYYPKNVLGTNYYIKVRAGDNKYMHLKVFKSLEDFIAADDDEDLVLTGYQVDKNKDDELTGF

SEQ ID NO: 269 - protein, 111 aa, Artificial Sequence
MIPGGLSEAKPATPEIQEIVDKVKPQLEEKTGETYGKLEAVQYKTQVVFLEWHFWEWGTNYYIKVRAGDNKYMHLKVFKSLDSQEFPSHLEDLVLTGYQVDKNKDDELTGF

SEQ ID NO: 270 - protein, 111 aa, Artificial Sequence
MIPGGLSEAKPATPEIQEIVDKVKPQLEEKTGETYGKLEAVQYKTQVVSWVRGTNQLGTNYYIKVRAGDNKYMHLKVFKSLEPDWPDFLIEDLVLTGYQVDKNKDDELTGF

SEQ ID NO: 271 - protein, 111 aa, Artificial Sequence
MIPGGLSEAKPATPEIQEIVDKVKPQLEEKTGETYGKLEAVQYKTQVVWRKLLSWWKGTNYYIKVRAGDNKYMHLKVFKSLILNPKSWNFEDLVLTGYQVDKNKDDELTGF

SEQ ID NO: 272 - protein, 111 aa, Artificial Sequence
MIPGGLSEAKPATPEIQEIVDKVKPQLEEKTGETYGKLEAVQYKTQVVPKSHQTNEQGTNYYIKVRAGDNKYMHLKVFKSLWNENHFSVWEDLVLTGYQVDKNKDDELTGF

SEQ ID NO: 273 - protein, 111 aa, Artificial Sequence
MIPGGLSEAKPATPEIQEIVDKVKPQLEEKTGETYGKLEAVQYKTQVVNWNQIDNPLGTNYYIKVRAGDNKYMHLKVFKSLNKDWEDQIIEDLVLTGYQVDKNKDDELTGF

SEQ ID NO: 274 - protein, 111 aa, Artificial Sequence
MIPGGLSEAKPATPEIQEIVDKVKPQLEEKTGETYGKLEAVQYKTQVVFWVGLHNQLGTNYYIKVRAGDNKYMHLKVFKSLYYNGDNTQIEDLVLTGYQVDKNKDDELTGF

SEQ ID NO: 275 - protein, 111 aa, Artificial Sequence
MIPGGLSEAKPATPEIQEIVDKVKPQLEEKTGETYGKLEAVQYKTQVVFTQPFNEPIGTNYYIKVRAGDNKYMHLKVFKSLYWDDKVGYYEDLVLTGYQVDKNKDDELTGF

SEQ ID NO: 276 - protein, 111 aa, Artificial Sequence
MIPGGLSEAKPATPEIQEIVDKVKPQLEEKTGETYGKLEAVQYKTQVVPEYQPQPKAGTNYYIKVRAGDNKYMHLKVFKSLFHFRKPQDREDLVLTGYQVDKNKDDELTGF

SEQ ID NO: 277 - protein, 111 aa, Artificial Sequence
MIPGGLSEAKPATPEIQEIVDKVKPQLEEKTGETYGKLEAVQYKTQVVNDPYFQSFSGTNYYIKVRAGDNKYMHLKVFKSLPYWYREPENEDLVLTGYQVDKNKDDELTGF

SEQ ID NO: 278 - protein, 111 aa, Artificial Sequence
MIPGGLSEAKPATPEIQEIVDKVKPQLEEKTGETYGKLEAVQYKTQVVHQDDVAWQSGTNYYIKVRAGDNKYMHLKVFKSLEYGWYHLPYEDLVLTGYQVDKNKDDELTGF

SEQ ID NO: 279 - protein, 111 aa, Artificial Sequence
MIPGGLSEAKPATPEIQEIVDKVKPQLEEKTGETYGKLEAVQYKTQVVKGYFHTVEAGTNYYIKVRAGDNKYMHLKVFKSLTYHFRTDLNEDLVLTGYQVDKNKDDELTGF

SEQ ID NO: 280 - protein, 111 aa, Artificial Sequence
MIPGGLSEAKPATPEIQEIVDKVKPQLEEKTGETYGKLEAVQYKTQVVVDQVWSENAGTNYYIKVRAGDNKYMHLKVFKSLPYLWRKHAVEDLVLTGYQVDKNKDDELTGF

SEQ ID NO: 281 - protein, 111 aa, Artificial Sequence
MIPGGLSEAKPATPEIQEIVDKVKPQLEEKTGETYGKLEAVQYKTQVVLSSIWQDVAGTNYYIKVRAGDNKYMHLKVFKSLLYQFRKEPVEDLVLTGYQVDKNKDDELTGF

SEQ ID NO: 282 - protein, 111 aa, Artificial Sequence
MIPGGLSEAKPATPEIQEIVDKVKPQLEEKTGETYGKLEAVQYKTQVVTASLYWNYAGTNYYIKVRAGDNKYMHLKVFKSLFYYRGPQPVEDLVLTGYQVDKNKDDELTGF

SEQ ID NO: 283 - protein, 111 aa, Artificial Sequence
MIPGGLSEAKPATPEIQEIVDKVKPQLEEKTGETYGKLEAVQYKTQVVSWKQWHNYLGTNYYIKVRAGDNKYMHLKVFKSLYPDGDLILYEDLVLTGYQVDKNKDDELTGF

SEQ ID NO: 284 - protein, 111 aa, Artificial Sequence
MIPGGLSEAKPATPEIQEIVDKVKPQLEEKTGETYGKLEAVQYKTQVVQVHLDNSPLGTNYYIKVRAGDNKYMHLKVFKSLQFGEIIWWEEDLVLTGYQVDKNKDDELTGF

SEQ ID NO: 285 - protein, 111 aa, Artificial Sequence
MIPGGLSEAKPATPEIQEIVDKVKPQLEEKTGETYGKLEAVQYKTQVVQNNWYLSNYGTNYYIKVRAGDNKYMHLKVFKSLVEERWGLWVEDLVLTGYQVDKNKDDELTGF

SEQ ID NO: 286 - protein, 111 aa, Artificial Sequence
MIPGGLSEAKPATPEIQEIVDKVKPQLEEKTGETYGKLEAVQYKTQVVWEWALLLEYGTNYYIKVRAGDNKYMHLKVFKSLHHPWQPAKQEDLVLTGYQVDKNKDDELTGF

SEQ ID NO: 287 - protein, 111 aa, Artificial Sequence
MIPGGLSEAKPATPEIQEIVDKVKPQLEEKTGETYGKLEAVQYKTQVVGDSYWEYVSGTNYYIKVRAGDNKYMHLKVFKSLPYRWRPDHAEDLVLTGYQVDKNKDDELTGF

SEQ ID NO: 288 - protein, 111 aa, Artificial Sequence
MIPGGLSEAKPATPEIQEIVDKVKPQLEEKTGETYGKLEAVQYKTQVVGQKWWQHKIGTNYYIKVRAGDNKYMHLKVFKSLHSNAWNLQHEDLVLTGYQVDKNKDDELTGF

SEQ ID NO: 289 - protein, 111 aa, Artificial Sequence
MIPGGLSEAKPATPEIQEIVDKVKPQLEEKTGETYGKLEAVQYKTQVVLDGLYHVNSGTNYYIKVRAGDNKYMHLKVFKSLFYYYRSEPTEDLVLTGYQVDKNKDDELTGF

SEQ ID NO: 290 - protein, 111 aa, Artificial Sequence
MIPGGLSEAKPATPEIQEIVDKVKPQLEEKTGETYGKLEAVQYKTQVVHAPAPVQAIGTNYYIKVRAGDNKYMHLKVFKSLPYWYRPNRPEDLVLTGYQVDKNKDDELTGF

SEQ ID NO: 291 - protein, 111 aa, Artificial Sequence
MIPGGLSEAKPATPEIQEIVDKVKPQLEEKTGETYGKLEAVQYKTQVVWEDHWNYQYGTNYYIKVRAGDNKYMHLKVFKSLELYSNQIVWEDLVLTGYQVDKNKDDELTGF

SEQ ID NO: 292 - protein, 111 aa, Artificial Sequence
MIPGGLSEAKPATPEIQEIVDKVKPQLEEKTGETYGKLEAVQYKTQVVSWRYKSNQLGTNYYIKVRAGDNKYMHLKVFKSLYKDWVVNPPEDLVLTGYQVDKNKDDELTGF

SEQ ID NO: 293 - protein, 111 aa, Artificial Sequence
MIPGGLSEAKPATPEIQEIVDKVKPQLEEKTGETYGKLEAVQYKTQVVRVDWWLPEVGTNYYIKVRAGDNKYMHLKVFKSLPYQYRKDPKEDLVLTGYQVDKNKDDELTGF

SEQ ID NO: 294 - protein, 111 aa, Artificial Sequence
MIPGGLSEAKPATPEIQEIVDKVKPQLEEKTGETYGKLEAVQYKTQVVSWIEISNQLGTNYYIKVRAGDNKYMHLKVFKSLYYGNTSILIEDLVLTGYQVDKNKDDELTGF

SEQ ID NO: 295 - protein, 111 aa, Artificial Sequence
MIPGGLSEAKPATPEIQEIVDKVKPQLEEKTGETYGKLEAVQYKTQVVSLGQAETWAGTNYYIKVRAGDNKYMHLKVFKSLFKYRHQQDKEDLVLTGYQVDKNKDDELTGF

SEQ ID NO: 296 - protein, 111 aa, Artificial Sequence
MIPGGLSEAKPATPEIQEIVDKVKPQLEEKTGETYGKLEAVQYKTQVVKIGQLPSRVGTNYYIKVRAGDNKYMHLKVFKSLYWYRNPADREDLVLTGYQVDKNKDDELTGF

SEQ ID NO: 297 - protein, 111 aa, Artificial Sequence
MIPGGLSEAKPATPEIQEIVDKVKPQLEEKTGETYGKLEAVQYKTQVVAWHTKNNSIGTNYYIKVRAGDNKYMHLKVFKSLETKLAHEDIEDLVLTGYQVDKNKDDELTGF

SEQ ID NO: 298 - protein, 111 aa, Artificial Sequence
MIPGGLSEAKPATPEIQEIVDKVKPQLEEKTGETYGKLEAVQYKTQVVQTKLVTWWWGTNYYIKVRAGDNKYMHLKVFKSLLGEQYIDVDEDLVLTGYQVDKNKDDELTGF

SEQ ID NO: 299 - protein, 111 aa, Artificial Sequence
MIPGGLSEAKPATPEIQEIVDKVKPQLEEKTGETYGKLEAVQYKTQVVAVFDYADPSGTNYYIKVRAGDNKYMHLKVFKSLPYRYRTHHKEDLVLTGYQVDKNKDDELTGF

SEQ ID NO: 300 - protein, 111 aa, Artificial Sequence
MIPGGLSEAKPATPEIQEIVDKVKPQLEEKTGETYGKLEAVQYKTQVVHVKIVTWWKGTNYYIKVRAGDNKYMHLKVFKSLYNPKPGIDNEDLVLTGYQVDKNKDDELTGF

SEQ ID NO: 301 - protein, 111 aa, Artificial Sequence
MIPGGLSEAKPATPEIQEIVDKVKPQLEEKTGETYGKLEAVQYKTQVVHVLKVSSVSGTNYYIKVRAGDNKYMHLKVFKSLFYYRKRYDREDLVLTGYQVDKNKDDELTGF

SEQ ID NO: 302 - protein, 111 aa, Artificial Sequence
MIPGGLSEAKPATPEIQEIVDKVKPQLEEKTGETYGKLEAVQYKTQVVYQDYDSATHGTNYYIKVRAGDNKYMHLKVFKSLYQYRNPIDKEDLVLTGYQVDKNKDDELTGF

SEQ ID NO: 303 - protein, 111 aa, Artificial Sequence
MIPGGLSEAKPATPEIQEIVDKVKPQLEEKTGETYGKLEAVQYKTQVVSWGKVSNELGTNYYIKVRAGDNKYMHLKVFKSLIEYQSPALYEDLVLTGYQVDKNKDDELTGF

SEQ ID NO: 304 - protein, 111 aa, Artificial Sequence
MIPGGLSEAKPATPEIQEIVDKVKPQLEEKTGETYGKLEAVQYKTQVVLEDEWWSILGTNYYIKVRAGDNKYMHLKVFKSLPDAPAYSKSEDLVLTGYQVDKNKDDELTGF

SEQ ID NO: 305 - protein, 111 aa, Artificial Sequence
MIPGGLSEAKPATPEIQEIVDKVKPQLEEKTGETYGKLEAVQYKTQVVYYKLVTWWRGTNYYIKVRAGDNKYMHLKVFKSLPDLNYEVTLEDLVLTGYQVDKNKDDELTGF

SEQ ID NO: 306 - protein, 111 aa, Artificial Sequence
MIPGGLSEAKPATPEIQEIVDKVKPQLEEKTGETYGKLEAVQYKTQVVAWVKEHNLIGTNYYIKVRAGDNKYMHLKVFKSLYDQNQWSPHEDLVLTGYQVDKNKDDELTGF

SEQ ID NO: 307 - protein, 111 aa, Artificial Sequence
MIPGGLSEAKPATPEIQEIVDKVKPQLEEKTGETYGKLEAVQYKTQVVQEYLWKQYIGTNYYIKVRAGDNKYMHLKVFKSLRWQYRHPQTEDLVLTGYQVDKNKDDELTGF

SEQ ID NO: 308 - protein, 111 aa, Artificial Sequence
MIPGGLSEAKPATPEIQEIVDKVKPQLEEKTGETYGKLEAVQYKTQVVFNKDLFLGWGTNYYIKVRAGDNKYMHLKVFKSLRFSAGEEWEEDLVLTGYQVDKNKDDELTGF

SEQ ID NO: 309 - protein, 111 aa, Artificial Sequence
MIPGGLSEAKPATPEIQEIVDKVKPQLEEKTGETYGKLEAVQYKTQVVHFGIRYAHVGTNYYIKVRAGDNKYMHLKVFKSLDYPRHHQDQEDLVLTGYQVDKNKDDELTGF

SEQ ID NO: 310 - protein, 111 aa, Artificial Sequence
MIPGGLSEAKPATPEIQEIVDKVKPQLEEKTGETYGKLEAVQYKTQVVWYAWQEGWQGTNYYIKVRAGDNKYMHLKVFKSLFRKKWAQLWEDLVLTGYQVDKNKDDELTGF

SEQ ID NO: 311 - protein, 111 aa, Artificial Sequence
MIPGGLSEAKPATPEIQEIVDKVKPQLEEKTGETYGKLEAVQYKTQVVGNAAWGSFAGTNYYIKVRAGDNKYMHLKVFKSLPFFYRKDNPEDLVLTGYQVDKNKDDELTGF

SEQ ID NO: 312 - protein, 111 aa, Artificial Sequence
MIPGGLSEAKPATPEIQEIVDKVKPQLEEKTGETYGKLEAVQYKTQVVREDLDLFYTGTNYYIKVRAGDNKYMHLKVFKSLEFILQPWWYEDLVLTGYQVDKNKDDELTGF

SEQ ID NO: 313 - protein, 111 aa, Artificial Sequence
MIPGGLSEAKPATPEIQEIVDKVKPQLEEKTGETYGKLEAVQYKTQVVNENVYRVTQGTNYYIKVRAGDNKYMHLKVFKSLKYRHRLTYEEDLVLTGYQVDKNKDDELTGF

SEQ ID NO: 314 - protein, 111 aa, Artificial Sequence
MIPGGLSEAKPATPEIQEIVDKVKPQLEEKTGETYGKLEAVQYKTQVVWHKIVTQWPGTNYYIKVRAGDNKYMHLKVFKSLYAQRGEVYFEDLVLTGYQVDKNKDDELTGF

SEQ ID NO: 315 - protein, 111 aa, Artificial Sequence
MIPGGLSEAKPATPEIQEIVDKVKPQLEEKTGETYGKLEAVQYKTQVVHYRIITHWEGTNYYIKVRAGDNKYMHLKVFKSLVRAFLYYKDEDLVLTGYQVDKNKDDELTGF

SEQ ID NO: 316 - protein, 111 aa, Artificial Sequence
MIPGGLSEAKPATPEIQEIVDKVKPQLEEKTGETYGKLEAVQYKTQVVLVFDASTSAGTNYYIKVRAGDNKYMHLKVFKSLPWEFRGDHKEDLVLTGYQVDKNKDDELTGF

SEQ ID NO: 317 - protein, 111 aa, Artificial Sequence
MIPGGLSEAKPATPEIQEIVDKVKPQLEEKTGETYGKLEAVQYKTQVVQYAEFLEHIGTNYYIKVRAGDNKYMHLKVFKSLGWSHYFQYLEDLVLTGYQVDKNKDDELTGF

SEQ ID NO: 318 - protein, 111 aa, Artificial Sequence
MIPGGLSEAKPATPEIQEIVDKVKPQLEEKTGETYGKLEAVQYKTQVVGNVQEDWHIGTNYYIKVRAGDNKYMHLKVFKSLFSEDLTLNGEDLVLTGYQVDKNKDDELTGF

SEQ ID NO: 319 - protein, 111 aa, Artificial Sequence
MIPGGLSEAKPATPEIQEIVDKVKPQLEEKTGETYGKLEAVQYKTQVVGWSASYPESGTNYYIKVRAGDNKYMHLKVFKSLTQWEFIEWPEDLVLTGYQVDKNKDDELTGF

SEQ ID NO: 320 - protein, 111 aa, Artificial Sequence
MIPGGLSEAKPATPEIQEIVDKVKPQLEEKTGETYGKLEAVQYKTQVVYQFEHISYGGTNYYIKVRAGDNKYMHLKVFKSLFTYRLPQHREDLVLTGYQVDKNKDDELTGF

SEQ ID NO: 321 - protein, 111 aa, Artificial Sequence
MIPGGLSEAKPATPEIQEIVDKVKPQLEEKTGETYGKLEAVQYKTQVVAWITPVNVLGTNYYIKVRAGDNKYMHLKVFKSLDEIFHGAYNEDLVLTGYQVDKNKDDELTGF

SEQ ID NO: 322 - protein, 111 aa, Artificial Sequence
MIPGGLSEAKPATPEIQEIVDKVKPQLEEKTGETYGKLEAVQYKTQVVESYAAIFWGGTNYYIKVRAGDNKYMHLKVFKSLWGEIQHWRQEDLVLTGYQVDKNKDDELTGF

SEQ ID NO: 323 - protein, 111 aa, Artificial Sequence
MIPGGLSEAKPATPEIQEIVDKVKPQLEEKTGETYGKLEAVQYKTQVVRVWPWTWDRGTNYYIKVRAGDNKYMHLKVFKSLEQWLPNPYFEDLVLTGYQVDKNKDDELTGF

SEQ ID NO: 324 - protein, 111 aa, Artificial Sequence
MIPGGLSEAKPATPEIQEIVDKVKPQLEEKTGETYGKLEAVQYKTQVVQVKKWWEYFVTNYYIKVRAGDNKYMHLKVFKSLQLLSHQWTEEDLVLTGYQVDKNKDDELTGF

SEQ ID NO: 325 - protein, 111 aa, Artificial Sequence
MIPGGLSEAKPATPEIQEIVDKVKPQLEEKTGETYGKLEAVQYKTQVVIGQISEQQWGTNYYIKVRAGDNKYMHLKVFKSLHRYWTRDVTEDLVLTGYQVDKNKDDELTGF

SEQ ID NO: 326 - protein, 111 aa, Artificial Sequence
MIPGGLSEAKPATPEIQEIVDKVKPQLEEKTGETYGKLEAVQYKTQVVAFHKLGWILGTNYYIKVRAGDNKYMHLKVFKSLGDESHKWHKEDLVLTGYQVDKNKDDELTGF

SEQ ID NO: 327 - protein, 111 aa, Artificial Sequence
MIPGGLSEAKPATPEIQEIVDKVKPQLEEKTGETYGKLEAVQYKTQVVFKKWWWKYKGTNYYIKVRAGDNKYMHLKVFKSLRVDEHYIQFEDLVLTGYQVDKNKDDELTGF

SEQ ID NO: 328 - protein, 111 aa, Artificial Sequence
MIPGGLSEAKPATPEIQEIVDKVKPQLEEKTGETYGKLEAVQYKTQVVASQRLWIIYGTNYYIKVRAGDNKYMHLKVFKSLSDWRHHGGWEDLVLTGYQVDKNKDDELTGF

SEQ ID NO: 329 - protein, 111 aa, Artificial Sequence
MIPGGLSEAKPATPEIQEIVDKVKPQLEEKTGETYGKLEAVQYKTQVVQRETHILWSGTNYYIKVRAGDNKYMHLKVFKSLWFDNLHNNFEDLVLTGYQVDKNKDDELTGF

SEQ ID NO: 330 - protein, 111 aa, Artificial Sequence
MIPGGLSEAKPATPEIQEIVDKVKPQLEEKTGETYGKLEAVQYKTQVVGQYWFWAPGGTNYYIKVRAGDNKYMHLKVFKSLPSSGGGPKWEDLVLTGYQVDKNKDDELTGF

SEQ ID NO: 331 - protein, 111 aa, Artificial Sequence
MIPGGLSEAKPATPEIQEIVDKVKPQLEEKTGETYGKLEAVQYKTQVVRDWAYYIYFGTNYYIKVRAGDNKYMHLKVFKSLRSDTLHYWNEDLVLTGYQVDKNKDDELTGF

SEQ ID NO: 332 - protein, 111 aa, Artificial Sequence
MIPGGLSEAKPATPEIQEIVDKVKPQLEEKTGETYGKLEAVQYKTQVVIGYKLNYIWGTNYYIKVRAGDNKYMHLKVFKSLIQYRWQDRVEDLVLTGYQVDKNKDDELTGF

SEQ ID NO: 333 - protein, 111 aa, Artificial Sequence
MIPGGLSEAKPATPEIQEIVDKVKPQLEEKTGETYGKLEAVQYKTQVVVSLTEQRWKGTNYYIKVRAGDNKYMHLKVFKSLFQPIKLANAEDLVLTGYQVDKNKDDELTGF

SEQ ID NO: 334 - protein, 111 aa, Artificial Sequence
MIPGGLSEAKPATPEIQEIVDKVKPQLEEKTGETYGKLEAVQYKTQVVWVSQQHYSHGTNYYIKVRAGDNKYMHLKVFKSLFAFRKYEDREDLVLTGYQVDKNKDDELTGF

SEQ ID NO: 335 - protein, 111 aa, Artificial Sequence
MIPGGLSEAKPATPEIQEIVDKVKPQLEEKTGETYGKLEAVQYKTQVVDDDNQHYGLGTNYYIKVRAGDNKYMHLKVFKSLLHNWWKGNWEDLVLTGYQVDKNKDDELTGF

SEQ ID NO: 336 - protein, 111 aa, Artificial Sequence
MIPGGLSEAKPATPEIQEIVDKVKPQLEEKTGETYGKLEAVQYKTQVVPTRWISIYWGTNYYIKVRAGDNKYMHLKVFKSLLNRYYHASIEDLVLTGYQVDKNKDDELTGF

SEQ ID NO: 337 - protein, 111 aa, Artificial Sequence
MIPGGLSEAKPATPEIQEIVDKVKPQLEEKTGETYGKLEAVQYKTQVVTAFAPNKASGTNYYIKVRAGDNKYMHLKVFKSLRYWAFRYLWEDLVLTGYQVDKNKDDELTGF

SEQ ID NO: 338 - protein, 111 aa, Artificial Sequence
MIPGGLSEAKPATPEIQEIVDKVKPQLEEKTGETYGKLEAVQYKTQVVHYTDFKWHKGTNYYIKVRAGDNKYMHLKVFKSLPFWANEHGWEDLVLTGYQVDKNKDDELTGF

SEQ ID NO: 339 - protein, 111 aa, Artificial Sequence
MIPGGLSEAKPATPEIQEIVDKVKPQLEEKTGETYGKLEAVQYKTQVVNKFWSWAPGGTNYYIKVRAGDNKYMHLKVFKSLADSGFNATPEDLVLTGYQVDKNKDDELTGF

SEQ ID NO: 340 - protein, 111 aa, Artificial Sequence
MIPGGLSEAKPATPEIQEIVDKVKPQLEEKTGETYGKLEAVQYKTQVVELDEPAWDWGTNYYIKVRAGDNKYMHLKVFKSLRQHKKPHPNEDLVLTGYQVDKNKDDELTGF

SEQ ID NO: 341 - protein, 111 aa, Artificial Sequence
MIPGGLSEAKPATPEIQEIVDKVKPQLEEKTGETYGKLEAVQYKTQVVHEKWGFWELGTNYYIKVRAGDNKYMHLKVFKSLHSHRFHEAHEDLVLTGYQVDKNKDDELTGF

SEQ ID NO: 342 - protein, 111 aa, Artificial Sequence
MIPGGLSEAKPATPEIQEIVDKVKPQLEEKTGETYGKLEAVQYKTQVVVATADLIKAGTNYYIKVRAGDNKYMHLKVFKSLPWHYPPNKWEDLVLTGYQVDKNKDDELTGF

SEQ ID NO: 343 - protein, 111 aa, Artificial Sequence
MIPGGLSEAKPATPEIQEIVDKVKPQLEEKTGETYGKLEAVQYKTQVVYYKVISWWHGTNYYIKVRAGDNKYMHLKVFKSLYKTPFPQYTEDLVLTGYQVDKNKDDELTGF

SEQ ID NO: 344 - protein, 111 aa, Artificial Sequence
MIPGGLSEAKPATPEIQEIVDKVKPQLEEKTGETYGKLEAVQYKTQVVHWHHYDNIIGTNYYIKVRAGDNKYMHLKVFKSLYQLVDLDLDEDLVLTGYQVDKNKDDELTGF

SEQ ID NO: 345 - protein, 111 aa, Artificial Sequence
MIPGGLSEAKPATPEIQEIVDKVKPQLEEKTGETYGKLEAVQYKTQVVVYKIITFWSGTNYYIKVRAGDNKYMHLKVFKSLEYPPVQQVLEDLVLTGYQVDKNKDDELTGF

SEQ ID NO: 346 - protein, 111 aa, Artificial Sequence
MIPGGLSEAKPATPEIQEIVDKVKPQLEEKTGETYGKLEAVQYKTQVVGWIQRHNLIGTNYYIKVRAGDNKYMHLKVFKSLYSEPPPVQNEDLVLTGYQVDKNKDDELTGF

SEQ ID NO: 347 - protein, 111 aa, Artificial Sequence
MIPGGLSEAKPATPEIQEIVDKVKPQLEEKTGETYGKLEAVQYKTQVVKTWEDTVVAGTNYYIKVRAGDNKYMHLKVFKSLEYLYRPLNPEDLVLTGYQVDKNKDDELTGF

SEQ ID NO: 348 - protein, 111 aa, Artificial Sequence
MIPGGLSEAKPATPEIQEIVDKVKPQLEEKTGETYGKLEAVQYKTQVVLDQHHVYQVGTNYYIKVRAGDNKYMHLKVFKSLALLIHHDPWEDLVLTGYQVDKNKDDELTGF

SEQ ID NO: 349 - protein, 111 aa, Artificial Sequence
MIPGGLSEAKPATPEIQEIVDKVKPQLEEKTGETYGKLEAVQYKTQVVLEDVWGVWAGTNYYIKVRAGDNKYMHLKVFKSLEFQHRTFNHEDLVLTGYQVDKNKDDELTGF

SEQ ID NO: 350 - protein, 111 aa, Artificial Sequence
MIPGGLSEAKPATPEIQEIVDKVKPQLEEKTGETYGKLEAVQYKTQVVWLPWTVELIGTNYYIKVRAGDNKYMHLKVFKSLGEIWSAKHKEDLVLTGYQVDKNKDDELTGF

SEQ ID NO: 351 - protein, 111 aa, Artificial Sequence
MIPGGLSEAKPATPEIQEIVDKVKPQLEEKTGETYGKLEAVKYKTQVVQHFTWDWFWGTNYYIKVRAGDNKYMHLKVFKSLPEYKPVDHTEDLVLTGYQVDKNKDDELTGF

SEQ ID NO: 352 - protein, 111 aa, Artificial Sequence
MIPGGLSEAKPATPEIQEIVDKVKPQLEEKTGETYGKLEAVQYKTQVVLFEVLQGSSGTNYYIKVRAGDNKYMHLKVFKSLGEIVWYQVEEDLVLTGYQVDKNKDDELTGF

SEQ ID NO: 353 - protein, 112 aa, Artificial Sequence
MIPGGLSEAKPATPEIQEIVDKVKPQLEEKTGETYGKLEAVQYKTQVVPYSWQHEVVGTNYYIKVRAGDNKYMHLKVFKSLIVFYLQEYYEEDLVLTGYQVDKNKDDELTGF

SEQ ID NO: 354 - protein, 111 aa, Artificial Sequence
MIPGGLSEAKPATPEIQEIVDKVKPQLEEKTGETYGKLEAVQYKTQVVWWQENAEWIGTNYYIKVRAGDNKYMHLKVFKSLGYAVFHKYLEDLVLTGYQVDKNKDDELTGF

SEQ ID NO: 355 - protein, 111 aa, Artificial Sequence
MIPGGLSEAKPATPEIQEIVDKVKPQLEEKTGETYGKLEAVQYKTQVVSYDPVYQDTGTNYYIKVRAGDNKYMHLKVFKSLFFHRTSVVYEDLVLTGYQVDKNKDDELTGF

SEQ ID NO: 356 - protein, 111 aa, Artificial Sequence
MIPGGLSEAKPATPEIQEIVDKVKPQLEEKTGETYGKLEAVQYKTQVVRVFDTPLAAGTNYYIKVRAGDNKYMHLKVFKSLPWQYRNNPEEDLVLTGYQVDKNKDDELTGF

SEQ ID NO: 357 - protein, 111 aa, Artificial Sequence
MIPGGLSEAKPATPEIQEIVDKVKPQLEEKTGETYGKLEAVQYKTQVVWWDIPWIWVGTNYYIKVRAGDNKYMHLKVFKSLQNDELYPYKEDLVLTGYQVDKNKDDELTGF

SEQ ID NO: 358 - protein, 111 aa, Artificial Sequence
MIPGGLSEAKPATPEIQEIVDKVKPQLEEKTGETYGKLEAVQYKTQVVYQKVITWWQGTNYYIKVRAGDNKYMHLKVFKSLYWENHRGHVEDLVLTGYQVDKNKDDELTGF

SEQ ID NO: 359 - protein, 111 aa, Artificial Sequence
MIPGGLSEAKPATPEIQEIVDKVKPQLEEKTGETYGKLEAVQYKTQVVQWIKWGNILGTNYYIKVRAGDNKYMHLKVFKSLYEAIERWHGEDLVLTGYQVDKNKDDELTGF

SEQ ID NO: 360 - protein, 111 aa, Artificial Sequence
MIPGGLSEAKPATPEIQEIVDKVKPQLEEKTGETYGKLEAVQYKTQVVATPEKKYVVGTNYYIKVRAGDNKYMHLKVFKSLWNANILRYWEDLVLTGYQVDKNKDDELTGF

SEQ ID NO: 361 - protein, 111 aa, Artificial Sequence
MIPGGLSEAKPATPEIQEIVDKVKPQLEEKTGETYGKLEAVQYKTQVVTSERLWILYGTNYYIKVRAGDNKYMHLKVFKSLTPRYVPLNPEDLVLTGYQVDKNKDDELTGF

SEQ ID NO: 362 - protein, 111 aa, Artificial Sequence
MIPGGLSEAKPATPEIQEIVDKVKPQLEEKTGETYGKLEAVQYKTQVVEHHSQPLAHGTNYYIKVRAGDNKYMHLKVFKSLPYHAFDWYWEDLVLTGYQVDKNKDDELTGF

SEQ ID NO: 363 - protein, 111 aa, Artificial Sequence
MIPGGLSEAKPATPEIQEIVDKVKPQLEEKTGETYGKLEAVQYKTQVVWTADWLWTVGTNYYIKVRAGDNKYMHLKVFKSLYDPSEWFPREDLVLTGYQVDKNKDDELTGF

SEQ ID NO: 364 - protein, 111 aa, Artificial Sequence
MIPGGLSEAKPATPEIQEIVDKVKPQLEEKTGETYGKLEAVQYKTQVVSFQREHYSWGTNYYIKVRAGDNKYMHLKVFKSLFDIFYFNPIEDLVLTGYQVDKNKDDELTGF

SEQ ID NO: 365 - protein, 111 aa, Artificial Sequence
MIPGGLSEAKPATPEIQEIVDKVKPQLEEKTGETYGKLEAVQYKTQVVGKTWHKHNRGTNYYIKVRAGDNKYMHLKVFKSLNLYFFFYQTEDLVLTGYQVDKNKDDELTGF

SEQ ID NO: 366 - DNA, 402 bp, Artificial Sequence
  source 1..402: mol_type = genomic DNA
atgattcccggcggactttcggaagccaagccagccactccggagattcaggaaatcgtggacaaggtcaaaccgcagctggaagagaaaaccggcgaaacctacggcaaactggaagccgtccagtataagactcaagtcgtccatgatgtgttttacgatcagaaagcaggtacgaactactacatcaaggttcgtgcgggtgacaacaagtatatgcacctgaaagtgtttaagagcctgaaatggtggtacagaatcggtaacccagaagatttggtgctgacgggctaccaggttgacaagaacaaagatgacgagctgacgggtttcgcggccgctgaacagaagctgatctccgaagaagatctggccgcgcatcaccatcaccaccactaatga

SEQ ID NO: 367 - DNA, 402 bp, Artificial Sequence
  source 1..402: mol_type = genomic DNA
atgattcccggcggactttcggaagccaagccagccactccggagattcaggaaatcgtggacaaggtcaaaccgcagctggaagagaaaaccggcgaaacctacggcaaactggaagccgtccagtataagactcaagtcgtcccattcaaaatcatcaccgtttggcatggtacgaactactacatcaaggttcgtgcgggtgacaacaagtatatgcacctgaaagtgtttaagagcctgctggaaagattcaacttccatggtgaagaagatttggtgctgacgggctaccaggttgacaagaacaaagatgacgagctgacgggtttcgcggccgctgaacagaagctgatctccgaagaagatctggccgcgcatcaccatcaccaccactaatga

SEQ ID NO: 368 - DNA, 402 bp, Artificial Sequence
  source 1..402: mol_type = genomic DNA
atgattcccggcggactttcggaagccaagccagccactccggagattcaggaaatcgtggacaaggtcaaaccgcagctggaagagaaaaccggcgaaacctacggcaaactggaagccgtccagtataagactcaagtcgtccagtacaaaatcatcacctggtggtctggtacgaactactacatcaaggttcgtgcgggtgacaacaagtatatgcacctgaaagtgtttaagagcctggtttacaaaaacaaaagaggtggtcatgaagatttggtgctgacgggctaccaggttgacaagaacaaagatgacgagctgacgggtttcgcggccgctgaacagaagctgatctccgaagaagatctggccgcgcatcaccatcaccaccactaatga

SEQ ID NO: 369 - DNA, 402 bp, Artificial Sequence
  source 1..402: mol_type = genomic DNA
atgattcccggcggactttcggaagccaagccagccactccggagattcaggaaatcgtggacaaggtcaaaccgcagctggaagagaaaaccggcgaaacctacggcaaactggaagccgtccagtataagactcaagtcgtccactactacgttcattacaacgatcagggtacgaactactacatcaaggttcgtgcgggtgacaacaagtatatgcacctgaaagtgtttaagagcctgtggggtgaaaacctgttcgcaaaatgggaagatttggtgctgacgggctaccaggttgacaagaacaaagatgacgagctgacgggtttcgcggccgctgaacagaagctgatctccgaagaagatctggccgcgcatcaccatcaccaccactaatga

SEQ ID NO: 370 - DNA, 402 bp, Artificial Sequence
  source 1..402: mol_type = genomic DNA
atgattcccggcggactttcggaagccaagccagccactccggagattcaggaaatcgtggacaaggtcaaaccgcagctggaagagaaaaccggcgaaacctacggcaaactggaagccgtccagtataagactcaagtcgtctactaccagatcatcacctggtggcagggtacgaactactacatcaaggttcgtgcgggtgacaacaagtatatgcacctgaaagtgtttaagagcctgggtatcagaaaaaaacagcagcagagagaagatttggtgctgacgggctaccaggttgacaagaacaaagatgacgagctgacgggtttcgcggccgctgaacagaagctgatctccgaagaagatctggccgcgcatcaccatcaccaccactaatga

SEQ ID NO: 371 - DNA, 402 bp, Artificial Sequence
  source 1..402: mol_type = genomic DNA
atgattcccggcggactttcggaagccaagccagccactccggagattcaggaaatcgtggacaaggtcaaaccgcagctggaagagaaaaccggcgaaacctacggcaaactggaagccgtccagtataagactcaagtcgtcgttcatggtccacatctggaacaggcaggtacgaactactacatcaaggttcgtgcgggtgacaacaagtatatgcacctgaaagtgtttaagagcctgggtcatgcattctacttcgcattcgttgaagatttggtgctgacgggctaccaggttgacaagaacaaagatgacgagctgacgggtttcgcggccgctgaacagaagctgatctccgaagaagatctggccgcgcatcaccatcaccaccactaatga

SEQ ID NO: 372 - DNA, 402 bp, Artificial Sequence
  source 1..402: mol_type = genomic DNA
atgattcccggcggactttcggaagccaagccagccactccggagattcaggaaatcgtggacaaggtcaaaccgcagctggaagagaaaaccggcgaaacctacggcaaactggaagccgtccagtataagactcaagtcgtcctgcaggatcagtggccatggcgtgatggtacgaactactacatcaaggttcgtgcgggtgacaacaagtatatgcacctgaaagtgtttaagagcctgacctacggtaaaaaatggtactcttgggaagatttggtgctgacgggctaccaggttgacaagaacaaagatgacgagctgacgggtttcgcggccgctgaacagaagctgatctccgaagaagatctggccgcgcatcaccatcaccaccactaatga

SEQ ID NO: 373 - DNA, 378 bp, Artificial Sequence
  source 1..378: mol_type = genomic DNA
atgattcccggcggactttcggaagccaagccagccactccggagattcaggaaatcgtggacaaggtcaaaccgcagctggaagagaaaaccggcgaaacctacggcaaactggaagccgtccagtataagactcaagtcgacgcgggtacgaactactacatcaaggttcgtgcgggtgacaacaagtatatgcacctgaaagtgtttaagagcctgtacttctacagacattgggaagatagagaagatttggtgctgacgggctaccaggttgacaagaacaaagatgacgagctgacgggtttcgcggccgctgaacagaagctgatctccgaagaagatctggccgcgcatcaccatcaccaccactaatga

SEQ ID NO: 374 - DNA, 402 bp, Artificial Sequence
  source 1..402: mol_type = genomic DNA
atgattcccggcggactttcggaagccaagccagccactccggagattcaggaaatcgtggacaaggtcaaaccgcagctggaagagaaaaccggcgaaacctacggcaaactggaagccgtccagtataagactcaagtcgtctcttgggttaaaccagataacgaactgggtacgaactactacatcaaggttcgtgcgggtgacaacaagtatatgcacctgaaagtgtttaagagcctgtggcaggttcatgataaacagtggctggaagatttggtgctgacgggctaccaggttgacaagaacaaagatgacgagctgacgggtttcgcggccgctgaacagaagctgatctccgaagaagatctggccgcgcatcaccatcaccaccactaatga

SEQ ID NO: 375 - DNA, 402 bp, Artificial Sequence
  source 1..402: mol_type = genomic DNA
atgattcccggcggactttcggaagccaagccagccactccggagattcaggaaatcgtggacaaggtcaaaccgcagctggaagagaaaaccggcgaaacctacggcaaactggaagccgtccagtataagactcaagtcgtcaactctctgggtgtttctgaatgggttggtacgaactactacatcaaggttcgtgcgggtgacaacaagtatatgcacctgaaagtgtttaagagcctgccatactggtacagaaaaaacaacctggaagatttggtgctgacgggctaccaggttgacaagaacaaagatgacgagctgacgggtttcgcggccgctgaacagaagctgatctccgaagaagatctggccgcgcatcaccatcaccaccactaatga

SEQ ID NO: 376 - DNA, 402 bp, Artificial Sequence
  source 1..402: mol_type = genomic DNA
atgattcccggcggactttcggaagccaagccagccactccggagattcaggaaatcgtggacaaggtcaaaccgcagctggaagagaaaaccggcgaaacctacggcaaactggaagccgtccagtataagactcaagtcgtcgtttaccgtatcgtttcttggtggcgtggtacgaactactacatcaaggttcgtgcgggtgacaacaagtatatgcacctgaaagtgtttaagagcctggcatctgatatctacctgagaatcgatgaagatttggtgctgacgggctaccaggttgacaagaacaaagatgacgagctgacgggtttcgcggccgctgaacagaagctgatctccgaagaagatctggccgcgcatcaccatcaccaccactaatga

SEQ ID NO: 377 - DNA, 402 bp, Artificial Sequence
  source 1..402: mol_type = genomic DNA
atgattcccggcggactttcggaagccaagccagccactccggagattcaggaaatcgtggacaaggtcaaaccgcagctggaagagaaaaccggcgaaacctacggcaaactggaagccgtccagtataagactcaagtcgtctactaccgtcagctgaaattcaacaccggtacgaactactacatcaaggttcgtgcgggtgacaacaagtatatgcacctgaaagtgtttaagagcctgttcctgcatagaaaaccacaggatagagaagatttggtgctgacgggctaccaggttgacaagaacaaagatgacgagctgacgggtttcgcggccgctgaacagaagctgatctccgaagaagatctggccgcgcatcaccatcaccaccactaatga

SEQ ID NO: 378 - DNA, 402 bp, Artificial Sequence
  source 1..402: mol_type = genomic DNA
atgattcccggcggactttcggaagccaagccagccactccggagattcaggaaatcgtggacaaggtcaaaccgcagctggaagagaaaaccggcgaaacctacggcaaactggaagccgtccagtataagactcaagtcgtcggttggatcaaagttgataacgttctgggtacgaactactacatcaaggttcgtgcgggtgacaacaagtatatgcacctgaaagtgtttaagagcctgtggcaggatcatcataacgttaaaagagaagatttggtgctgacgggctaccaggttgacaagaacaaagatgacgagctgacgggtttcgcggccgctgaacagaagctgatctccgaagaagatctggccgcgcatcaccatcaccaccactaatga

SEQ ID NO: 379 - DNA, 402 bp, Artificial Sequence
  source 1..402: mol_type = genomic DNA
atgattcccggcggactttcggaagccaagccagccactccggagattcaggaaatcgtggacaaggtcaaaccgcagctggaagagaaaaccggcgaaacctacggcaaactggaagccgtccagtataagactcaagtcgtcaccgcatactacatccatgttaacgcaggtacgaactactacatcaaggttcgtgcgggtgacaacaagtatatgcacctgaaagtgtttaagagcctgccatacggttacagagcaaaagcaccagaagatttggtgctgacgggctaccaggttgacaagaacaaagatgacgagctgacgggtttcgcggccgctgaacagaagctgatctccgaagaagatctggccgcgcatcaccatcaccaccactaatga

SEQ ID NO: 380 - DNA, 402 bp, Artificial Sequence
  source 1..402: mol_type = genomic DNA
atgattcccggcggactttcggaagccaagccagccactccggagattcaggaaatcgtggacaaggtcaaaccgcagctggaagagaaaaccggcgaaacctacggcaaactggaagccgtccagtataagactcaagtcgtcgttcgtgttgaaccaaccccaaacgatggtacgaactactacatcaaggttcgtgcgggtgacaacaagtatatgcacctaaaagtgtttaagagcctgccactggttcaggaactgtggggtttcgaagatttggtgctgacgggctaccaagttgacaagaacaaagatgacgagctgacgggtttcgcggccgctgaacagaagctgatctccgaagaagatctggccgcgcatcaccatcaccaccactaatga

SEQ ID NO: 381 - DNA, 402 bp, Artificial Sequence
  source 1..402: mol_type = genomic DNA
atgattcccggcggactttcggaagccaagccagccactccggagattcaggaaatcgtggacaaggtcaaaccgcagctggaagagaaaaccggcgaaacctacggcaaactggaagccgtccagtataagactcaagtcgtcgatctgaactcttctgtttggtaccagggtacgaactactacatcaaggttcgtgcgggtgacaacaagtatatgcacctgaaagtgtttaagagcctgtactggctgctggaaatcgaacatagagaagatttggtgctgacgggctaccaggttgacaagaacaaagatgacgagctgacgggtttcgcggccgctgaacagaagctgatctccgaagaagatctggccgcgcatcaccatcaccaccactaatga

SEQ ID NO: 382 - DNA, 402 bp, Artificial Sequence
  source 1..402: mol_type = genomic DNA
atgattcccggcggactttcggaagccaagccagccactccggagattcaggaaatcgtggacaaggtcaaaccgcagctggaagagaaaaccggcgaaacctacggcaaactggaagccgtccagtataagactcaagtcgtcttcacctaccagatctcttacaccgttggtacgaactactacatcaaggttcgtgcgggtgacaacaagtatatgcacctgaaagtgtttaagagcctgagatggagatacccagcaagaaaaccagaagatttggtgctgacgggctaccaggttgacaagaacaaagatgacgagctgacgggtttcgcggccgctgaacagaagctgatctccgaagaagatctggccgcgcatcaccatcaccaccactaatga

SEQ ID NO: 383 - DNA, 402 bp, Artificial Sequence
  source 1..402: mol_type = genomic DNA
atgattcccggcggactttcggaagccaagccagccactccggagattcaggaaatcgtggacaaggtcaaaccgcagctggaagagaaaaccggcgaaacctacggcaaactggaagccgtccagtataagactcaagtcgtccgtgaaaactggtacggtgaattcgcaggtacgaactactacatcaaggttcgtgcgggtgacaacaagtatatgcacctgaaagtgtttaagagcctgctgtacatctacagacatccaaactacgaagatttggtgctgacgggctaccaggttgacaagaacaaagatgacgagctgacgggtttcgcggccgctgaacagaagctgatctccgaagaagatctggccgcgcatcaccatcaccaccactaatga

SEQ ID NO: 384 - DNA, 402 bp, Artificial Sequence
  source 1..402: mol_type = genomic DNA
atgattcccggcggactttcggaagccaagccagccactccggagattcaggaaatcgtggacaaggtcaaaccgcagctggaagagaaaaccggcgaaacctacggcaaactggaagccgtccagtataagactcaagtcgtcaccgcactggcatggaacacccaggcaggtacgaactactacatcaaggttcgtgcgggtgacaacaagtatatgcacctgaaagtgtttaagagcctgccatggctgtacagacagaaatctgatgaagatttggtgctgacgggctaccaggttgacaagaacaaagatgacgagctgacgggtttcgcggccgctgaacagaagctgatctccgaagaagatctggccgcgcatcaccatcaccaccactaatga

SEQ ID NO: 385 - DNA, 402 bp, Artificial Sequence
  source 1..402: mol_type = genomic DNA
atgattcccggcggactttcggaagccaagccagccactccggagattcaggaaatcgtggacaaggtcaaaccgcagctggaagagaaaaccggcgaaacctacggcaaactggaagccgtccagtataagactcaagtcgtccatatcccagcactgaaagttcatgcaggtacgaactactacatcaaggttcgtgcgggtgacaacaagtatatgcacctgaaagtgtttaagagcctgccatactggtacagacatgatcaggaagaagatttggtgctgacgggctaccaggttgacaagaacaaagatgacgagctgacgggtttcgcggccgctgaacagaagctgatctccgaagaagatctggccgcgcatcaccatcaccaccactaatga

SEQ ID NO: 386 - DNA, 402 bp, Artificial Sequence
  source 1..402: mol_type = genomic DNA
atgattcccggcggactttcggaagccaagccagccactccggagattcaggaaatcgtggacaaggtcaaaccgcagctggaagagaaaaccggcgaaacctacggcaaactggaagccgtccagtataagactcaagtcgtccatcatgcatacgcagcagtttacgttggtacgaactactacatcaaggttcgtgcgggtgacaacaagtatatgcacctgaaagtgtttaagagcctgccatactggtacagaaaatacccagatgaagatttggtgctgacgggctaccaggttgacaagaacaaagatgacgagctgacgggtttcgcggccgctgaacagaagctgatctccgaagaagatctggccgcgcatcaccatcaccaccactaatga

SEQ ID NO: 387 - DNA, 399 bp, Artificial Sequence
  source 1..399: mol_type = genomic DNA
atgattcccggcggactttcggaagccaagccagccactccggagattcaggaaatcgtggacaaggtcaaaccgcagctggaagagaaaaccggcgaaacctacggcaaactggaagccgtccagtataagactcaagtcgtctacgatgaactgtaccatgaaaaagcaggtacgaactactacatcaaggttcgtgcgggtgacaacaagtatatgcacctgaaagtgtttaagagcctggaatacaaattcagaaacctggaagaagatttggtgctgacgggctaccaggttgacaagaacaaagatgacgagctgacgggtttcgcggccgctgaacagaagctgatctccgaagaagatctggccgcgcatcaccatcaccaccactaatga

SEQ ID NO: 388 - DNA, 402 bp, Artificial Sequence
  source 1..402: mol_type = genomic DNA
atgattcccggcggactttcggaagccaagccagccactccggagattcaggaaatcgtggacaaggtcaaaccgcagctggaagagaaaaccggcgaaacctacggcaaactggaagccgtccagtataagactcaagtcgtctcttggtactacccaaaaaacgttctgggtacgaactactacatcaaggttcgtgcgggtgacaacaagtatatgcacctgaaagtgtttaagagcctggaagatttcatcgcagcagatgatgatgaagatttggtgctgacgggctaccaggttgacaagaacaaagatgacgagctgacgggtttcgcggccgctgaacagaagctgatctccgaagaagatctggccgcgcatcaccatcaccaccactaatga

SEQ ID NO: 389 - DNA, 402 bp, Artificial Sequence
  source 1..402: mol_type = genomic DNA
atgattcccggcggactttcggaagccaagccagccactccggagattcaggaaatcgtggacaaggtcaaaccgcagctggaagagaaaaccggcgaaacctacggcaaactggaagccgtccagtataagactcaagtcgtcttcctggaatggcacttctgggaatggggtacgaactactacatcaaggttcgtgcgggtgacaacaagtatatgcacctgaaagtgtttaagagcctggattctcaggaattcccatctcatctggaagatttggtgctgacgggctaccaggttgacaagaacaaagatgacgagctgacgggtttcgcggccgctgaacagaagctgatctccgaagaagatctggccgcgcatcaccatcaccaccactaatga

SEQ ID NO: 390 - DNA, 402 bp, Artificial Sequence
  source 1..402: mol_type = genomic DNA
atgattcccggcggactttcggaagccaagccagccactccggagattcaggaaatcgtggacaaggtcaaaccgcagctggaagagaaaaccggcgaaacctacggcaaactggaagccgtccagtataagactcaagtcgtctcttgggttcgtggtaccaaccagctgggtacgaactactacatcaaggttcgtgcgggtgacaacaagtatatgcacctgaaagtgtttaagagcctggaaccagattggccagatttcctgatcgaagatttggtgctgacgggctaccaggttgacaagaacaaagatgacgagctgacgggtttcgcggccgctgaacagaagctgatctccgaagaagatctggccgcgcatcaccatcaccaccactaatga

SEQ ID NO: 391 - DNA, 402 bp, Artificial Sequence
  source 1..402: mol_type = genomic DNA
atgattcccggcggactttcggaagccaagccagccactccggagattcaggaaatcgtggacaaggtcaaaccgcagctggaagagaaaaccggcgaaacctacggcaaactggaagccgtccagtataagactcaagtcgtctggcgtaaactgctgtcttggtggaaaggtacgaactactacatcaaggttcgtgcgggtgacaacaagtatatgcacctgaaagtgtttaagagcctgatcctgaacccaaaatcttggaacttcgaagatttggtgctgacgggctaccaggttgacaagaacaaagatgacgagctgacgggtttcgcggccgctgaacagaagctgatctccgaagaagatctggccgcgcatcaccatcaccaccactaatga

SEQ ID NO: 392 - DNA, 402 bp, Artificial Sequence
  source 1..402: mol_type = genomic DNA
atgattcccggcggactttcggaagccaagccagccactccggagattcaggaaatcgtggacaaggtcaaaccgcagctggaagagaaaaccggcgaaacctacggcaaactggaagccgtccagtataagactcaagtcgtcccaaaatctcatcagaccaacgaacagggtacgaactactacatcaaggttcgtgcgggtgacaacaagtatatgcacctgaaagtgtttaagagcctgtggaacgaaaaccatttctctgtttgggaagatttggtgctgacgggctaccaggttgacaagaacaaagatgacgagctgacgggtttcgcggccgctgaacagaagctgatctccgaagaagatctggccgcgcatcaccatcaccaccactaatga

SEQ ID NO: 393 - DNA, 414 bp, Artificial Sequence
  source 1..414: mol_type = genomic DNA
atgattcccggcggactttcggaagccaagccagccactccggagattcaggaaatcgtggacaaggtcaaaccgcagctggaagagaaaaccggcgaaacctacggcaaactggaagccgtccagtataagactcaagtcgtcaactggaaccagatcgataacccactgggtacgaactactacatcaaggttcgtgcgggtgacaacaagtatatgcacctgaaagtgtttaagagcctgaacaaagattgggaagatcagatcatcgaagatttggtgctgacgggctaccaggttgacaagaacaaagatgacgagctgacgggtttcgcggccgcgggtggaagagcagaacagaagctgatctccgaagaagatctggccgcgcatcaccatcaccaccactaatga

SEQ ID NO: 394 - DNA, 402 bp, Artificial Sequence
  source 1..402: mol_type = genomic DNA
atgattcccggcggactttcggaagccaagccagccactccggagattcaggaaatcgtggacaaggtcaaaccgcagctggaagagaaaaccggcgaaacctacggcaaactggaagccgtccagtataagactcaagtcgtcttctgggttggtctgcataaccagctgggtacgaactactacatcaaggttcgtgcgggtgacaacaagtatatgcacctgaaagtgtttaagagcctgtactacaacggtgataacacccagatcgaagatttggtgctgacgggctaccaggttgacaagaacaaagatgacgagctgacgggtttcgcggccgctgaacagaagctgatctccgaagaagatctggccgcgcatcaccatcaccaccactaatga

SEQ ID NO: 395 - DNA, 402 bp, Artificial Sequence
  source 1..402: mol_type = genomic DNA
atgattcccggcggactttcggaagccaagccagccactccggagattcaggaaatcgtggacaaggtcaaaccgcagctggaagagaaaaccggcgaaacctacggcaaactggaagccgtccagtataagactcaagtcgtcttcacccagccattcaacgaaccaatcggtacgaactactacatcaaggttcgtgcgggtgacaacaagtatatgcacctgaaagtgtttaagagcctgtattgggatgataaagttggttactacgaagatttggtgctgacgggctaccaggttgacaagaacaaagatgacgagctgacgggtttcgcggccgctgaacagaagctgatctccgaagaagatctggccgcgcatcaccatcaccaccactaatga

SEQ ID NO: 396 - DNA, 402 bp, Artificial Sequence
  source 1..402: mol_type = genomic DNA
atgattcccggcggactttcggaagccaagccagccactccggagattcaggaaatcgtggacaaggtcaaaccgcagctggaagagaaaaccggcgaaacctacggcaaactggaagccgtccagtataagactcaagtcgtcccagaataccagccacagccaaaagcaggtacgaactactacatcaaggttcgtgcgggtgacaacaagtatatgcacctgaaagtgtttaagagcctgttccatttcagaaaaccacaggatagagaagatttggtgctgacgggctaccaggttgacaagaacaaagatgacgagctgacgggtttcgcggccgctgaacagaagctgatctccgaagaagatctggccgcgcatcaccatcaccaccactaatga

SEQ ID NO: 397 - DNA, 402 bp, Artificial Sequence
  source 1..402: mol_type = genomic DNA
atgattcccggcggactttcggaagccaagccagccactccggagattcaggaaatcgtggacaaggtcaaaccgcagctggaagagaaaaccggcgaaacctacggcaaactggaagccgtccagtataagactcaagtcgtcaacgatccatacttccagtctttctctggtacgaactactacatcaaggttcgtgcgggtgacaacaagtatatgcacctgaaagtgtttaagagcctgccatactggtacagagaaccagaaaacgaagatttggtgctgacgggctaccaggttgacaagaacaaagatgacgagctgacgggtttcgcggccgctgaacagaagctgatctccgaagaagatctggccgcgcatcaccatcaccaccactaatga

SEQ ID NO: 398 - DNA, 402 bp, Artificial Sequence
  source 1..402: mol_type = genomic DNA
atgattcccggcggactttcggaagccaagccagccactccggagattcaggaaatcgtggacaaggtcaaaccgcagctggaagagaaaaccggcgaaacctacggcaaactggaagccgtccagtataagactcaagtcgtccatcaggatgatgttgcatggcagtctggtacgaactactacatcaaggttcgtgcgggtgacaacaagtatatgcacctgaaagtgtttaagagcctggaatacggttggtaccatctgccatacgaagatttggtgctgacgggctaccaggttgacaagaacaaagatgacgagctgacgggtttcgcggccgctgaacagaagctgatctccgaagaagatctggccgcgcatcaccatcaccaccactaatga

SEQ ID NO: 399 - DNA, 402 bp, Artificial Sequence
  source 1..402: mol_type = genomic DNA
atgattcccggcggactttcggaagccaagccagccactccggagattcaggaaatcgtggacaaggtcaaaccgcagctggaagagaaaaccggcgaaacctacggcaaactggaagccgtccagtataagactcaagtcgtcaaaggttacttccataccgttgaagcaggtacgaactactacatcaaggttcgtgcgggtgacaacaagtatatgcacctgaaagtgtttaagagcctgacctaccatttcagaaccgatctgaacgaagatttggtgctgacgggctaccaggttgacaagaacaaagatgacgagctgacgggtttcgcggccgctgaacagaagctgatctccgaagaagatctggccgcgcatcaccatcaccaccactaatga

SEQ ID NO: 400 - DNA, 402 bp, Artificial Sequence
  source 1..402: mol_type = genomic DNA
atgattcccggcggactttcggaagccaagccagccactccggagattcaggaaatcgtggacaaggtcaaaccgcagctggaagagaaaaccggcgaaacctacggcaaactggaagccgtccagtataagactcaagtcgtcgttgatcaggtttggtctgaaaacgcaggtacgaactactacatcaaggttcgtgcgggtgacaacaagtatatgcacctgaaagtgtttaagagcctgccatacctgtggagaaaacatgcagttgaagatttggtgctgacgggctaccaggttgacaagaacaaagatgacgagctgacgggtttcgcggccgctgaacagaagctgatctccgaagaagatctggccgcgcatcaccatcaccaccactaatga

SEQ ID NO: 401 - DNA, 402 bp, Artificial Sequence
  source 1..402: mol_type = genomic DNA
atgattcccggcggactttcggaagccaagccagccactccggagattcaggaaatcgtggacaaggtcaaaccgcagctggaagagaaaaccggcgaaacctacggcaaactggaagccgtccagtataagactcaagtcgtcctgtcttctatctggcaggatgttgcaggtacgaactactacatcaaggttcgtgcgggtgacaacaagtatatgcacctgaaagtgtttaagagcctgctgtaccagttcagaaaagaaccagttgaagatttggtgctgacgggctaccaggttgacaagaacaaagatgacgagctgacgggtttcgcggccgctgaacagaagctgatctccgaagaagatctggccgcgcatcaccatcaccaccactaatga

SEQ ID NO: 402 - DNA, 402 bp, Artificial Sequence
  source 1..402: mol_type = genomic DNA
atgattcccggcggactttcggaagccaagccagccactccggagattcaggaaatcgtggacaaggtcaaaccgcagctggaagagaaaaccggcgaaacctacggcaaactggaagccgtccagtataagactcaagtcgtcaccgcatctctgtactggaactacgcaggtacgaactactacatcaaggttcgtgcgggtgacaacaagtatatgcacctgaaagtgtttaagagcctgttctactacagaggtccacagccagttgaagatttggtgctgacgggctaccaggttgacaagaacaaagatgacgagctgacgggtttcgcggccgctgaacagaagctgatctccgaagaagatctggccgcgcatcaccatcaccaccactaatga

SEQ ID NO: 403 - DNA, 402 bp, Artificial Sequence
  source 1..402: mol_type = genomic DNA
atgattcccggcggactttcggaagccaagccagccactccggagattcaggaaatcgtggacaaggtcaaaccgcagctggaagagaaaaccggcgaaacctacggcaaactggaagccgtccagtataagactcaagtcgtctcttggaaacagtggcataactacctgggtacgaactactacatcaaggttcgtgcgggtgacaacaagtatatgcacctgaaagtgtttaagagcctgtacccagatggtgatctgatcctgtacgaagatttggtgctgacgggctaccaggttgacaagaacaaagatgacgagctgacgggtttcgcggccgctgaacagaagctgatctccgaagaagatctggccgcgcatcaccatcaccaccactaatga

SEQ ID NO: 404 - DNA, 402 bp, Artificial Sequence
  source 1..402: mol_type = genomic DNA
atgattcccggcggactttcggaagccaagccagccactccggagattcaggaaatcgtggacaaggtcaaaccgcagctggaagagaaaaccggcgaaacctacggcaaactggaagccgtccagtataagactcaagtcgtccaggttcatctggataactctccactgggtacgaactactacatcaaggttcgtgcgggtgacaacaagtatatgcacctgaaagtgtttaagagcctgcagttcggtgaaatcatctggtgggaagaagatttggtgctgacgggctaccaggttgacaagaacaaagatgacgagctgacgggtttcgcggccgctgaacagaagctgatctccgaagaagatctggccgcgcatcaccatcaccaccactaatga

SEQ ID NO: 405 - DNA, 402 bp, Artificial Sequence
  source 1..402: mol_type = genomic DNA
atgattcccggcggactttcggaagccaagccagccactccggagattcaggaaatcgtggacaaggtcaaaccgcagctggaagagaaaaccggcgaaacctacggcaaactggaagccgtccagtataagactcaagtcgtccagaacaactggtacctgtctaactacggtacgaactactacatcaaggttcgtgcgggtgacaacaagtatatgcacctgaaagtgtttaagagcctggttgaagaaagatggggtctgtgggttgaagatttggtgctgacgggctaccaggttgacaagaacaaagatgacgagctgacgggtttcgcggccgctgaacagaagctgatctccgaagaagatctggccgcgcatcaccatcaccaccactaatga

SEQ ID NO: 406 - DNA, 402 bp, Artificial Sequence
  source 1..402: mol_type = genomic DNA
atgattcccggcggactttcggaagccaagccagccactccggagattcaggaaatcgtggacaaggtcaaaccgcagctggaagagaaaaccggcgaaacctacggcaaactggaagccgtccagtataagactcaagtcgtctgggaatgggcactgctgctggaatacggtacgaactactacatcaaggttcgtgcgggtgacaacaagtatatgcacctgaaagtgtttaagagcctgcatcatccatggcagccagcaaaacaggaagatttggtgctgacgggctaccaggttgacaagaacaaagatgacgagctgacgggtttcgcggccgctgaacagaagctgatctccgaagaagatctggccgcgcatcaccatcaccaccactaatga

SEQ ID NO: 407 - DNA, 402 bp, Artificial Sequence
  source 1..402: mol_type = genomic DNA
atgattcccggcggactttcggaagccaagccagccactccggagattcaggaaatcgtggacaaggtcaaaccgcagctggaagagaaaaccggcgaaacctacggcaaactggaagccgtccagtataagactcaagtcgtcggtgattcttactgggaatacgtttctggtacgaactactacatcaaggttcgtgcgggtgacaacaagtatatgcacctgaaagtgtttaagagcctgccatacagatggagaccagatcatgcagaagatttggtgctgacgggctaccaggttgacaagaacaaagatgacgagctgacgggtttcgcggccgctgaacagaagctgatctccgaagaagatctggccgcgcatcaccatcaccaccactaatga

SEQ ID NO: 408 - DNA, 402 bp, Artificial Sequence
  source 1..402: mol_type = genomic DNA
atgattcccggcggactttcggaagccaagccagccactccggagattcaggaaatcgtggacaaggtcaaaccgcagctggaagagaaaaccggcgaaacctacggcaaactggaagccgtccagtataagactcaagtcgtcggtcagaaatggtggcagcataaaatcggtacgaactactacatcaaggttcgtgcgggtgacaacaagtatatgcacctgaaagtgtttaagagcctgcattctaacgcatggaacctgcagcatgaagatttggtgctgacgggctaccaggttgacaagaacaaagatgacgagctgacgggtttcgcggccgctgaacagaagctgatctccgaagaagatctggccgcgcatcaccatcaccaccactaatga

SEQ ID NO: 409 - DNA, 402 bp, Artificial Sequence
  source 1..402: mol_type = genomic DNA
atgattcccggcggactttcggaagccaagccagccactccggagattcaggaaatcgtggacaaggtcaaaccgcagctggaagagaaaaccggcgaaacctacggcaaactggaagccgtccagtataagactcaagtcgtcctggatggtctgtaccatgttaactctggtacgaactactacatcaaggttcgtgcgggtgacaacaagtatatgcacctgaaagtgtttaagagcctgttctactactacagatctgaaccaaccgaagatttggtgctgacgggctaccaggttgacaagaacaaagatgacgagctgacgggtttcgcggccgctgaacagaagctgatctccgaagaagatctggccgcgcatcaccatcaccaccactaatga

SEQ ID NO: 410 - DNA, 402 bp, Artificial Sequence
  source 1..402: mol_type = genomic DNA
atgattcccggcggactttcggaagccaagccagccactccggagattcaggaaatcgtggacaaggtcaaaccgcagctggaagagaaaaccggcgaaacctacggcaaactggaagccgtccagtataagactcaagtcgtccatgcaccagcaccagttcaggcaatcggtacgaactactacatcaaggttcgtgcgggtgacaacaagtatatgcacctgaaagtgtttaagagcctgccatactggtacagaccaaacagaccagaagatttggtgctgacgggctaccaggttgacaagaacaaagatgacgagctgacgggtttcgcggccgctgaacagaagctgatctccgaagaagatctggccgcgcatcaccatcaccaccactaatga

SEQ ID NO: 411 - DNA, 402 bp, Artificial Sequence
  source 1..402: mol_type = genomic DNA
atgattcccggcggactttcggaagccaagccagccactccggagattcaggaaatcgtggacaaggtcaaaccgcagctggaagagaaaaccggcgaaacctacggcaaactggaagccgtccagtataagactcaagtcgtctgggaagatcattggaactaccagtacggtacgaactactacatcaaggttcgtgcgggtgacaacaagtatatgcacctgaaagtgtttaagagcctggaactgtactctaaccagatcgtttgggaagatttggtgctgacgggctaccaggttgacaagaacaaagatgacgagctgacgggtttcgcggccgctgaacagaagctgatctccgaagaagatctggccgcgcatcaccatcaccaccactaatga

SEQ ID NO: 412 - DNA, 402 bp, Artificial Sequence
  source 1..402: mol_type = genomic DNA
atgattcccggcggactttcggaagccaagccagccactccggagattcaggaaatcgtggacaaggtcaaaccgcagctggaagagaaaaccggcgaaacctacggcaaactggaagccgtccagtataagactcaagtcgtctcttggcgttacaaatctaaccagctgggtacgaactactacatcaaggttcgtgcgggtgacaacaagtatatgcacctgaaagtgtttaagagcctgtacaaagattgggttgttaacccaccagaagatttggtgctgacgggctaccaggttgacaagaacaaagatgacgagctgacgggtttcgcggccgctgaacagaagctgatctccgaagaagatctggccgcgcatcaccatcaccaccactaatga

SEQ ID NO: 413 - DNA, 402 bp, Artificial Sequence
  source 1..402: mol_type = genomic DNA
atgattcccggcggactttcggaagccaagccagccactccggagattcaggaaatcgtggacaaggtcaaaccgcagctggaagagaaaaccggcgaaacctacggcaaactggaagccgtccagtataagactcaagtcgtccgtgttgattggtggctgccagaagttggtacgaactactacatcaaggttcgtgcgggtgacaacaagtatatgcacctgaaagtgtttaagagcctgccataccagtacagaaaagatccaaaagaagatttggtgctgacgggctaccaggttgacaagaacaaagatgacgagctgacgggtttcgcggccgctgaacagaagctgatctccgaagaagatctggccgcgcatcaccatcaccaccactaatga

SEQ ID NO: 414 - DNA, 402 bp, Artificial Sequence
  source 1..402: mol_type = genomic DNA
atgattcccggcggactttcggaagccaagccagccactccggagattcaggaaatcgtggacaaggtcaaaccgcagctggaagagaaaaccggcgaaacctacggcaaactggaagccgtccagtataagactcaagtcgtctcttggatcgaaatctctaaccagctgggtacgaactactacatcaaggttcgtgcgggtgacaacaagtatatgcacctgaaagtgtttaagagcctgtactacggtaacacctctatcctgatcgaagatttggtgctgacgggctaccaggttgacaagaacaaagatgacgagctgacgggtttcgcggccgctgaacagaagctgatctccgaagaagatctggccgcgcatcaccatcaccaccactaatga

SEQ ID NO: 415 - DNA, 402 bp, Artificial Sequence
  source 1..402: mol_type = genomic DNA
atgattcccggcggactttcggaagccaagccagccactccggagattcaggaaatcgtggacaaggtcaaaccgcagctggaagagaaaaccggcgaaacctacggcaaactggaagccgtccagtataagactcaagtcgtctctctgggtcaggcagaaacctgggcaggtacgaactactacatcaaggttcgtgcgggtgacaacaagtatatgcacctgaaagtgtttaagagcctgttcaaatacagacatcagcaggataaagaagatttggtgctgacgggctaccaggttgacaagaacaaagatgacgagctgacgggtttcgcggccgctgaacagaagctgatctccgaagaagatctggccgcgcatcaccatcaccaccactaatga

SEQ ID NO: 416 - DNA, 402 bp, Artificial Sequence
  source 1..402: mol_type = genomic DNA
atgattcccggcggactttcggaagccaagccagccactccggagattcaggaaatcgtggacaaggtcaaaccgcagctggaagagaaaaccggcgaaacctacggcaaactggaagccgtccagtataagactcaagtcgtcaaaatcggtcagctgccatctcgtgttggtacgaactactacatcaaggttcgtgcgggtgacaacaagtatatgcacctgaaagtgtttaagagcctgtactggtacagaaacccagcagatagagaagatttggtgctgacgggctaccaggttgacaagaacaaagatgacgagctgacgggtttcgcggccgctgaacagaagctgatctccgaagaagatctggccgcgcatcaccatcaccaccactaatga

SEQ ID NO: 417 - DNA, 402 bp, Artificial Sequence
  source 1..402: mol_type = genomic DNA
atgattcccggcggactttcggaagccaagccagccactccggagattcaggaaatcgtggacaaggtcaaaccgcagctggaagagaaaaccggcgaaacctacggcaaactggaagccgtccagtataagactcaagtcgtcgcatggcataccaaaaacaactctatcggtacgaactactacatcaaggttcgtgcgggtgacaacaagtatatgcacctgaaagtgtttaagagcctggaaaccaaactggcacatgaagatatcgaagatttggtgctgacgggctaccaggttgacaagaacaaagatgacgagctgacgggtttcgcggccgctgaacagaagctgatctccgaagaagatctggccgcgcatcaccatcaccaccactaatga

SEQ ID NO: 418 - DNA, 402 bp, Artificial Sequence
  source 1..402: mol_type = genomic DNA
atgattcccggcggactttcggaagccaagccagccactccggagattcaggaaatcgtggacaaggtcaaaccgcagctggaagagaaaaccggcgaaacctacggcaaactggaagccgtccagtataagactcaagtcgtccagaccaaactggttacctggtggtggggtacgaactactacatcaaggttcgtgcgggtgacaacaagtatatgcacctgaaagtgtttaagagcctgctgggtgaacagtacatcgatgttgatgaagatttggtgctgacgggctaccaggttgacaagaacaaagatgacgagctgacgggtttcgcggccgctgaacagaagctgatctccgaagaagatctggccgcgcatcaccatcaccaccactaatga

SEQ ID NO: 419 - DNA, 402 bp, Artificial Sequence
  source 1..402: mol_type = genomic DNA
atgattcccggcggactttcggaagccaagccagccactccggagattcaggaaatcgtggacaaggtcaaaccgcagctggaagagaaaaccggcgaaacctacggcaaactggaagccgtccagtataagactcaagtcgtcgcagttttcgattacgcagatccatctggtacgaactactacatcaaggttcgtgcgggtgacaacaagtatatgcacctgaaagtgtttaagagcctgccatacagatacagaacccatcataaagaagatttggtgctgacgggctaccaggttgacaagaacaaagatgacgagctgacgggtttcgcggccgctgaacagaagctgatctccgaagaagatctggccgcgcatcaccatcaccaccactaatga

SEQ ID NO: 420 - DNA, 402 bp, Artificial Sequence
  source 1..402: mol_type = genomic DNA
atgattcccggcggactttcggaagccaagccagccactccggagattcaggaaatcgtggacaaggtcaaaccgcagctggaagagaaaaccggcgaaacctacggcaaactggaagccgtccagtataagactcaagtcgtccatgttaaaatcgttacctggtggaaaggtacgaactactacatcaaggttcgtgcgggtgacaacaagtatatgcacctgaaagtgtttaagagcctgtacaacccaaaaccaggtatcgataacgaagatttggtgctgacgggctaccaggttgacaagaacaaagatgacgagctgacgggtttcgcggccgctgaacagaagctgatctccgaagaagatctggccgcgcatcaccatcaccaccactaatga

SEQ ID NO: 421 - DNA, 402 bp, Artificial Sequence
  source 1..402: mol_type = genomic DNA
atgattcccggcggactttcggaagccaagccagccactccggagattcaggaaatcgtggacaaggtcaaaccgcagctggaagagaaaaccggcgaaacctacggcaaactggaagccgtccagtataagactcaagtcgtccatgttctgaaagtttcttctgtttctggtacgaactactacatcaaggttcgtgcgggtgacaacaagtatatgcacctgaaagtgtttaagagcctgttctactacagaaaaagatacgatagagaagatttggtgctgacgggctaccaggttgacaagaacaaagatgacgagctgacgggtttcgcggccgctgaacagaagctgatctccgaagaagatctggccgcgcatcaccatcaccaccactaatga

SEQ ID NO: 422 - DNA, 402 bp, Artificial Sequence
  source 1..402: mol_type = genomic DNA
atgattcccggcggactttcggaagccaagccagccactccggagattcaggaaatcgtggacaaggtcaaaccgcagctggaagagaaaaccggcgaaacctacggcaaactggaagccgtccagtataagactcaagtcgtctaccaggattacgattctgcaacccatggtacgaactactacatcaaggttcgtgcgggtgacaacaagtatatgcacctgaaagtgtttaagagcctgtaccagtacagaaacccaatcgataaagaagatttggtgctgacgggctaccaggttgacaagaacaaagatgacgagctgacgggtttcgcggccgctgaacagaagctgatctccgaagaagatctggccgcgcatcaccatcaccaccactaatga

SEQ ID NO: 423 - DNA, 402 bp, Artificial Sequence
  source 1..402: mol_type = genomic DNA
atgattcccggcggactttcggaagccaagccagccactccggagattcaggaaatcgtggacaaggtcaaaccgcagctggaagagaaaaccggcgaaacctacggcaaactggaagccgtccagtataagactcaagtcgtctcttggggtaaagtttctaacgaactgggtacgaactactacatcaaggttcgtgcgggtgacaacaagtatatgcacctgaaagtgtttaagagcctgatcgaataccagtctccagcactgtacgaagatttggtgctgacgggctaccaggttgacaagaacaaagatgacgagctgacgggtttcgcggccgctgaacagaagctgatctccgaagaagatctggccgcgcatcaccatcaccaccactaatga

SEQ ID NO: 424 - DNA, 402 bp, Artificial Sequence
  source 1..402: mol_type = genomic DNA
atgattcccggcggactttcggaagccaagccagccactccggagattcaggaaatcgtggacaaggtcaaaccgcagctggaagagaaaaccggcgaaacctacggcaaactggaagccgtccagtataagactcaagtcgtcctggaagatgaatggtggtctatcctgggtacgaactactacatcaaggttcgtgcgggtgacaacaagtatatgcacctgaaagtgtttaagagcctgccagatgcaccagcatactctaaatctgaagatttggtgctgacgggctaccaggttgacaagaacaaagatgacgagctgacgggtttcgcggccgctgaacagaagctgatctccgaagaagatctggccgcgcatcaccatcaccaccactaatga

SEQ ID NO: 425 - DNA, 402 bp, Artificial Sequence
  source 1..402: mol_type = genomic DNA
atgattcccggcggactttcggaagccaagccagccactccggagattcaggaaatcgtggacaaggtcaaaccgcagctggaagagaaaaccggcgaaacctacggcaaactggaagccgtccagtataagactcaagtcgtctactacaaactggttacctggtggcgtggtacgaactactacatcaaggttcgtgcgggtgacaacaagtatatgcacctgaaagtgtttaagagcctgccagatctgaactacgaagttaccctggaagatttggtgctgacgggctaccaggttgacaagaacaaagatgacgagctgacgggtttcgcggccgctgaacagaagctgatctccgaagaagatctggccgcgcatcaccatcaccaccactaatga

SEQ ID NO: 426 - DNA, 402 bp, Artificial Sequence
  source 1..402: mol_type = genomic DNA
atgattcccggcggactttcggaagccaagccagccactccggagattcaggaaatcgtggacaaggtcaaaccgcagctggaagagaaaaccggcgaaacctacggcaaactggaagccgtccagtataagactcaagtcgtcgcatgggttaaagaacataacctgatcggtacgaactactacatcaaggttcgtgcgggtgacaacaagtatatgcacctgaaagtgtttaagagcctgtacgatcagaaccagtggtctccacatgaagatttggtgctgacgggctaccaggttgacaagaacaaagatgacgagctgacgggtttcgcggccgctgaacagaagctgatctccgaagaagatctggccgcgcatcaccatcaccaccactaatga

SEQ ID NO: 427 - DNA, 402 bp, Artificial Sequence
  source 1..402: mol_type = genomic DNA
atgattcccggcggactttcggaagccaagccagccactccggagattcaggaaatcgtggacaaggtcaaaccgcagctggaagagaaaaccggcgaaacctacggcaaactggaagccgtccagtataagactcaagtcgtccaggaatacctgtggaaacagtacatcggtacgaactactacatcaaggttcgtgcgggtgacaacaagtatatgcacctgaaagtgtttaagagcctgagatggcagtacagacatccacagaccgaagatttggtgctgacgggctaccaggttgacaagaacaaagatgacgagctgacgggtttcgcggccgctgaacagaagctgatctccgaagaagatctggccgcgcatcaccatcaccaccactaatga

SEQ ID NO: 428 - DNA, 402 bp, Artificial Sequence
  source 1..402: mol_type = genomic DNA
atgattcccggcggactttcggaagccaagccagccactccggagattcaggaaatcgtggacaaggtcaaaccgcagctggaagagaaaaccggcgaaacctacggcaaactggaagccgtccagtataagactcaagtcgtcttcaacaaagatctgttcctgggttggggtacgaactactacatcaaggttcgtgcgggtgacaacaagtatatgcacctgaaagtgtttaagagcctgagattctctgcaggtgaagaatgggaagaagatttggtgctgacgggctaccaggttgacaagaacaaagatgacgagctgacgggtttcgcggccgctgaacagaagctgatctccgaagaagatctggccgcgcatcaccatcaccaccactaatga

SEQ ID NO: 429 - DNA, 402 bp, Artificial Sequence
  source 1..402: mol_type = genomic DNA
atgattcccggcggactttcggaagccaagccagccactccggagattcaggaaatcgtggacaaggtcaaaccgcagctggaagagaaaaccggcgaaacctacggcaaactggaagccgtccagtataagactcaagtcgtccatttcggtatccgttacgcacatgttggtacgaactactacatcaaggttcgtgcgggtgacaacaagtatatgcacctgaaagtgtttaagagcctggattacccaagacatcatcaggatcaggaagatttggtgctgacgggctaccaggttgacaagaacaaagatgacgagctgacgggtttcgcggccgctgaacagaagctgatctccgaagaagatctggccgcgcatcaccatcaccaccactaatga

SEQ ID NO: 430 - DNA, 402 bp, Artificial Sequence
  source 1..402: mol_type = genomic DNA
atgattcccggcggactttcggaagccaagccagccactccggagattcaggaaatcgtggacaaggtcaaaccgcagctggaagagaaaaccggcgaaacctacggcaaactggaagccgtccagtataagactcaagtcgtctggtacgcatggcaggaaggttggcagggtacgaactactacatcaaggttcgtgcgggtgacaacaagtatatgcacctgaaagtgtttaagagcctgttcagaaaaaaatgggcacagctgtgggaagatttggtgctgacgggctaccaggttgacaagaacaaagatgacgagctgacgggtttcgcggccgctgaacagaagctgatctccgaagaagatctggccgcgcatcaccatcaccaccactaatga

SEQ ID NO: 431 - DNA, 402 bp, Artificial Sequence
  source 1..402: mol_type = genomic DNA
atgattcccggcggactttcggaagccaagccagccactccggagattcaggaaatcgtggacaaggtcaaaccgcagctggaagagaaaaccggcgaaacctacggcaaactggaagccgtccagtataagactcaagtcgtcggtaacgcagcatggggttctttcgcaggtacgaactactacatcaaggttcgtgcgggtgacaacaagtatatgcacctgaaagtgtttaagagcctgccattcttctacagaaaagataacccagaagatttggtgctgacgggctaccaggttgacaagaacaaagatgacgagctgacgggtttcgcggccgctgaacagaagctgatctccgaagaagatctggccgcgcatcaccatcaccaccactaatga

SEQ ID NO: 432 - DNA, 402 bp, Artificial Sequence
  source 1..402: mol_type = genomic DNA
atgattcccggcggactttcggaagccaagccagccactccggagattcaggaaatcgtggacaaggtcaaaccgcagctggaagagaaaaccggcgaaacctacggcaaactggaagccgtccagtataagactcaagtcgtccgtgaagatctggatctgttctacaccggtacgaactactacatcaaggttcgtgcgggtgacaacaagtatatgcacctgaaagtgtttaagagcctggaattcatcctgcagccatggtggtacgaagatttggtgctgacgggctaccaggttgacaagaacaaagatgacgagctgacgggtttcgcggccgctgaacagaagctgatctccgaagaagatctggccgcgcatcaccatcaccaccactaatga

SEQ ID NO: 433 - DNA, 402 bp, Artificial Sequence
  source 1..402: mol_type = genomic DNA
atgattcccggcggactttcggaagccaagccagccactccggagattcaggaaatcgtggacaaggtcaaaccgcagctggaagagaaaaccggcgaaacctacggcaaactggaagccgtccagtataagactcaagtcgtcaacgaaaacgtttaccgtgttacccagggtacgaactactacatcaaggttcgtgcgggtgacaacaagtatatgcacctgaaagtgtttaagagcctgaaatacagacatagactgacctacgaagaagatttggtgctgacgggctaccaagttgacaagaacaaagatgacgagctgacgggtttcgcggccgctgaacagaagctgatctccgaagaagatctggccgcgcatcaccatcaccaccactaatga

SEQ ID NO: 434 - DNA, 402 bp, Artificial Sequence
  source 1..402: mol_type = genomic DNA
atgattcccggcggactttcggaagccaagccagccactccggagattcaggaaatcgtggacaaggtcaaaccgcagctggaagagaaaaccggcgaaacctacggcaaactggaagccgtccagtataagactcaagtcgtctggcataaaatcgttacccagtggccaggtacgaactactacatcaaggttcgtgcgggtgacaacaagtatatgcacctgaaagtgtttaagagcctgtacgcacagagaggtgaagtttacttcgaagatttggtgctgacgggctaccaggttgacaagaacaaagatgacgagctgacgggtttcgcggccgctgaacagaagctgatctccgaagaagatctggccgcgcatcaccatcaccaccactaatga

SEQ ID NO: 435 - DNA, 402 bp, Artificial Sequence
  source 1..402: mol_type = genomic DNA
atgattcccggcggactttcggaagccaagccagccactccggagattcaggaaatcgtggacaaggtcaaaccgcagctggaagagaaaaccggcgaaacctacggcaaactggaagccgtccagtataagactcaagtcgtccattaccgtatcatcacccattgggaaggtacgaactactacatcaaggttcgtgcgggtgacaacaagtatatgcacctgaaagtgtttaagagcctggttagagcattcctgtactacaaagatgaagatttggtgctgacgggctaccaggttgacaagaacaaagatgacgagctgacgggtttcgcggccgctgaacagaagctgatctccgaagaagatctggccgcgcatcaccatcaccaccactaatga

SEQ ID NO: 436 - DNA, 402 bp, Artificial Sequence
  source 1..402: mol_type = genomic DNA
atgattcccggcggactttcggaagccaagccagccactccggagattcaggaaatcgtggacaaggtcaaaccgcagctggaagagaaaaccggcgaaacctacggcaaactggaagccgtccagtataagactcaagtcgtcctggttttcgatgcatctacctctgcaggtacgaactactacatcaaggttcgtgcgggtgacaacaagtatatgcacctgaaagtgtttaagagcctgccatgggaattcagaggtgatcataaagaagatttggtgctgacgggctaccaggttgacaagaacaaagatgacgagctgacgggtttcgcggccgctgaacagaagctgatctccgaagaagatctggccgcgcatcaccatcaccaccactaatga

SEQ ID NO: 437 - DNA, 402 bp, Artificial Sequence
  source 1..402: mol_type = genomic DNA
atgattcccggcggactttcggaagccaagccagccactccggagattcaggaaatcgtggacaaggtcaaaccgcagctggaagagaaaaccggcgaaacctacggcaaactggaagccgtccagtataagactcaagtcgtccagtacgcagaattcctggaacatatcggtacgaactactacatcaaggttcgtgcgggtgacaacaagtatatgcacctgaaagtgtttaagagcctgggttggtctcattacttccagtacctggaagatttggtgctgacgggctaccaggttgacaagaacaaagatgacgagctgacgggtttcgcggccgctgaacagaagctgatctccgaagaagatctggccgcgcatcaccatcaccaccactaatga

SEQ ID NO: 438 - DNA, 402 bp, Artificial Sequence
  source 1..402: mol_type = genomic DNA
atgattcccggcggactttcggaagccaagccagccactccggagattcaggaaatcgtggacaaggtcaaaccgcagctggaagagaaaaccggcgaaacctacggcaaactggaagccgtccagtataagactcaagtcgtcggtaacgttcaggaagattggcatatcggtacgaactactacatcaaggttcgtgcgggtgacaacaagtatatgcacctgaaagtgtttaagagcctgttctctgaagatctgaccctgaacggtgaagatttggtgctgacgggctaccaggttgacaagaacaaagatgacgagctgacgggtttcgcggccgctgaacagaagctgatctccgaagaagatctggccgcgcatcaccatcaccaccactaatga

SEQ ID NO: 439 - DNA, 402 bp, Artificial Sequence
  source 1..402: mol_type = genomic DNA
atgattcccggcggactttcggaagccaagccagccactccggagattcaggaaatcgtggacaaggtcaaaccgcagctggaagagaaaaccggcgaaacctacggcaaactggaagccgtccagtataagactcaagtcgtcggttggtctgcatcttacccagaatctggtacgaactactacatcaaggttcgtgcgggtgacaacaagtatatgcacctgaaagtgtttaagagcctgacccagtgggaattcatcgaatggccagaagatttggtgctgacgggctaccaggttgacaagaacaaagatgacgagctgacgggtttcgcggccgctgaacagaagctgatctccgaagaagatctggccgcgcatcaccatcaccaccactaatga

SEQ ID NO: 440 - DNA, 402 bp, Artificial Sequence
  source 1..402: mol_type = genomic DNA
atgattcccggcggactttcggaagccaagccagccactccggagattcaggaaatcgtggacaaggtcaaaccgcagctggaagagaaaaccggcgaaacctacggcaaactggaagccgtccagtataagactcaagtcgtctaccagttcgaacatatctcctacggtggtacgaactactacatcaaggttcgtgcgggtgacaacaagtatatgcacctgaaagtgtttaagagcctgttcacctacagactgccacagcatagagaagatttggtgctgacgggctaccaggttgacaagaacaaagatgacgagctgacgggtttcgcggccgctgaacagaagctgatctccgaagaagatctggccgcgcatcaccatcaccaccactaatga

SEQ ID NO: 441 - DNA, 402 bp, Artificial Sequence
  source 1..402: mol_type = genomic DNA
atgattcccggcggactttcggaagccaagccagccactccggagattcaggaaatcgtggacaaggtcaaaccgcagctggaagagaaaaccggcgaaacctacggcaaactggaagccgtccagtataagactcaagtcgtcgcatggatcaccccagttaacgttctgggtacgaactactacatcaaggttcgtgcgggtgacaacaagtatatgcacctgaaagtgtttaagagcctggatgaaatcttccatggtgcatacaacgaagatttggtgctgacgggctaccaggttgacaagaacaaagatgacgagctgacgggtttcgcggccgctgaacagaagctgatctccgaagaagatctggccgcgcatcaccatcaccaccactaatga

SEQ ID NO: 442 - DNA, 402 bp, Artificial Sequence
  source 1..402: mol_type = genomic DNA
atgattcccggcggactttcggaagccaagccagccactccggagattcaggaaatcgtggacaaggtcaaaccgcagctggaagagaaaaccggcgaaacctacggaaaactggaagccgtccagtataagactcaagtcgtcgaatcttacgcagcaatcttctggggtggtacgaactactacatcaaggttcgtgcgggtgacaacaagtatatgcacctgaaagtgtttaagagcctgtggggtgaaatccagcattggagacaggaagatttggtgctgacgggctaccaggttgacaagaacaaagatgacgagctgacgggtttcgcggccgctgaacagaagctgatctccgaagaagatctggccgcgcatcaccatcaccaccactaatga

SEQ ID NO: 443 - DNA, 402 bp, Artificial Sequence
  source 1..402: mol_type = genomic DNA
atgattcccggcggactttcggaagccaagccagccactccggagattcaggaaatcgtggacaaggtcaaaccgcagctggaagagaaaaccggcgaaacctacggcaaactggaagccgtccagtataagactcaagtcgtccgtgtttggccatggacctgggatcgtggtacgaactactacatcaaggttcgtgcgggtgacaacaagtatatgcacctgaaagtgtttaagagcctggagcagtggctgccaaacccatacttcgaagatttggtgctgacgggctaccaggttgacaagaacaaagatgacgagctgacgggtttcgcggccgctgaacagaagctgatctccgaagaagatctggccgcgcatcaccatcaccaccactaatga

SEQ ID NO: 444 - DNA, 402 bp, Artificial Sequence
  source 1..402: mol_type = genomic DNA
atgattcccggcggactttcggaagccaagccagccactccggagattcaggaaatcgtggacaaggtcaaaccgcagctggaagagaaaaccggcgaaacctacggcaaactggaagccgtccagtataagactcaagtcgtccaggttaaaaaatggtgggaatacttcgttacgaactactacatcaaggttcgtgcgggtgacaacaagtatatgcacctgaaagtgtttaagagcctgcagctgctgtctcatcagtggaccgaagaagatttggtgctgacgggctaccaggttgacaagaacaaagatgacgagctgacgggtttcgcggccgctgaacagaagctgatctccgaagaagatctggccgcgcatcaccatcaccaccactaatga

SEQ ID NO: 445 - DNA, 402 bp, Artificial Sequence
  source 1..402: mol_type = genomic DNA
atgattcccggcggactttcggaagccaagccagccactccggagattcaggaaatcgtggacaaggtcaaaccgcagctggaagagaaaaccggcgaaacctacggcaaactggaagccgtccagtataagactcaagtcgtcatcggtcagatctctgaacagcagtggggtacgaactactacatcaaggttcgtgcgggtgacaacaagtatatgcacctgaaagtgtttaagagcctgcatagatactggaccagagatgttaccgaagatttggtgctgacgggctaccaggttgacaagaacaaagatgacgagctgacgggtttcgcggccgctgaacagaagctgatctccgaagaagatctggccgcgcatcaccatcaccaccactaatga

SEQ ID NO: 446 - DNA, 402 bp, Artificial Sequence
  source 1..402: mol_type = genomic DNA
atgattcccggcggactttcggaagccaagccagccactccggagattcaggaaatcgtggacaaggtcaaaccgcagctggaagagaaaaccggcgaaacctacggcaaactggaagccgtccagtataagactcaagtcgtcgcattccataaactgggttggatcctgggtacgaactactacatcaaggttcgtgcgggtgacaacaagtatatgcacctgaaagtgtttaagagcctgggtgatgaatctcataaatggcataaagaagatttggtgctgacgggctaccaggttgacaagaacaaagatgacgagctgacgggtttcgcggccgctgaacagaagctgatctccgaagaagatctggccgcgcatcaccatcaccaccactaatga

SEQ ID NO: 447 - DNA, 402 bp, Artificial Sequence
  source 1..402: mol_type = genomic DNA
atgattcccggcggactttcggaagccaagccagccactccggagattcaggaaatcgtggacaaggtcaaaccgcagctggaagagaaaaccggcgaaacctacggcaaactggaagccgtccagtataagactcaagtcgtcttcaaaaaatggtggtggaaatacaaaggtacgaactactacatcaaggttcgtgcgggtgacaacaagtatatgcacctgaaagtgtttaagagcctgagagttgatgaacattacatccagttcgaagatttggtgctgacgggctaccaggttgacaagaacaaagatgacgagctgacgggtttcgcggccgctgaacagaagctgatctccgaagaagatctggccgcgcatcaccatcaccaccactaatga

SEQ ID NO: 448 - DNA, 402 bp, Artificial Sequence
  source 1..402: mol_type = genomic DNA
atgattcccggcggactttcggaagccaagccagccactccggagattcaggaaatcgtggacaaggtcaaaccgcagctggaagagaaaaccggcgaaacctacggcaaactggaagccgtccagtataagactcaagtcgtcgcatctcagcgtctgtggatcatctacggtacgaactactacatcaaggttcgtgcgggtgacaacaagtatatgcacctgaaagtgtttaagagcctgtctgattggagacatcatggtggttgggaagatttggtgctgacgggctaccaggttgacaagaacaaagatgacgagctgacgggtttcgcggccgctgaacagaagctgatctccgaagaagatctggccgcgcatcaccatcaccaccactaatga

SEQ ID NO: 449 - DNA, 402 bp, Artificial Sequence
  source 1..402: mol_type = genomic DNA
atgattcccggcggactttcggaagccaagccagccactccggagattcaggaaatcgtggacaaggtcaaaccgcagctggaagagaaaaccggcgaaacctacggcaaactggaagccgtccagtataagactcaagtcgtccagcgtgaaacccatatcctgtggtctggtacgaactactacatcaaggttcgtgcgggtgacaacaagtatatgcacctgaaagtgtttaagagcctgtggttcgataacctgcataacaacttcgaagatttggtgctgacgggctaccaggttgacaagaacaaagatgacgagctgacgggtttcgcggccgctgaacagaagctgatctccgaagaagatctggccgcgcatcaccatcaccaccactaatga

SEQ ID NO: 450 - DNA, 402 bp, Artificial Sequence
  source 1..402: mol_type = genomic DNA
atgattcccggcggactttcggaagccaagccagccactccggagattcaggaaatcgtggacaaggtcaaaccgcagctggaagagaaaaccggcgaaacctacggcaaactggaagccgtccagtataagactcaagtcgtcggtcagtactggttctgggcaccaggtggtacgaactactacatcaaggttcgtgcgggtgacaacaagtatatgcacctgaaagtgtttaagagcctgccatcttctggtggtggtccaaaatgggaagatttggtgctgacgggctaccaggttgacaagaacaaagatgacgagctgacgggtttcgcggccgctgaacagaagctgatctccgaagaagatctggccgcgcatcaccatcaccaccactaatga

SEQ ID NO: 451 - DNA, 402 bp, Artificial Sequence
  source 1..402: mol_type = genomic DNA
atgattcccggcggactttcggaagccaagccagccactccggagattcaggaaatcgtggacaaggtcaaaccgcagctggaagagaaaaccggcgaaacctacggcaaactggaagccgtccagtataagactcaagtcgtccgtgattgggcatactacatctacttcggtacgaactactacatcaaggttcgtgcgggtgacaacaagtatatgcacctgaaagtgtttaagagcctgagatctgataccctgcattactggaacgaagatttggtgctgacgggctaccaggttgacaagaacaaagatgacgagctgacgggtttcgcggccgctgaacagaagctgatctccgaagaagatctggccgcgcatcaccatcaccaccactaatga

SEQ ID NO: 452 - DNA, 402 bp, Artificial Sequence
  source 1..402: mol_type = genomic DNA
atgattcccggcggactttcggaagccaagccagccactccggagattcaggaaatcgtggacaaggtcaaaccgcagctggaagagaaaaccggcgaaacctacggcaaactggaagccgtccagtataagactcaagtcgtcatcggttacaaactgaactacatctggggtacgaactactacatcaaggttcgtgcgggtgacaacaagtatatgcacctgaaagtgtttaagagcctgatccagtacagatggcaggatagagttgaagatttggtgctgacgggctaccaggttgacaagaacaaagatgacgagctgacgggtttcgcggccgctgaacagaagctgatctccgaagaagatctggccgcgcatcaccatcaccaccactaatga

SEQ ID NO: 453 - DNA, 402 bp, Artificial Sequence
  source 1..402: mol_type = genomic DNA
atgattcccggcggactttcggaagccaagccagccactccggagattcaggaaatcgtggacaaggtcaaaccgcagctggaagagaaaaccggcgaaacctacggcaaactggaagccgtccagtataagactcaagtcgtcgtttctctgaccgaacagcgttggaaaggtacgaactactacatcaaggttcgtgcgggtgacaacaagtatatgcacctgaaagtgtttaagagcctgttccagccaatcaaactggcaaacgcagaagatttggtgctgacgggctaccaggttgacaagaacaaagatgacgagctgacgggtttcgcggccgctgaacagaagctgatctccgaagaagatctggccgcgcatcaccatcaccaccactaatga

SEQ ID NO: 454 - DNA, 402 bp, Artificial Sequence
  source 1..402: mol_type = genomic DNA
atgattcccggcggactttcggaagccaagccagccactccggagattcaggaaatcgtggacaaggtcaaaccgcagctggaagagaaaaccggcgaaacctacggcaaactggaagccgtccagtataagactcaagtcgtctgggtttctcagcagcattactctcatggtacgaactactacatcaaggttcgtgcgggtgacaacaagtatatgcacctgaaagtgtttaagagcctgttcgcattcagaaaatacgaagatagagaagatttggtgctgacgggctaccaggttgacaagaacaaagatgacgagctgacgggtttcgcggccgctgaacagaagctgatctccgaagaagatctggccgcgcatcaccatcaccaccactaatga

SEQ ID NO: 455 - DNA, 402 bp, Artificial Sequence
  source 1..402: mol_type = genomic DNA
atgattcccggcggactttcggaagccaagccagccactccggagattcaggaaatcgtggacaaggtcaaaccgcagctggaagagaaaaccggcgaaacctacggcaaactggaagccgtccagtataagactcaagtcgtcgatgatgataaccagcattacggtctgggtacgaactactacatcaaggttcgtgcgggtgacaacaagtatatgcacctgaaagtgtttaagagcctgctgcataactggtggaaaggtaactgggaagatttggtgctgacgggctaccaggttgacaagaacaaagatgacgagctgacgggtttcgcggccgctgaacagaagctgatctccgaagaagatctggccgcgcatcaccatcaccaccactaatga

SEQ ID NO: 456 - DNA, 402 bp, Artificial Sequence
  source 1..402: mol_type = genomic DNA
atgattcccggcggactttcggaagccaagccagccactccggagattcaggaaatcgtggacaaggtcaaaccgcagctggaagagaaaaccggcgaaacctacggcaaactggaagccgtccagtataagactcaagtcgtcccaacccgttggatctctatctactggggtacgaactactacatcaaggttcgtgcgggtgacaacaagtatatgcacctgaaagtgtttaagagcctgctgaacagatactaccatgcatctatcgaagatttggtgctgacgggctaccaggttgacaagaacaaagatgacgagctgacgggtttcgcggccgctgaacagaagctgatctccgaagaagatctggccgcgcatcaccatcaccaccactaatga

SEQ ID NO: 457 - DNA, 402 bp, Artificial Sequence
  source 1..402: mol_type = genomic DNA
atgattcccggcggactttcggaagccaagccagccactccggagattcaggaaatcgtggacaaggtcaaaccgcagctggaagagaaaaccggcgaaacctacggcaaactggaagccgtccagtataagactcaagtcgtcaccgcattcgcaccaaacaaagcatctggtacgaactactacatcaaggttcgtgcgggtgacaacaagtatatgcacctgaaagtgtttaagagcctgagatactgggcattcagatacctgtgggaagatttggtgctgacgggctaccaggttgacaagaacaaagatgacgagctgacgggtttcgcggccgctgaacagaagctgatctccgaagaagatctggccgcgcatcaccatcaccaccactaatga

SEQ ID NO: 458 - DNA, 402 bp, Artificial Sequence
  source 1..402: mol_type = genomic DNA
atgattcccggcggactttcggaagccaagccagccactccggagattcaggaaatcgtggacaaggtcaaaccgcagctggaagagaaaaccggcgaaacctacggcaaactggaagccgtccagtataagactcaagtcgtccattacaccgatttcaaatggcataaaggtacgaactactacatcaaggttcgtgcgggtgacaacaagtatatgcacctgaaagtgtttaagagcctgccattctgggcaaacgaacatggttgggaagatttggtgctgacgggctaccaggttgacaagaacaaagatgacgagctgacgggtttcgcggccgctgaacagaagctgatctccgaagaagatctggccgcgcatcaccatcaccaccactaatga

SEQ ID NO: 459 - DNA, 402 bp, Artificial Sequence
  source 1..402: mol_type = genomic DNA
atgattcccggcggactttcggaagccaagccagccactccggagattcaggaaatcgtggacaaggtcaaaccgcagctggaagagaaaaccggcgaaacctacggcaaactggaagccgtccagtataagactcaagtcgtcaacaaattctggtcttgggcaccaggtggtacgaactactacatcaaggttcgtgcgggtgacaacaagtatatgcacctgaaagtgtttaagagcctggcagattctggtttcaacgcaaccccagaagatttggtgctgacgggctaccaggttgacaagaacaaagatgacgagctgacgggtttcgcggccgctgaacagaagctgatctccgaagaagatctggccgcgcatcaccatcaccaccactaatga

SEQ ID NO: 460 - DNA, 402 bp, Artificial Sequence
  source 1..402: mol_type = genomic DNA
atgattcccggcggactttcggaagccaagccagccactccggagattcaggaaatcgtggacaaggtcaaaccgcagctggaagagaaaaccggcgaaacctacggcaaactggaagccgtccagtataagactcaagtcgtcgaactggatgaaccagcatgggattggggtacgaactactacatcaaggttcgtgcgggtgacaacaagtatatgcacctgaaagtgtttaagagcctgagacagcataaaaaaccacatccaaacgaagatttggtgctgacgggctaccaggttgacaagaacaaagatgacgagctgacgggtttcgcggccgctgaacagaagctgatctccgaagaagatctggccgcgcatcaccatcaccaccactaatga

SEQ ID NO: 461 - DNA, 402 bp, Artificial Sequence
  source 1..402: mol_type = genomic DNA
atgattcccggcggactttcggaagccaagccagccactccggagattcaggaaatcgtggacaaggtcaaaccgcagctggaagagaaaaccggcgaaacctacggcaaactggaagccgtccagtataagactcaagtcgtccatgaaaaatggggtttctgggaactgggtacgaactactacatcaaggttcgtgcgggtgacaacaagtatatgcacctgaaagtgtttaagagcctgcattctcatagattccatgaagcacatgaagatttggtgctgacgggctaccaggttgacaagaacaaagatgacgagctgacgggtttcgcggccgctgaacagaagctgatctccgaagaagatctggccgcgcatcaccatcaccaccactaatga

SEQ ID NO: 462 - DNA, 402 bp, Artificial Sequence
  source 1..402: mol_type = genomic DNA
atgattcccggcggactttcggaagccaagccagccactccggagattcaggaaatcgtggacaaggtcaaaccgcagctggaagagaaaaccggcgaaacctacggcaaactggaagccgtccagtataagactcaagtcgtcgttgcaaccgcagatctgatcaaagcaggtacgaactactacatcaaggttcgtgcgggtgacaacaagtatatgcacctgaaagtgtttaagagcctgccatggcattacccaccaaacaaatgggaagatttggtgctgacgggctaccaggttgacaagaacaaagatgacgagctgacgggtttcgcggccgctgaacagaagctgatctccgaagaagatctggccgcgcatcaccatcaccaccactaatga

SEQ ID NO: 463 - DNA, 402 bp, Artificial Sequence
  source 1..402: mol_type = genomic DNA
atgattcccggcggactttcggaagccaagccagccactccggagattcaggaaatcgtggacaaggtcaaaccgcagctggaagagaaaaccggcgaaacctacggcaaactggaagccgtccagtataagactcaagtcgtctactacaaagttatctcttggtggcatggtacgaactactacatcaaggttcgtgcgggtgacaacaagtatatgcacctgaaagtgtttaagagcctgtacaaaaccccattcccacagtacaccgaagatttggtgctgacgggctaccaggttgacaagaacaaagatgacgagctgacgggtttcgcggccgctgaacagaagctgatctccgaagaagatctggccgcgcatcaccatcaccaccactaatga

SEQ ID NO: 464 - DNA, 402 bp, Artificial Sequence
  source 1..402: mol_type = genomic DNA
atgattcccggcggactttcggaagccaagccagccactccggagattcaggaaatcgtggacaaggtcaaaccgcagctggaagagaaaaccggcgaaacctacggcaaactggaagccgtccagtataagactcaagtcgtccattggcatcactacgataacatcatcggtacgaactactacatcaaggttcgtgcgggtgacaacaagtatatgcacctgaaagtgtttaagagcctgtaccagctggttgatctggatctggatgaagatttggtgctgacgggctaccaggttgacaagaacaaagatgacgagctgacgggtttcgcggccgctgaacagaagctgatctccgaagaagatctggccgcgcatcaccatcaccaccactaatga

SEQ ID NO: 465 - DNA, 402 bp, Artificial Sequence
  source 1..402: mol_type = genomic DNA
atgattcccggcggactttcggaagccaagccagccactccggagattcaggaaatcgtggacaaggtcaaaccgcagctggaagagaaaaccggcgaaacctacggcaaactggaagccgtccagtataagactcaagtcgtcgtttacaaaatcatcaccttctggtctggtacgaactactacatcaaggttcgtgcgggtgacaacaagtatatgcacctgaaagtgtttaagagcctggaatacccaccagttcagcaggttctggaagatttggtgctgacgggctaccaggttgacaagaacaaagatgacgagctgacgggtttcgcggccgctgaacagaagctgatctccgaagaagatctggccgcgcatcaccatcaccaccactaatga

SEQ ID NO: 466 - DNA, 402 bp, Artificial Sequence
  source 1..402: mol_type = genomic DNA
atgattcccggcggactttcggaagccaagccagccactccggagattcaggaaatcgtggacaaggtcaaaccgcagctggaagagaaaaccggcgaaacctacggcaaactggaagccgtccagtataagactcaagtcgtcggttggatccagcgtcataacctgatcggtacgaactactacatcaaggttcgtgcgggtgacaacaagtatatgcacctgaaagtgtttaagagcctgtactctgaaccaccaccagttcagaacgaagatttggtgctgacgggctaccaggttgacaagaacaaagatgacgagctgacgggtttcgcggccgctgaacagaagctgatctccgaagaagatctggccgcgcatcaccatcaccaccactaatga

SEQ ID NO: 467 - DNA, 402 bp, Artificial Sequence
  source 1..402: mol_type = genomic DNA
atgattcccggcggactttcggaagccaagccagccactccggagattcaggaaatcgtggacaaggtcaaaccgcagctggaagagaaaaccggcgaaacctacggcaaactggaagccgtccagtataagactcaagtcgtcaaaacctgggaagataccgttgttgcaggtacgaactactacatcaaggttcgtgcgggtgacaacaagtatatgcacctgaaagtgtttaagagcctggaatacctgtacagaccactgaacccagaagatttggtgctgacgggctaccaggttgacaagaacaaagatgacgagctgacgggtttcgcggccgctgaacagaagctgatctccgaagaagatctggccgcgcatcaccatcaccaccactaatga

SEQ ID NO: 468 - DNA, 402 bp, Artificial Sequence
  source 1..402: mol_type = genomic DNA
atgattcccggcggactttcggaagccaagccagccactccggagattcaggaaatcgtggacaaggtcaaaccgcagctggaagagaaaaccggcgaaacctacggcaaactggaagccgtccagtataagactcaagtcgtcctggatcagcatcatgtttaccaggttggtacgaactactacatcaaggttcgtgcgggtgacaacaagtatatgcacctgaaagtgtttaagagcctggcactgctgatccatcatgatccatgggaagatttggtgctgacgggctaccaggttgacaagaacaaagatgacgagctgacgggtttcgcggccgctgaacagaagctgatctccgaagaagatctggccgcgcatcaccatcaccaccactaatga

SEQ ID NO: 469 - DNA, 402 bp, Artificial Sequence
  source 1..402: mol_type = genomic DNA
atgattcccggcggactttcggaagccaagccagccactccggagattcaggaaatcgtggacaaggtcaaaccgcagctggaagagaaaaccggcgaaacctacggcaaactggaagccgtccagtataagactcaagtcgtcctggaagatgtttggggtgtttgggcaggtacgaactactacatcaaggttcgtgcgggtgacaacaagtatatgcacctgaaagtgtttaagagcctggaattccagcatagaaccttcaaccatgaagatttggtgctgacgggctaccaggttgacaagaacaaagatgacgagctgacgggtttcgcggccgctgaacagaagctgatctccgaagaagatctggccgcgcatcaccatcaccaccactaatga

SEQ ID NO: 470 - DNA, 402 bp, Artificial Sequence
  source 1..402: mol_type = genomic DNA
atgattcccggcggactttcggaagccaagccagccactccggagattcaggaaatcgtggacaaggtcaaaccgcagctggaagagaaaaccggcgaaacctacggcaaactggaagccgtccagtataagactcaagtcgtctggctgccatggaccgttgaactgatcggtacgaactactacatcaaggttcgtgcgggtgacaacaagtatatgcacctgaaagtgtttaagagcctgggtgaaatctggtctgcaaaacataaagaagatttggtgctgacgggctaccaggttgacaagaacaaagatgacgagctgacgggtttcgcggccgctgaacagaagctgatctccgaagaagatctggccgcgcatcaccatcaccaccactaatga

SEQ ID NO: 471 - DNA, 402 bp, Artificial Sequence
  source 1..402: mol_type = genomic DNA
atgattcccggcggactttcggaagccaagccagccactccggagattcaggaaatcgtggacaaggtcaaaccgcagctggaagagaaaaccggcgaaacctacggcaaactggaagccgtcaagtataagactcaagtcgtccagcatttcacctgggattggttctggggtacgaactactacatcaaggttcgtgcgggtgacaacaagtatatgcacctgaaagtgtttaagagcctgccagaatacaaaccagttgatcataccgaagatttggtgctgacgggctaccaggttgacaagaacaaagatgacgagctgacgggtttcgcggccgctgaacagaagctgatctccgaagaagatctggccgcgcatcaccatcaccaccactaatga

SEQ ID NO: 472 - DNA, 402 bp, Artificial Sequence
  source 1..402: mol_type = genomic DNA
atgattcccggcggactttcggaagccaagccagccactccggagattcaggaaatcgtggacaaggtcaaaccgcagctggaagagaaaaccggcgaaacctacggcaaactggaagccgtccagtataagactcaagtcgtcctgttcgaagttctgcaggggtcttctggtacgaactactacatcaaggttcgtgcgggtgacaacaagtatatgcacctgaaagtgtttaagagcctgggtgaaatcgtttggtaccaggttgaagaagatttggtgctgacgggctaccaggttgacaagaacaaagatgacgagctgacgggtttcgcggccgctgaacagaagctgatctccgaagaagatctggccgcgcatcaccatcaccaccactaatga

SEQ ID NO: 473 - DNA, 405 bp, Artificial Sequence
  source 1..405: mol_type = genomic DNA
atgattcccggcggactttcggaagccaagccagccactccggagattcaggaaatcgtggacaaggtcaaaccgcagctggaagagaaaaccggcgaaacctacggcaaactggaagccgtccagtataagactcaagtcgtcccatactcttggcagcatgaagttgttggtacgaactactacatcaaggttcgtgcgggtgacaacaagtatatgcacctgaaagtgtttaagagcctgatcgttttctacctgcaggaatactacgaagaagatttggtgctgacgggctaccaggttgacaagaacaaagatgacgagctgacgggtttcgcggccgctgaacagaagctgatctccgaagaagatctggccgcgcatcaccatcaccaccactaatga

SEQ ID NO: 474 - DNA, 402 bp, Artificial Sequence
  source 1..402: mol_type = genomic DNA
atgattcccggcggactttcggaagccaagccagccactccggagattcaggaaatcgtggacaaggtcaaaccgcagctggaagagaaaaccggcgaaacctacggcaaactggaagccgtccagtataagactcaagtcgtctggtggcaggaaaacgcagaatggatcggtacgaactactacatcaaggttcgtgcgggtgacaacaagtatatgcacctgaaagtgtttaagagcctgggttacgcagttttccataaatacctggaagatttggtgctgacgggctaccaggttgacaagaacaaagatgacgagctgacgggtttcgcggccgctgaacagaagctgatctccgaagaagatctggccgcgcatcaccatcaccaccactaatga

SEQ ID NO: 475 - DNA, 402 bp, Artificial Sequence
  source 1..402: mol_type = genomic DNA
atgattcccggcggactttcggaagccaagccagccactccggagattcaggaaatcgtggacaaggtcaaaccgcagctggaagagaaaaccggcgaaacctacggcaaactggaagccgtccagtataagactcaagtcgtctcttacgatccagtttaccaggataccggtacgaactactacatcaaggttcgtgcgggtgacaacaagtatatgcacctgaaagtgtttaagagcctgttcttccataggacctctgttgtttacgaagatttggtgctgacgggctaccaggttgacaagaacaaagatgacgagctgacgggtttcgcggccgctgaacagaagctgatctccgaagaagatctggccgcgcatcaccatcaccaccactaatga

SEQ ID NO: 476 - DNA, 402 bp, Artificial Sequence
  source 1..402: mol_type = genomic DNA
atgattcccggcggactttcggaagccaagccagccactccggagattcaggaaatcgtggacaaggtcaaaccgcagctggaagagaaaaccggcgaaacctacggcaaactggaagccgtccagtataagactcaagtcgtccgtgttttcgataccccactggcagcaggtacgaactactacatcaaggttcgtgcgggtgacaacaagtatatgcacctgaaagtgtttaagagcctgccatggcagtacagaaacaacccagaagaagatttggtgctgacgggctaccaggttgacaagaacaaagatgacgagctgacgggtttcgcggccgctgaacagaagctgatctccgaagaagatctggccgcgcatcaccatcaccaccactaatga

SEQ ID NO: 477 - DNA, 402 bp, Artificial Sequence
  source 1..402: mol_type = genomic DNA
atgattcccggcggactttcggaagccaagccagccactccggagattcaggaaatcgtggacaaggtcaaaccgcagctggaagagaaaaccggcgaaacctacggcaaactggaagccgtccagtataagactcaagtcgtctggtgggatatcccatggatctgggttggtacgaactactacatcaaggttcgtgcgggtgacaacaagtatatgcacctgaaagtgtttaagagcctgcagaacgatgaactgtacccatacaaagaagatttggtgctgacgggctaccaggttgacaagaacaaagatgacgagctgacgggtttcgcggccgctgaacagaagctgatctccgaagaagatctggccgcgcatcaccatcaccaccactaatga

SEQ ID NO: 478 - DNA, 402 bp, Artificial Sequence
  source 1..402: mol_type = genomic DNA
atgattcccggcggactttcggaagccaagccagccactccggagattcaggaaatcgtggacaaggtcaaaccgcagctggaagagaaaaccggcgaaacctacggcaaactggaagccgtccagtataagactcaagtcgtctaccagaaagttatcacctggtggcagggtacgaactactacatcaaggttcgtgcgggtgacaacaagtatatgcacctgaaagtgtttaagagcctgtactgggaaaaccatagaggtcatgttgaagatttggtgctgacgggctaccaggttgacaagaacaaagatgacgagctgacgggtttcgcggccgctgaacagaagctgatctccgaagaagatctggccgcgcatcaccatcaccaccactaatga

SEQ ID NO: 479 - DNA, 402 bp, Artificial Sequence
  source 1..402: mol_type = genomic DNA
atgattcccggcggactttcggaagccaagccagccactccggagattcaggaaatcgtggacaaggtcaaaccgcagctggaagagaaaaccggcgaaacctacggcaaactggaagccgtccagtataagactcaagtcgtccagtggatcaaatggggtaacatcctgggtacgaactactacatcaaggttcgtgcgggtgacaacaagtatatgcacctgaaagtgtttaagagcctgtacgaagcaatcgaaagatggcatggtgaagatttggtgctgacgggctaccaggttgacaagaacaaagatgacgagctgacgggtttcgcggccgctgaacagaagctgatctccgaagaagatctggccgcgcatcaccatcaccaccactaatga

SEQ ID NO: 480 - DNA, 402 bp, Artificial Sequence
  source 1..402: mol_type = genomic DNA
atgattcccggcggactttcggaagccaagccagccactccggagattcaggaaatcgtggacaaggtcaaaccgcagctggaagagaaaaccggcgaaacctacggcaaactggaagccgtccagtataagactcaagtcgtcgcaaccccagaaaaaaaatacgttgttggtacgaactactacatcaaggttcgtgcgggtgacaacaagtatatgcacctgaaagtgtttaagagcctgtggaacgcaaacatcctgagatactgggaagatttggtgctgacgggctaccaggttgacaagaacaaagatgacgagctgacgggtttcgcggccgctgaacagaagctgatctccgaagaagatctggccgcgcatcaccatcaccaccactaatga

SEQ ID NO: 481 - DNA, 402 bp, Artificial Sequence
  source 1..402: mol_type = genomic DNA
atgattcccggcggactttcggaagccaagccagccactccggagattcaggaaatcgtggacaaggtcaaaccgcagctggaagagaaaaccggcgaaacctacggcaaactggaagccgtccagtataagactcaagtcgtcacctctgaacgtctgtggatcctgtacggtacgaactactacatcaaggttcgtgcgggtgacaacaagtatatgcacctgaaagtgtttaagagcctgaccccaagatacgttccactgaacccagaagatttggtgctgacgggctaccaggttgacaagaacaaagatgacgagctgacgggtttcgcggccgctgaacagaagctgatctccgaagaagatctggccgcgcatcaccatcaccaccactaatga

SEQ ID NO: 482 - DNA, 402 bp, Artificial Sequence
  source 1..402: mol_type = genomic DNA
atgattcccggcggactttcggaagccaagccagccactccggagattcaggaaatcgtggacaaggtcaaaccgcagctggaagagaaaaccggcgaaacctacggcaaactggaagccgtccagtataagactcaagtcgtcgaacatcattctcagccactggcacatggtacgaactactacatcaaggttcgtgcgggtgacaacaagtatatgcacctgaaagtgtttaagagcctgccataccatgcattcgattggtactgggaagatttggtgctgacgggctaccaggttgacaagaacaaagatgacgagctgacgggtttcgcggccgctgaacagaagctgatctccgaagaagatctggccgcgcatcaccatcaccaccactaatga

SEQ ID NO: 483 - DNA, 402 bp, Artificial Sequence
  source 1..402: mol_type = genomic DNA
atgattcccggcggactttcggaagccaagccagccactccggagattcaggaaatcgtggacaaggtcaaaccgcagctggaagagaaaaccggcgaaacctacggcaaactggaagccgtccagtataagactcaagtcgtctggaccgcagattggctgtggaccgttggtacgaactactacatcaaggttcgtgcgggtgacaacaagtatatgcacctgaaagtgtttaagagcctgtacgatccatctgaatggttcccaagagaagatttggtgctgacgggctaccaggttgacaagaacaaagatgacgagctgacgggtttcgcggccgctgaacagaagctgatctccgaagaagatctggccgcgcatcaccatcaccaccactaatga

SEQ ID NO: 484 - DNA, 402 bp, Artificial Sequence
  source 1..402: mol_type = genomic DNA
atgattcccggcggactttcggaagccaagccagccactccggagattcaggaaatcgtggacaaggtcaaaccgcagctggaagagaaaaccggcgaaacctacggcaaactggaagccgtccagtataagactcaagtcgtctctttccagcgtgaacattactcttggggtacgaactactacatcaaggttcgtgcgggtgacaacaagtatatgcacctgaaagtgtttaagagcctgttcgatatcttctacttcaacccaatcgaagatttggtgctgacgggctaccaggttgacaagaacaaagatgacgagctgacgggtttcgcggccgctgaacagaagctgatctccgaagaagatctggccgcgcatcaccatcaccaccactaatga

SEQ ID NO: 485 - DNA, 402 bp, Artificial Sequence
  source 1..402: mol_type = genomic DNA
atgattcccggcggactttcggaagccaagccagccactccggagattcaggaaatcgtggacaaggtcaaaccgcagctggaagagaaaaccggcgaaacctacggcaaactggaagccgtccagtataagactcaagtcgtcggtaaaacctggcataaacataaccgtggtacgaactactacatcaaggttcgtgcgggtgacaacaagtatatgcacctgaaagtgtttaagagcctgaacctgtacttcttcttctaccagaccgaagatttggtgctgacgggctaccaggttgacaagaacaaagatgacgagctgacgggtttcgcggccgctgaacagaagctgatctccgaagaagatctggccgcgcatcaccatcaccaccactaatga

SEQ ID NO: 486 - protein, 18 aa, unidentified
MKWVTFISLLFLFSSAYS

SEQ ID NO: 487 - protein, 22 aa, unidentified
MDMRAPAGIFGFLLVLFPGYRS

SEQ ID NO: 488 - protein, 19 aa, unidentified
MTRLTVLALLAGLLASSRA

SEQ ID NO: 489 - protein, 19 aa, unidentified
MELGLSWIFLLAILKGVQC

SEQ ID NO: 490 - protein, 19 aa, unidentified
MELGLRWVFLVAILEGVQC

SEQ ID NO: 491 - protein, 19 aa, unidentified
MKHLWFFLLLVAAPRWVLS

SEQ ID NO: 492 - protein, 19 aa, unidentified
MDWTWRILFLVAAATGAHS

SEQ ID NO: 493 - protein, 19 aa, unidentified
MDWTWRFLFVVAAATGVQS

SEQ ID NO: 494 - protein, 19 aa, unidentified
MEFGLSWLFLVAILKGVQC

SEQ ID NO: 495 - protein, 19 aa, unidentified
MEFGLSWVFLVALFRGVQC

SEQ ID NO: 496 - protein, 26 aa, unidentified
MDLLHKNMKHLWFFLLLVAAPRWVLS

SEQ ID NO: 497 - protein, 22 aa, unidentified
MDMRVPAQLLGLLLLWLSGARC

SEQ ID NO: 498 - protein, 22 aa, unidentified
MKYLLPTAAAGLLLLAAQPAMA

SEQ ID NO: 499 - protein, 17 aa, unidentified
MGVKVLFALICIAVAEA

SEQ ID NO: 500 - protein, 18 aa, unidentified
MAFLWLLSCWALLGTTFG

SEQ ID NO: 501 - protein, 14 aa, unidentified
MQLLSCIALILALV

SEQ ID NO: 502 - protein, 15 aa, unidentified
MNLLLILTFVAAAVA

SEQ ID NO: 503 - protein, 16 aa, unidentified
MPLLLLLPLLWAGALA

SEQ ID NO: 504 - protein, 30 aa, unidentified
MDSKGSSQKGSRLLLLLVVSNLLLCQGVVS

SEQ ID NO: 505 - protein, 23 aa, unidentified
MDAMKRGLCCVLLLCGAVFVSPS

SEQ ID NO: 506 - protein, 16 aa, synthetic construct
MLLLLLLLLLLALALA

SEQ ID NO: 507 - protein, 21 aa, synthetic construct
MWWRLWWLLLLLLLLWPMVWA

SEQ ID NO: 508 - protein, 5 aa, Artificial Sequence
  REGION >5: note = The entire sequence of amino acids 1-5 can be repeated one or more times
GGGGS

SEQ ID NO: 509 - protein, 5 aa, Artificial Sequence
  REGION >5: note = The entire sequence of amino acids 1-5 can be repeated one or more times
EAAAK

SEQ ID NO: 510 - protein, 8 aa, Artificial Sequence
GGGGGGGG

SEQ ID NO: 511 - protein, 6 aa, Artificial Sequence
GGGGGG

SEQ ID NO: 512 - protein, 18 aa, Artificial Sequence
KESGSVSSEQLAQFRSLD

SEQ ID NO: 513 - protein, 14 aa, Artificial Sequence
EGKSSGSGSESKST

SEQ ID NO: 514 - protein, 12 aa, Artificial Sequence
GSAGSAAGSGEF

SEQ ID NO: 515 - protein, 46 aa, Artificial Sequence
AEAAAKEAAAKEAAAKEAAAKALEAEAAAKEAAAKEAAAKEAAAKA

SEQ ID NO: 516 - protein, 5 aa, Artificial Sequence
PAPAP

SEQ ID NO: 517 - protein, 12 aa, Artificial Sequence
AEAAAKEAAAKA

SEQ ID NO: 518 - skipped

SEQ ID NO: 519 - protein, 4 aa, Artificial Sequence
GGSG

SEQ ID NO: 520 - protein, 4 aa, Artificial Sequence
GSGS

SEQ ID NO: 521 - protein, 4 aa, Artificial Sequence
GGGS

SEQ ID NO: 522 - protein, 4 aa, Artificial Sequence
  REGION >4: note = The sequence of amino acids 2-4 can be repeated one or more times
SGGS

SEQ ID NO: 523 - protein, 7 aa, Artificial Sequence
GGGSGGG

SEQ ID NO: 524 - protein, 8 aa, Artificial Sequence
ESGGGGVT

SEQ ID NO: 525 - protein, 9 aa, Artificial Sequence
LESGGGGVT

SEQ ID NO: 526 - protein, 6 aa, Artificial Sequence
GRAQVT

SEQ ID NO: 527 - protein, 6 aa, Artificial Sequence
WRAQVT

SEQ ID NO: 528 - protein, 8 aa, Artificial Sequence
ARGRAQVT

SEQ ID NO: 529 - protein, 33 aa, Artificial Sequence
SGTTSGTTRLLSGHTCFTLTGLLGTLVTMGLLT

SEQ ID NO: 530 - protein, 26 aa, Artificial Sequence
SGTSPGLSAGATVGIMIGVLVGVALI

SEQ ID NO: 531 - protein, 24 aa, Artificial Sequence
SAPVLSAVATVGITIGVLARVALI

SEQ ID NO: 532 - protein, 24 aa, Artificial Sequence
SSPDLSAGTAVSIMIGVLAGMALI

SEQ ID NO: 533 - protein, 25 aa, Artificial Sequence
TLGGNSASYTFVSLLFSAVTLLLLC

SEQ ID NO: 534 - protein, 26 aa, Artificial Sequence
SGTSPGLSAGATVGIMIGVLVGVALI

SEQ ID NO: 535 - protein, 227 aa, Homo sapiens
DKTHTCPPCPAPELLGGPSVFLFPPKPKDTLMISRTPEVTCVVVDVSHEDPEVKFNWYVDGVEVHNAKTKPREEQYNSTYRVVSVLTVLHQDWLNGKEYKCKVSNKALPAPIEKTISKAKGQPREPQVYTLPPSRDELTKNQVSLTCLVKGFYPSDIAVEWESNGQPENNYKTTPPVLDSDGSFFLYSKLTVDKSRWQQGNVFSCSVMHEALHNHYTQKSLSLSPGK

SEQ ID NO: 536 - protein, 16 aa, Homo sapiens
DKTHTCPPCPAPELLG

SEQ ID NO: 537 - protein, 16 aa, Artificial Sequence
GSTHTCPPCPAPELLG

SEQ ID NO: 538 - protein, 21 aa, Artificial Sequence
EPKSCDKTHTCPPCPAPELLG

SEQ ID NO: 539 - protein, 24 aa, Artificial Sequence
EPKSCDKTHTCPPCPAPELLGGPS

SEQ ID NO: 540 - protein, 24 aa, Artificial Sequence
EPKSSDKTHTCPPCPAPELLGGPS

SEQ ID NO: 541 - protein, 24 aa, Artificial Sequence
EPKSSDKTHTCPPCPAPELLGGSS

SEQ ID NO: 542 - protein, 24 aa, Artificial Sequence
EPKSSGSTHTCPPCPAPELLGGSS

SEQ ID NO: 543 - protein, 19 aa, Artificial Sequence
DKTHTCPPCPAPELLGGPS

SEQ ID NO: 544 - protein, 19 aa, Artificial Sequence
DKTHTCPPCPAPELLGGSS

SEQ ID NO: 545 - protein, 227 aa, Homo sapiens; identical to SEQ ID NO: 535

SEQ ID NO: 546 - protein, 225 aa, Homo sapiens
DKTHTCPPCPAPELLGGPSVFLFPPKPKDTLMISRTPEVTCVVVDVSHEDPEVKFNWYVDGVEVHNAKTKPREEQYNSTYRVVSVLTVLHQDWLNGKEYKCKVSNKALPAPIEKTISKAKGQPREPQVYTLPPSRDELTKNQVSLTCLVKGFYPSDIAVEWESNGQPENNYKTTPPVLDSDGSFFLYSKLTVDKSRWQQGNVFSCSVMHEALHNHYTQKSLSLSP

SEQ ID NO: 547 - protein, 227 aa, Homo sapiens
DKTHTCPPCPAPELLGGPSVFLFPPKPKDTLMISRTPEVTCVVVDVSHEDPEVKFNWYVDGVEVHNAKTKPREEQYNSTYRVVSVLTVLHQDWLNGKEYKCKVSNKALPAPIEKTISKAKGQPREPQVYTLPPSRDEMTKNQVSLTCLVKGFYPSDIAVEWESNGQPENNYKTTPPVLDSDGSFFLYSKLTVDKSRWQQGNVFSCSVMHEALHNHYTQKSLSLSPGK

SEQ ID NO: 548 - protein, 227 aa, Homo sapiens
DKTHTCPPCPAPEAEGAPSVFLFPPKPKDTLMISRTPEVTCVVVDVSHEDPEVKFNWYVDGVEVHNAKTKPREEQYNSTYRVVSVLTVLHQDWLNGKEYKCKVSNKALPSSIEKTISKAKGQPREPQVYTLPPSREEMTKNQVSLTCLVKGFYPSDIAVEWESNGQPENNYKTTPPVLDSDGSFFLYSKLTVDKSRWQQGNVFSCSVMHEALHNHYTQKSLSLSPGK

SEQ ID NO: 549 - protein, 232 aa, Homo sapiens
EPKSSDKTHTCPPCPAPEAEGAPSVFLFPPKPKDTLMISRTPEVTCVVVDVSHEDPEVKFNWYVDGVEVHNAKTKPREEQYNSTYRVVSVLTVLHQDWLNGKEYKCKVSNKALPSSIEKTISKAKGQPREPQVYTLPPSREEMTKNQVSLTCLVKGFYPSDIAVEWESNGQPENNYKTTPPVLDSDGSFFLYSKLTVDKSRWQQGNVFSCSVMHEALHNHYTQKSLSLSPGK

SEQ ID NO: 550 - protein, 227 aa, Homo sapiens
DKTHTCPPCPAPELLGGPSVFLFPPKPKDTLMISRTPEVTCVVVDVSHEDPEVKFNWYVDGVEVHNAKTKPREEQYGSTYRVVSVLTVLHQDWLNGKEYKCKVSNKALPAPIEKTISKAKGQPREPQVYTLPPSRDELTKNQVSLTCLVKGFYPSDIAVEWESNGQPENNYKTTPPVLDSDGSFFLYSKLTVDKSRWQQGNVFSCSVMHEALHNHYTQKSLSLSPGK

SEQ ID NO: 551 - protein, 226 aa, Homo sapiens
DKTHTCPPCPAPELLGGPSVFLFPPKPKDTLMISRTPEVTCVVVDVSHEDPEVKFNWYVDGVEVHNAKTKPREEQYNSTYRVVSVLTVLHQDWLNGKEYKCKVSNKALPAPIEKTISKAKGQPREPQVYTLPPSRDELTKNQVSLTCLVKGFYPSDIAVEWESNGQPENNYKTTPPVLDSDGSFFLYSKLTVDKSRWQQGNVFSCSVMHEALHNHYTQKSLSLSPG

SEQ ID NO: 552 - protein, 227 aa, Homo sapiens
DKTHTCPPCPAPELLGGPSVFLFPPKPKDTLMISRTPEVTCVVVDVSHEDPEVKFNWYVDGVEVHNAKTKPREEQYQSTYRVVSVLTVLHQDWLNGKEYKCKVSNKALPAPIEKTISKAKGQPREPQVYTLPPSRDELTKNQVSLTCLVKGFYPSDIAVEWESNGQPENNYKTTPPVLDSDGSFFLYSKLTVDKSRWQQGNVFSCSVMHEALHNHYTQKSLSLSPGK

SEQ ID NO: 553 - protein, 227 aa, Homo sapiens
DKTHTCPPCPAPELLGGPSVFLFPPKPKDTLMISRTPEVTCVVVDVSHEDPEVKFNWYVDGVEVHNAKTKPREEQYSSTYRVVSVLTVLHQDWLNGKEYKCKVSNKALPAPIEKTISKAKGQPREPQVYTLPPSRDELTKNQVSLTCLVKGFYPSDIAVEWESNGQPENNYKTTPPVLDSDGSFFLYSKLTVDKSRWQQGNVFSCSVMHEALHNHYTQKSLSLSPGK

SEQ ID NO: 554 - protein, 227 aa, Homo sapiens
DKTHTCPPCPAPELLGGPSVFLFPPKPKDTLMISRTPEVTCVVVDVSHEDPEVKFNWYVDGVEVHNAKTKPREEQYASTYRVVSVLTVLHQDWLNGKEYKCKVSNKALPAPIEKTISKAKGQPREPQVYTLPPSRDELTKNQVSLTCLVKGFYPSDIAVEWESNGQPENNYKTTPPVLDSDGSFFLYSKLTVDKSRWQQGNVFSCSVMHEALHNHYTQKSLSLSPGK

SEQ ID NO: 555 - protein, 227 aa, Homo sapiens
DKTHTCPPCPAPELLGGPSVFLFPPKPKDTLMISRTPEVTCVVVDVSHEDPEVKFNWYVDGVEVHNAKTKPREEQYHSTYRVVSVLTVLHQDWLNGKEYKCKVSNKALPAPIEKTISKAKGQPREPQVYTLPPSRDELTKNQVSLTCLVKGFYPSDIAVEWESNGQPENNYKTTPPVLDSDGSFFLYSKLTVDKSRWQQGNVFSCSVMHEALHNHYTQKSLSLSPGK

SEQ ID NO: 556 - protein, 233 aa, Homo sapiens
DKRVESKYGPPCPSCPAPEFLGGPSVFLFPPKPKDTLMISRTPEVTCVVVDVSQEDPEVQFNWYVDGVEVHNAKTKPREEQFNSTYRVVSVLTVLHQDWLNGKEYKCKVSNKGLPSSIEKTISKAKGQPREPQVYTLPPSQEEMTKNQVSLTCLVKGFYPSDIAVEWESNGQPENNYKTTPPVLDSDGSFFLYSRLTVDKSRWQEGNVFSCSVMHEALHNHYTQKSLSLSLGK

SEQ ID NO: 557 - protein, 233 aa, Homo sapiens
DKRVESKYGPPCPPCPAPEFLGGPSVFLFPPKPKDTLMISRTPEVTCVVVDVSQEDPEVQFNWYVDGVEVHNAKTKPREEQFNSTYRVVSVLTVLHQDWLNGKEYKCKVSNKGLPSSIEKTISKAKGQPREPQVYTLPPSQEEMTKNQVSLTCLVKGFYPSDIAVEWESNGQPENNYKTTPPVLDSDGSFFLYSRLTVDKSRWQEGNVFSCSVMHEALHNHYTQKSLSLSLGK

SEQ ID NO: 558 - protein, 233 aa, Homo sapiens
SEPKSCDKTHTCPPCPAPEAAGGPSVFLFPPKPKDTLMISRTPEVTCVVVDVSHEDPEVKFNWYVDGVEVHNAKTKPREEQYNSTYRVVSVLTVLHQDWLNGKEYKCKVSNKALPAPIEKTISKAKGQPREPQVYTLPPSREEMTKNQVSLTCLVKGFYPSDIAVEWESNGQPENNYKTTPPVLDSDGSFFLYSKLTVDKSRWQQGNVFSCSVMHEALHNHYTQKSLSLSPGK

SEQ ID NO: 559 - protein, 585 aa, Homo sapiens [sequence omitted]

SEQ ID NO: 560 - protein, 6 aa, Homo sapiens
RGVFRR

SEQ ID NO: 561 - protein, 9 aa, Artificial Sequence
  VARIANT 2: note = The amino acids X at residue 2 can be Y, F or H
  VARIANT 3: note = The amino acids X at residue 3 can be Y or W
  VARIANT 5: note = The amino acids X at residue 5 can be A, S or R
  VARIANT 6: note = note = The amino acids X at residue 6 can be K or Y
GXXAXXWPG

SEQ ID NO: 562 - protein, 9 aa, Artificial Sequence
WTQPKNEHH

SEQ ID NO: 563 - protein, 9 aa, Artificial Sequence
HLKHTDAQP

SEQ ID NO: 564 - protein, 9 aa, Artificial Sequence
HDQDVLHAW

SEQ ID NO: 565 - protein, 9 aa, Artificial Sequence
KFHRQEWAD

SEQ ID NO: 566 - protein, 9 aa, Artificial Sequence
PEDFWDPEH

SEQ ID NO: 567 - protein, 9 aa, Artificial Sequence
VVRTTGHVV

SEQ ID NO: 568 - protein, 9 aa, Artificial Sequence
YWWFCTGQS

SEQ ID NO: 569 - protein, 9 aa, Artificial Sequence
IHHRQARSL

SEQ ID NO: 570 - protein, 9 aa, Artificial Sequence
SHRRRAYIW

SEQ ID NO: 571 - protein, 9 aa, Artificial Sequence
WDSHHWRAP

SEQ ID NO: 572 - protein, 8 aa, Artificial Sequence
DKRVKYGQ

SEQ ID NO: 573 - protein, 9 aa, Artificial Sequence
SDWVYALQL

SEQ ID NO: 574 - protein, 6 aa, Artificial Sequence
FWWFWY

SEQ ID NO: 575 - protein, 9 aa, Artificial Sequence
VRDWPWNTF

SEQ ID NO: 576 - protein, 9 aa, Artificial Sequence
QKKRDEDYI

SEQ ID NO: 577 - protein, 9 aa, Artificial Sequence
GVHEEPRKL

SEQ ID NO: 578 - protein, 9 aa, Artificial Sequence
EWWQKHWPS

SEQ ID NO: 579 - protein, 9 aa, Artificial Sequence
NFFQRRWPG

SEQ ID NO: 580 - protein, 9 aa, Artificial Sequence
DWWQAKWPH

SEQ ID NO: 581 - protein, 9 aa, Artificial Sequence
GIWQSRWPG

SEQ ID NO: 582 - protein, 9 aa, Artificial Sequence
GYWAAKWPG

SEQ ID NO: 583 - protein, 9 aa, Artificial Sequence
GFYADHWPG

SEQ ID NO: 584 - protein, 9 aa, Artificial Sequence
NWYQQRWPG

SEQ ID NO: 585 - protein, 9 aa, Artificial Sequence
GFYARHWPG

SEQ ID NO: 586 - protein, 9 aa, Artificial Sequence
DFWKAHWPG

SEQ ID NO: 587 - protein, 9 aa, Artificial Sequence
DFYSVRWPG

SEQ ID NO: 588 - protein, 9 aa, Artificial Sequence
YWAANHASK

SEQ ID NO: 589 - protein, 9 aa, Artificial Sequence
IKRLEHWEY

SEQ ID NO: 590 - protein, 9 aa, Artificial Sequence
EWDSPWSEN

SEQ ID NO: 591 - protein, 9 aa, Artificial Sequence
KHKNLRWPF

SEQ ID NO: 592 - protein, 9 aa, Artificial Sequence
RHFPKQTNW

SEQ ID NO: 593 - protein, 9 aa, Artificial Sequence
VWGPEYQHQ

SEQ ID NO: 594 - protein, 9 aa, Artificial Sequence
TWKNNGQDV

SEQ ID NO: 595 - protein, 9 aa, Artificial Sequence
ATWLNYYLP

SEQ ID NO: 596 - protein, 9 aa, Artificial Sequence
DQESLFLNN

SEQ ID NO: 597 - protein, 9 aa, Artificial Sequence
GFYAQHWPD

SEQ ID NO: 598 - protein, 9 aa, Artificial Sequence
GHYARYWPG

SEQ ID NO: 599 - protein, 9 aa, Artificial Sequence
GFWASKWPG

SEQ ID NO: 600 - protein, 9 aa, Artificial Sequence
GFWQRKWPN

SEQ ID NO: 601 - protein, 9 aa, Artificial Sequence
VWPADNDLK

SEQ ID NO: 602 - protein, 9 aa, Artificial Sequence
HWAWTSPGY

SEQ ID NO: 603 - protein, 9 aa, Artificial Sequence
NFFQRRWPG

SEQ ID NO: 604 - protein, 9 aa, Artificial Sequence
HHSHRLKGQ

SEQ ID NO: 605 - protein, 9 aa, Artificial Sequence
YQNTIFLSI

SEQ ID NO: 606 - protein, 9 aa, Artificial Sequence
FQDQFTWSQ

SEQ ID NO: 607 - protein, 9 aa, Artificial Sequence
GEPHWPWQA

SEQ ID NO: 608 - protein, 9 aa, Artificial Sequence
ADPRHPWVE

SEQ ID NO: 609 - protein, 9 aa, Artificial Sequence
FHKRFQSQG

SEQ ID NO: 610 - protein, 9 aa, Artificial Sequence
EWWQNRWPN

SEQ ID NO: 611 - protein, 9 aa, Artificial Sequence
EWYQTRWPG

SEQ ID NO: 612 - protein, 9 aa, Artificial Sequence
EFWQRHWPG

SEQ ID NO: 613 - protein, 9 aa, Artificial Sequence
KFYERHWPG

SEQ ID NO: 614 - protein, 9 aa, Artificial Sequence
GWWQRRWPG

SEQ ID NO: 615 - protein, 9 aa, Artificial Sequence
RFKYFAHYQ

SEQ ID NO: 616 - protein, 9 aa, Artificial Sequence
FHDFWHRRW

SEQ ID NO: 617 - protein, 9 aa, Artificial Sequence
DWYHYWWEV

SEQ ID NO: 618 - protein, 9 aa, Artificial Sequence
STRSIHVTT

SEQ ID NO: 619 - protein, 9 aa, Artificial Sequence
KQHHHYLDK

SEQ ID NO: 620 - protein, 9 aa, Artificial Sequence
HSAQDREIP

SEQ ID NO: 621 - protein, 9 aa, Artificial Sequence
WVQSGYNSQ

SEQ ID NO: 622 - protein, 9 aa, Artificial Sequence
AVFWGKWSD

SEQ ID NO: 623 - protein, 9 aa, Artificial Sequence
QSFDKPWTT

SEQ ID NO: 624 - protein, 9 aa, Artificial Sequence
HYPLKYSFE

SEQ ID NO: 625 - protein, 9 aa, Artificial Sequence
WHHPWHRNR

SEQ ID NO: 626 - protein, 9 aa, Artificial Sequence
DPWWAWVVW

SEQ ID NO: 627 - protein, 9 aa, Artificial Sequence
FDNQDLIQY

SEQ ID NO: 628 - protein, 9 aa, Artificial Sequence
EKKNWYKWD

SEQ ID NO: 629 - protein, 9 aa, Artificial Sequence
DRHKSRWGI

SEQ ID NO: 630 - protein, 9 aa, Artificial Sequence
LNPFTPSVT

SEQ ID NO: 631 - protein, 9 aa, Artificial Sequence
YKGALLNHD

SEQ ID NO: 632 - protein, 9 aa, Artificial Sequence
WKFRNTERG

SEQ ID NO: 633 - protein, 9 aa, Artificial Sequence
YKVHQSSGG

SEQ ID NO: 634 - protein, 9 aa, Artificial Sequence
FHPIAGRPW

SEQ ID NO: 635 - protein, 9 aa, Artificial Sequence
FPNTSYDLQ

SEQ ID NO: 636 - protein, 9 aa, Artificial Sequence
FAHYNLKSG

SEQ ID NO: 637 - protein, 9 aa, Artificial Sequence
WHNYGESSG

SEQ ID NO: 638 - protein, 9 aa, Artificial Sequence
KFYYADHQW

SEQ ID NO: 639 - protein, 9 aa, Artificial Sequence
YTHADPHSQ

SEQ ID NO: 640 - protein, 9 aa, Artificial Sequence
FGVPQLGAG

SEQ ID NO: 641 - protein, 9 aa, Artificial Sequence
YSGFPFAGF

SEQ ID NO: 642 - protein, 9 aa, Artificial Sequence
WFSWPYTPL

SEQ ID NO: 643 - protein, 9 aa, Artificial Sequence
YYHPSIQST

SEQ ID NO: 644 - protein, 9 aa, Artificial Sequence
FLGWKDTVV

SEQ ID NO: 645 - protein, 9 aa, Artificial Sequence
DWWKWWWAK

SEQ ID NO: 646 - protein, 9 aa, Artificial Sequence
NAGWPLVPE

SEQ ID NO: 647 - protein, 9 aa, Artificial Sequence
YALDPFGGK

SEQ ID NO: 648 - protein, 9 aa, Artificial Sequence
GYKFWGVSD

SEQ ID NO: 649 - protein, 9 aa, Artificial Sequence
QGKQYILLR

SEQ ID NO: 650 - protein, 9 aa, Artificial Sequence
YKRHSAHDY

SEQ ID NO: 651 - protein, 9 aa, Artificial Sequence
WAQKSKVHQ

SEQ ID NO: 652 - protein, 9 aa, Artificial Sequence
FTAVSKKDA

SEQ ID NO: 653 - protein, 9 aa, Artificial Sequence
WGDKENIWF

SEQ ID NO: 654 - protein, 9 aa, Artificial Sequence
WSGHPWVQK

SEQ ID NO: 655 - protein, 9 aa, Artificial Sequence
YADYPLSPK

SEQ ID NO: 656 - protein, 9 aa, Artificial Sequence
WKFRNTDRG

SEQ ID NO: 657 - protein, 9 aa, Artificial Sequence
QTVATHYHY

SEQ ID NO: 658 - protein, 9 aa, Artificial Sequence
WHAKHLLSH

SEQ ID NO: 659 - protein, 9 aa, Artificial Sequence
SGIKKADSV

SEQ ID NO: 660 - protein, 9 aa, Artificial Sequence
KANLINVKS

SEQ ID NO: 661 - protein, 9 aa, Artificial Sequence
WKSHVEVRS

SEQ ID NO: 662 - protein, 9 aa, Artificial Sequence
WVTQKYIIQ

SEQ ID NO: 663 - protein, 9 aa, Artificial Sequence
WEHAKDWPT

SEQ ID NO: 664 - protein, 9 aa, Artificial Sequence
FHSKVLDKA

SEQ ID NO: 665 - protein, 9 aa, Artificial Sequence
YGAQKQAVW

SEQ ID NO: 666 - protein, 9 aa, Artificial Sequence
FSASHFTSQ

SEQ ID NO: 667 - protein, 9 aa, Artificial Sequence
  source 1..9: note = X individually can be any amino acid
  VARIANT 1..2
  VARIANT 4
  VARIANT 6
  VARIANT 8
XXAXKXDXQ

SEQ ID NO: 668 - protein, 112 aa, Artificial Sequence
MIPRGLSEAKPATPEIQEIVDKVKPQLEEKTNETYGKLEAVQYKTQVLADWWQAKWPHSTNYYIKVRAGDNKYMHLKVFNGPYKVHQSSGGADRVLTGYQVDKNKDDELTGF

SEQ ID NO: 669 - protein, 112 aa, Artificial Sequence
MIPRGLSEAKPATPEIQEIVDKVKPQLEEKTNETYGKLEAVQYKTQVLAGYWAAKWPGSTNYYIKVRAGDNKYMHLKVFNGPFPNTSYDLQADRVLTGYQVDKNKDDELTGF

SEQ ID NO: 670 - protein, 112 aa, Artificial Sequence
MIPRGLSEAKPATPEIQEIVDKVKPQLEEKTNETYGKLEAVQYKTQVLANWYQQRWPGSTNYYIKVRAGDNKYMHLKVFNGPWHNYGESSGADRVLTGYQVDKNKDDELTGF

SEQ ID NO: 671 - protein, 112 aa, Artificial Sequence
MIPRGLSEAKPATPEIQEIVDKVKPQLEEKTNETYGKLEAVQYKTQVLAVWGPEYQHQSTNYYIKVRAGDNKYMHLKVFNGPNAGWPLVPEADRVLTGYQVDKNKDDELTGF

SEQ ID NO: 672 - protein, 112 aa, Artificial Sequence
MIPRGLSEAKPATPEIQEIVDKVKPQLEEKTNETYGKLEAVQYKTQVLAGHYARYWPGSTNYYIKVRAGDNKYMHLKVFNGPWAQKSKVHQADRVLTGYQVDKNKDDELTGF

SEQ ID NO: 673 - protein, 112 aa, Artificial Sequence
MIPRGLSEAKPATPEIQEIVDKVKPQLEEKTNETYGKLEAVQYKTQVLAGFWASKWPGSTNYYIKVRAGDNKYMHLKVFNGPFTAVSKKDAADRVLTGYQVDKNKDDELTGF

SEQ ID NO: 674 - protein, 112 aa, Artificial Sequence
MIPRGLSEAKPATPEIQEIVDKVKPQLEEKTNETYGKLEAVQYKTQVLANFFQRRWPGSTNYYIKVRAGDNKYMHLKVFNGPWKFRNTDRGADRVLTGYQVDKNKDDELTGF

SEQ ID NO: 675 - DNA, 12 bp, Artificial Sequence
  source 1..12: mol_type = other DNA
accgttgccggt

SEQ ID NO: 676 - skipped

SEQ ID NO: 677 - protein, 251 aa, Artificial Sequence
IPGGLSEAKPATPEIQEIVDKVKPQLEEKTGETYGKLEAVQYKTQVVHYYVHYNDQGTNYYIKVRAGDNKYMHLKVFKSLWGENLFAKWEDLVLTGYQVDKNKDDELTGFGGGGSGGGGSGGGGSGGGGSGGGGSGGGGSMIPGGLSEAKPATPEIQEIVDKVKPQLEEKTGETYGKLEAVQYKTQVVHYYVHYNDQGTNYYIKVRAGDNKYMHLKVFKSLWGENLFAKWEDLVLTGYQVDKNKDDELTGF

SEQ ID NO: 678 - protein, 392 aa, Artificial Sequence
IPGGLSEAKPATPEIQEIVDKVKPQLEEKTGETYGKLEAVQYKTQVVHYYVHYNDQGTNYYIKVRAGDNKYMHLKVFKSLWGENLFAKWEDLVLTGYQVDKNKDDELTGFGGGGSGGGGSGGGGSGGGGSGGGGSGGGGSMIPGGLSEAKPATPEIQEIVDKVKPQLEEKTGETYGKLEAVQYKTQVVHYYVHYNDQGTNYYIKVRAGDNKYMHLKVFKSLWGENLFAKWEDLVLTGYQVDKNKDDELTGFGGGGSGGGGSGGGGSGGGGSGGGGSGGGGSMIPGGLSEAKPATPEIQEIVDKVKPQLEEKTGETYGKLEAVQYKTQVVHYYVHYNDQGTNYYIKVRAGDNKYMHLKVFKSLWGENLFAKWEDLVLTGYQVDKNKDDELTGF

SEQ ID NO: 679 - protein, 251 aa, Artificial Sequence
IPGGLSEAKPATPEIQEIVDKVKPQLEEKTGETYGKLEAVQYKTQVVHHAYAAVYVGTNYYIKVRAGDNKYMHLKVFKSLPYWYRKYPDEDLVLTGYQVDKNKDDELTGFGGGGSGGGGSGGGGSGGGGSGGGGSGGGGSMIPGGLSEAKPATPEIQEIVDKVKPQLEEKTGETYGKLEAVQYKTQVVHHAYAAVYVGTNYYIKVRAGDNKYMHLKVFKSLPYWYRKYPDEDLVLTGYQVDKNKDDELTGF

SEQ ID NO: 680 - protein, 392 aa, Artificial Sequence
IPGGLSEAKPATPEIQEIVDKVKPQLEEKTGETYGKLEAVQYKTQVVHHAYAAVYVGTNYYIKVRAGDNKYMHLKVFKSLPYWYRKYPDEDLVLTGYQVDKNKDDELTGFGGGGSGGGGSGGGGSGGGGSGGGGSGGGGSMIPGGLSEAKPATPEIQEIVDKVKPQLEEKTGETYGKLEAVQYKTQVVHHAYAAVYVGTNYYIKVRAGDNKYMHLKVFKSLPYWYRKYPDEDLVLTGYQVDKNKDDELTGFGGGGSGGGGSGGGGSGGGGSGGGGSGGGGSMIPGGLSEAKPATPEIQEIVDKVKPQLEEKTGETYGKLEAVQYKTQVVHHAYAAVYVGTNYYIKVRAGDNKYMHLKVFKSLPYWYRKYPDEDLVLTGYQVDKNKDDELTGF

SEQ ID NO: 681 - protein, 394 aa, Artificial Sequence
IPGGLSEAKPATPEIQEIVDKVKPQLEEKTGETYGKLEAVQYKTQVVHYYVHYNDQGTNYYIKVRAGDNKYMHLKVFKSLWGENLFAKWEDLVLTGYQVDKNKDDELTGFAEAAAKEAAAKEAAAKEAAAKEAAAKEAAAKMIPGGLSEAKPATPEIQEIVDKVKPQLEEKTGETYGKLEAVQYKTQVVHYYVHYNDQGTNYYIKVRAGDNKYMHLKVFKSLWGENLFAKWEDLVLTGYQVDKNKDDELTGFAEAAAKEAAAKEAAAKEAAAKEAAAKEAAAKMIPGGLSEAKPATPEIQEIVDKVKPQLEEKTGETYGKLEAVQYKTQVVHYYVHYNDQGTNYYIKVRAGDNKYMHLKVFKSLWGENLFAKWEDLVLTGYQVDKNKDDELTGF

SEQ ID NO: 682 - protein, 394 aa, Artificial Sequence
IPGGLSEAKPATPEIQEIVDKVKPQLEEKTGETYGKLEAVQYKTQVVFTYQISYTVGTNYYIKVRAGDNKYMHLKVFKSLRWRYPARKPEDLVLTGYQVDKNKDDELTGFAEAAAKEAAAKEAAAKEAAAKEAAAKEAAAKMIPGGLSEAKPATPEIQEIVDKVKPQLEEKTGETYGKLEAVQYKTQVVFTYQISYTVGTNYYIKVRAGDNKYMHLKVFKSLRWRYPARKPEDLVLTGYQVDKNKDDELTGFAEAAAKEAAAKEAAAKEAAAKEAAAKEAAAKMIPGGLSEAKPATPEIQEIVDKVKPQLEEKTGETYGKLEAVQYKTQVVFTYQISYTVGTNYYIKVRAGDNKYMHLKVFKSLRWRYPARKPEDLVLTGYQVDKNKDDELTGF

SEQ ID NO: 683 - protein, 394 aa, Artificial Sequence
IPGGLSEAKPATPEIQEIVDKVKPQLEEKTGETYGKLEAVQYKTQVVHIPALKVHAGTNYYIKVRAGDNKYMHLKVFKSLPYWYRHDQEEDLVLTGYQVDKNKDDELTGFAEAAAKEAAAKEAAAKEAAAKEAAAKEAAAKMIPGGLSEAKPATPEIQEIVDKVKPQLEEKTGETYGKLEAVQYKTQVVHIPALKVHAGTNYYIKVRAGDNKYMHLKVFKSLPYWYRHDQEEDLVLTGYQVDKNKDDELTGFAEAAAKEAAAKEAAAKEAAAKEAAAKEAAAKMIPGGLSEAKPATPEIQEIVDKVKPQLEEKTGETYGKLEAVQYKTQVVHIPALKVHAGTNYYIKVRAGDNKYMHLKVFKSLPYWYRHDQEEDLVLTGYQVDKNKDDELTGF

SEQ ID NO: 684 - protein, 394 aa, Artificial Sequence
IPGGLSEAKPATPEIQEIVDKVKPQLEEKTGETYGKLEAVQYKTQVVHHAYAAVYVGTNYYIKVRAGDNKYMHLKVFKSLPYWYRKYPDEDLVLTGYQVDKNKDDELTGFAEAAAKEAAAKEAAAKEAAAKEAAAKEAAAKMIPGGLSEAKPATPEIQEIVDKVKPQLEEKTGETYGKLEAVQYKTQVVHHAYAAVYVGTNYYIKVRAGDNKYMHLKVFKSLPYWYRKYPDEDLVLTGYQVDKNKDDELTGFAEAAAKEAAAKEAAAKEAAAKEAAAKEAAAKMIPGGLSEAKPATPEIQEIVDKVKPQLEEKTGETYGKLEAVQYKTQVVHHAYAAVYVGTNYYIKVRAGDNKYMHLKVFKSLPYWYRKYPDEDLVLTGYQVDKNKDDELTGF

SEQ ID NO: 685 - protein, 391 aa, Artificial Sequence
IPGGLSEAKPATPEIQEIVDKVKPQLEEKTGETYGKLEAVQYKTQVVYDELYHEKAGTNYYIKVRAGDNKYMHLKVFKSLEYKFRNLEEDLVLTGYQVDKNKDDELTGFAEAAAKEAAAKEAAAKEAAAKEAAAKEAAAKMIPGGLSEAKPATPEIQEIVDKVKPQLEEKTGETYGKLEAVQYKTQVVYDELYHEKAGTNYYIKVRAGDNKYMHLKVFKSLEYKFRNLEEDLVLTGYQVDKNKDDELTGFAEAAAKEAAAKEAAAKEAAAKEAAAKEAAAKMIPGGLSEAKPATPEIQEIVDKVKPQLEEKTGETYGKLEAVQYKTQVVYDELYHEKAGTNYYIKVRAGDNKYMHLKVFKSLEYKFRNLEEDLVLTGYQVDKNKDDELTGF

SEQ ID NO: 686 - protein, 394 aa, Artificial Sequence
IPGGLSEAKPATPEIQEIVDKVKPQLEEKTGETYGKLEAVQYKTQVVVDQVWSENAGTNYYIKVRAGDNKYMHLKVFKSLPYLWRKHAVEDLVLTGYQVDKNKDDELTGFAEAAAKEAAAKEAAAKEAAAKEAAAKEAAAKMIPGGLSEAKPATPEIQEIVDKVKPQLEEKTGETYGKLEAVQYKTQVVVDQVWSENAGTNYYIKVRAGDNKYMHLKVFKSLPYLWRKHAVEDLVLTGYQVDKNKDDELTGFAEAAAKEAAAKEAAAKEAAAKEAAAKEAAAKMIPGGLSEAKPATPEIQEIVDKVKPQLEEKTGETYGKLEAVQYKTQVVVDQVWSENAGTNYYIKVRAGDNKYMHLKVFKSLPYLWRKHAVEDLVLTGYQVDKNKDDELTGF

SEQ ID NO: 687 - protein, 394 aa, Artificial Sequence
IPGGLSEAKPATPEIQEIVDKVKPQLEEKTGETYGKLEAVQYKTQVVGDSYWEYVSGTNYYIKVRAGDNKYMHLKVFKSLPYRWRPDHAEDLVLTGYQVDKNKDDELTGFAEAAAKEAAAKEAAAKEAAAKEAAAKEAAAKMIPGGLSEAKPATPEIQEIVDKVKPQLEEKTGETYGKLEAVQYKTQVVGDSYWEYVSGTNYYIKVRAGDNKYMHLKVFKSLPYRWRPDHAEDLVLTGYQVDKNKDDELTGFAEAAAKEAAAKEAAAKEAAAKEAAAKEAAAKMIPGGLSEAKPATPEIQEIVDKVKPQLEEKTGETYGKLEAVQYKTQVVGDSYWEYVSGTNYYIKVRAGDNKYMHLKVFKSLPYRWRPDHAEDLVLTGYQVDKNKDDELTGF

SEQ ID NO: 688 - protein, 394 aa, Artificial Sequence
IPGGLSEAKPATPEIQEIVDKVKPQLEEKTGETYGKLEAVQYKTQVVLDGLYHVNSGTNYYIKVRAGDNKYMHLKVFKSLFYYYRSEPTEDLVLTGYQVDKNKDDELTGFAEAAAKEAAAKEAAAKEAAAKEAAAKEAAAKMIPGGLSEAKPATPEIQEIVDKVKPQLEEKTGETYGKLEAVQYKTQVVLDGLYHVNSGTNYYIKVRAGDNKYMHLKVFKSLFYYYRSEPTEDLVLTGYQVDKNKDDELTGFAEAAAKEAAAKEAAAKEAAAKEAAAKEAAAKMIPGGLSEAKPATPEIQEIVDKVKPQLEEKTGETYGKLEAVQYKTQVVLDGLYHVNSGTNYYIKVRAGDNKYMHLKVFKSLFYYYRSEPTEDLVLTGYQVDKNKDDELTGF

SEQ ID NO: 689 - protein, 394 aa, Artificial Sequence
IPGGLSEAKPATPEIQEIVDKVKPQLEEKTGETYGKLEAVQYKTQVVKTWEDTVVAGTNYYIKVRAGDNKYMHLKVFKSLEYLYRPLNPEDLVLTGYQVDKNKDDELTGFAEAAAKEAAAKEAAAKEAAAKEAAAKEAAAKMIPGGLSEAKPATPEIQEIVDKVKPQLEEKTGETYGKLEAVQYKTQVVKTWEDTVVAGTNYYIKVRAGDNKYMHLKVFKSLEYLYRPLNPEDLVLTGYQVDKNKDDELTGFAEAAAKEAAAKEAAAKEAAAKEAAAKEAAAKMIPGGLSEAKPATPEIQEIVDKVKPQLEEKTGETYGKLEAVQYKTQVVKTWEDTVVAGTNYYIKVRAGDNKYMHLKVFKSLEYLYRPLNPEDLVLTGYQVDKNKDDELTGF

SEQ ID NO: 690 - protein, 533 aa, Artificial Sequence
IPGGLSEAKPATPEIQEIVDKVKPQLEEKTGETYGKLEAVQYKTQVVHYYVHYNDQGTNYYIKVRAGDNKYMHLKVFKSLWGENLFAKWEDLVLTGYQVDKNKDDELTGFGGGGSGGGGSGGGGSGGGGSGGGGSGGGGSMIPGGLSEAKPATPEIQEIVDKVKPQLEEKTGETYGKLEAVQYKTQVVHYYVHYNDQGTNYYIKVRAGDNKYMHLKVFKSLWGENLFAKWEDLVLTGYQVDKNKDDELTGFGGGGSGGGGSGGGGSGGGGSGGGGSGGGGSMIPGGLSEAKPATPEIQEIVDKVKPQLEEKTGETYGKLEAVQYKTQVVHYYVHYNDQGTNYYIKVRAGDNKYMHLKVFKSLWGENLFAKWEDLVLTGYQVDKNKDDELTGFGGGGSGGGGSGGGGSGGGGSGGGGSGGGGSMIPGGLSEAKPATPEIQEIVDKVKPQLEEKTGETYGKLEAVQYKTQVVHYYVHYNDQGTNYYIKVRAGDNKYMHLKVFKSLWGENLFAKWEDLVLTGYQVDKNKDDELTGF

SEQ ID NO: 691 - protein, 536 aa, Artificial Sequence
IPGGLSEAKPATPEIQEIVDKVKPQLEEKTGETYGKLEAVQYKTQVVHYYVHYNDQGTNYYIKVRAGDNKYMHLKVFKSLWGENLFAKWEDLVLTGYQVDKNKDDELTGFAEAAAKEAAAKEAAAKEAAAKEAAAKEAAAKMIPGGLSEAKPATPEIQEIVDKVKPQLEEKTGETYGKLEAVQYKTQVVHYYVHYNDQGTNYYIKVRAGDNKYMHLKVFKSLWGENLFAKWEDLVLTGYQVDKNKDDELTGFAEAAAKEAAAKEAAAKEAAAKEAAAKEAAAKMIPGGLSEAKPATPEIQEIVDKVKPQLEEKTGETYGKLEAVQYKTQVVHYYVHYNDQGTNYYIKVRAGDNKYMHLKVFKSLWGENLFAKWEDLVLTGYQVDKNKDDELTGFAEAAAKEAAAKEAAAKEAAAKEAAAKEAAAKMIPGGLSEAKPATPEIQEIVDKVKPQLEEKTGETYGKLEAVQYKTQVVHYYVHYNDQGTNYYIKVRAGDNKYMHLKVFKSLWGENLFAKWEDLVLTGYQVDKNKDDELTGF

SEQ ID NO: 692 - protein, 534 aa, Artificial Sequence
IPGGLSEAKPATPEIQEIVDKVKPQLEEKTGETYGKLEAVQYKTQVVHYYVHYNDQGTNYYIKVRAGDNKYMHLKVFKSLWGENLFAKWEDLVLTGYQVDKNKDDELTGFGGGGSGGGGSGGGGSGGGGSGGGGSGGGGSMIPGGLSEAKPATPEIQEIVDKVKPQLEEKTGETYGKLEAVQYKTQVVHYYVHYNDQGTNYYIKVRAGDNKYMHLKVFKSLWGENLFAKWEDLVLTGYQVDKNKDDELTGFGGGGSGGGGSGGGGSGGGGSGGGGSGGGGSMIPGGLSEAKPATPEIQEIVDKVKPQLEEKTGETYGKLEAVQYKTQVVHYYVHYNDQGTNYYIKVRAGDNKYMHLKVFKSLWGENLFAKWEDLVLTGYQVDKNKDDELTGFGGGGSGGGGSGGGGSGGGGSGGGGSGGGGSMIPRGLSEAKPATPEIQEIVDKVKPQLEEKTGETYGKLEAVQYKTQVLANFFQRRWPGSTNYYIKVRAGDNKYMHLKVFNGPWKFRNTDRGADRVLTGYQVDKNKDDELTGF

SEQ ID NO: 693 - protein, 675 aa, Artificial Sequence
IPGGLSEAKPATPEIQEIVDKVKPQLEEKTGETYGKLEAVQYKTQVVHYYVHYNDQGTNYYIKVRAGDNKYMHLKVFKSLWGENLFAKWEDLVLTGYQVDKNKDDELTGFGGGGSGGGGSGGGGSGGGGSGGGGSGGGGSMIPGGLSEAKPATPEIQEIVDKVKPQLEEKTGETYGKLEAVQYKTQVVHYYVHYNDQGTNYYIKVRAGDNKYMHLKVFKSLWGENLFAKWEDLVLTGYQVDKNKDDELTGFGGGGSGGGGSGGGGSGGGGSGGGGSGGGGSMIPGGLSEAKPATPEIQEIVDKVKPQLEEKTGETYGKLEAVQYKTQVVHYYVHYNDQGTNYYIKVRAGDNKYMHLKVFKSLWGENLFAKWEDLVLTGYQVDKNKDDELTGFGGGGSGGGGSGGGGSGGGGSGGGGSGGGGSMIPGGLSEAKPATPEIQEIVDKVKPQLEEKTGETYGKLEAVQYKTQVVHYYVHYNDQGTNYYIKVRAGDNKYMHLKVFKSLWGENLFAKWEDLVLTGYQVDKNKDDELTGFGGGGSGGGGSGGGGSGGGGSGGGGSGGGGSMIPRGLSEAKPATPEIQEIVDKVKPQLEEKTGETYGKLEAVQYKTQVLANFFQRRWPGSTNYYIKVRAGDNKYMHLKVFNGPWKFRNTDRGADRVLTGYQVDKNKDDELTGF

SEQ ID NO: 694 - protein, 537 aa, Artificial Sequence
IPGGLSEAKPATPEIQEIVDKVKPQLEEKTGETYGKLEAVQYKTQVVHYYVHYNDQGTNYYIKVRAGDNKYMHLKVFKSLWGENLFAKWEDLVLTGYQVDKNKDDELTGFAEAAAKEAAAKEAAAKEAAAKEAAAKEAAAKMIPGGLSEAKPATPEIQEIVDKVKPQLEEKTGETYGKLEAVQYKTQVVHYYVHYNDQGTNYYIKVRAGDNKYMHLKVFKSLWGENLFAKWEDLVLTGYQVDKNKDDELTGFAEAAAKEAAAKEAAAKEAAAKEAAAKEAAAKMIPGGLSEAKPATPEIQEIVDKVKPQLEEKTGETYGKLEAVQYKTQVVHYYVHYNDQGTNYYIKVRAGDNKYMHLKVFKSLWGENLFAKWEDLVLTGYQVDKNKDDELTGFAEAAAKEAAAKEAAAKEAAAKEAAAKEAAAKMIPRGLSEAKPATPEIQEIVDKVKPQLEEKTGETYGKLEAVQYKTQVLANFFQRRWPGSTNYYIKVRAGDNKYMHLKVFNGPWKFRNTDRGADRVLTGYQVDKNKDDELTGF

SEQ ID NO: 695 - protein, 679 aa, Artificial Sequence
IPGGLSEAKPATPEIQEIVDKVKPQLEEKTGETYGKLEAVQYKTQVVHYYVHYNDQGTNYYIKVRAGDNKYMHLKVFKSLWGENLFAKWEDLVLTGYQVDKNKDDELTGFAEAAAKEAAAKEAAAKEAAAKEAAAKEAAAKMIPGGLSEAKPATPEIQEIVDKVKPQLEEKTGETYGKLEAVQYKTQVVHYYVHYNDQGTNYYIKVRAGDNKYMHLKVFKSLWGENLFAKWEDLVLTGYQVDKNKDDELTGFAEAAAKEAAAKEAAAKEAAAKEAAAKEAAAKMIPGGLSEAKPATPEIQEIVDKVKPQLEEKTGETYGKLEAVQYKTQVVHYYVHYNDQGTNYYIKVRAGDNKYMHLKVFKSLWGENLFAKWEDLVLTGYQVDKNKDDELTGFAEAAAKEAAAKEAAAKEAAAKEAAAKEAAAKMIPGGLSEAKPATPEIQEIVDKVKPQLEEKTGETYGKLEAVQYKTQVVHYYVHYNDQGTNYYIKVRAGDNKYMHLKVFKSLWGENLFAKWEDLVLTGYQVDKNKDDELTGFAEAAAKEAAAKEAAAKEAAAKEAAAKEAAAKMIPRGLSEAKPATPEIQEIVDKVKPQLEEKTGETYGKLEAVQYKTQVLANFFQRRWPGSTNYYIKVRAGDNKYMHLKVFNGPWKFRNTDRGADRVLTGYQVDKNKDDELTGF

SEQ ID NO: 696 - protein, 566 aa, Artificial Sequence
IPGGLSEAKPATPEIQEIVDKVKPQLEEKTGETYGKLEAVQYKTQVVHYYVHYNDQGTNYYIKVRAGDNKYMHLKVFKSLWGENLFAKWEDLVLTGYQVDKNKDDELTGFAEAAAKEAAAKEAAAKEAAAKEAAAKEAAAKMIPGGLSEAKPATPEIQEIVDKVKPQLEEKTGETYGKLEAVQYKTQVVHYYVHYNDQGTNYYIKVRAGDNKYMHLKVFKSLWGENLFAKWEDLVLTGYQVDKNKDDELTGFAEAAAKEAAAKEAAAKEAAAKEAAAKEAAAKMIPGGLSEAKPATPEIQEIVDKVKPQLEEKTGETYGKLEAVQYKTQVVHYYVHYNDQGTNYYIKVRAGDNKYMHLKVFKSLWGENLFAKWEDLVLTGYQVDKNKDDELTGFGGGGSGGGGSGGGGSGGGGSGGGGSGGGGSGGGGSGGGGSGGGGSGGGGSGGGGSGGGGSMIPRGLSEAKPATPEIQEIVDKVKPQLEEKTGETYGKLEAVQYKTQVLANFFQRRWPGSTNYYIKVRAGDNKYMHLKVFNGPWKFRNTDRGADRVLTGYQVDKNKDDELTGF

SEQ ID NO: 697 - protein, 534 aa, Artificial Sequence
IPGGLSEAKPATPEIQEIVDKVKPQLEEKTGETYGKLEAVQYKTQVVHYYVHYNDQGTNYYIKVRAGDNKYMHLKVFKSLWGENLFAKWEDLVLTGYQVDKNKDDELTGFGGGGSGGGGSGGGGSMIPGGLSEAKPATPEIQEIVDKVKPQLEEKTGETYGKLEAVQYKTQVVHYYVHYNDQGTNYYIKVRAGDNKYMHLKVFKSLWGENLFAKWEDLVLTGYQVDKNKDDELTGFGGGGSGGGGSGGGGSMIPGGLSEAKPATPEIQEIVDKVKPQLEEKTGETYGKLEAVQYKTQVVHYYVHYNDQGTNYYIKVRAGDNKYMHLKVFKSLWGENLFAKWEDLVLTGYQVDKNKDDELTGFGGGGSGGGGSGGGGSGGGGSGGGGSGGGGSGGGGSGGGGSGGGGSGGGGSGGGGSGGGGSMIPRGLSEAKPATPEIQEIVDKVKPQLEEKTGETYGKLEAVQYKTQVLANFFQRRWPGSTNYYIKVRAGDNKYMHLKVFNGPWKFRNTDRGADRVLTGYQVDKNKDDELTGF

SEQ ID NO: 698 - protein, 535 aa, Artificial Sequence
IPGGLSEAKPATPEIQEIVDKVKPQLEEKTGETYGKLEAVQYKTQVVHYYVHYNDQGTNYYIKVRAGDNKYMHLKVFKSLWGENLFAKWEDLVLTGYQVDKNKDDELTGFGGGGSGGGGSGGGGSMIPGGLSEAKPATPEIQEIVDKVKPQLEEKTGETYGKLEAVQYKTQVVHYYVHYNDQGTNYYIKVRAGDNKYMHLKVFKSLWGENLFAKWEDLVLTGYQVDKNKDDELTGFGGGGSGGGGSGGGGSMIPGGLSEAKPATPEIQEIVDKVKPQLEEKTGETYGKLEAVQYKTQVVHYYVHYNDQGTNYYIKVRAGDNKYMHLKVFKSLWGENLFAKWEDLVLTGYQVDKNKDDELTGFAEAAAKEAAAKEAAAKEAAAKEAAAKEAAAKEAAAKEAAAKEAAAKEAAAKEAAAKEAAAKMIPRGLSEAKPATPEIQEIVDKVKPQLEEKTGETYGKLEAVQYKTQVLANFFQRRWPGSTNYYIKVRAGDNKYMHLKVFNGPWKFRNTDRGADRVLTGYQVDKNKDDELTGF

SEQ ID NO: 699 - protein, 536 aa, Artificial Sequence
IPGGLSEAKPATPEIQEIVDKVKPQLEEKTGETYGKLEAVQYKTQVVHYYVHYNDQGTNYYIKVRAGDNKYMHLKVFKSLWGENLFAKWEDLVLTGYQVDKNKDDELTGFAEAAAKEAAAKEAAAKMIPGGLSEAKPATPEIQEIVDKVKPQLEEKTGETYGKLEAVQYKTQVVHYYVHYNDQGTNYYIKVRAGDNKYMHLKVFKSLWGENLFAKWEDLVLTGYQVDKNKDDELTGFAEAAAKEAAAKEAAAKMIPGGLSEAKPATPEIQEIVDKVKPQLEEKTGETYGKLEAVQYKTQVVHYYVHYNDQGTNYYIKVRAGDNKYMHLKVFKSLWGENLFAKWEDLVLTGYQVDKNKDDELTGFGGGGSGGGGSGGGGSGGGGSGGGGSGGGGSGGGGSGGGGSGGGGSGGGGSGGGGSGGGGSMIPRGLSEAKPATPEIQEIVDKVKPQLEEKTGETYGKLEAVQYKTQVLANFFQRRWPGSTNYYIKVRAGDNKYMHLKVFNGPWKFRNTDRGADRVLTGYQVDKNKDDELTGF

SEQ ID NO: 700 - protein, 537 aa, Artificial Sequence
IPGGLSEAKPATPEIQEIVDKVKPQLEEKTGETYGKLEAVQYKTQVVHYYVHYNDQGTNYYIKVRAGDNKYMHLKVFKSLWGENLFAKWEDLVLTGYQVDKNKDDELTGFAEAAAKEAAAKEAAAKMIPGGLSEAKPATPEIQEIVDKVKPQLEEKTGETYGKLEAVQYKTQVVHYYVHYNDQGTNYYIKVRAGDNKYMHLKVFKSLWGENLFAKWEDLVLTGYQVDKNKDDELTGFAEAAAKEAAAKEAAAKMIPGGLSEAKPATPEIQEIVDKVKPQLEEKTGETYGKLEAVQYKTQVVHYYVHYNDQGTNYYIKVRAGDNKYMHLKVFKSLWGENLFAKWEDLVLTGYQVDKNKDDELTGFAEAAAKEAAAKEAAAKEAAAKEAAAKEAAAKEAAAKEAAAKEAAAKEAAAKEAAAKEAAAKMIPRGLSEAKPATPEIQEIVDKVKPQLEEKTGETYGKLEAVQYKTQVLANFFQRRWPGSTNYYIKVRAGDNKYMHLKVFNGPWKFRNTDRGADRVLTGYQVDKNKDDELTGF

SEQ ID NO: 701 - protein, 537 aa, Artificial Sequence
IPGGLSEAKPATPEIQEIVDKVKPQLEEKTGETYGKLEAVQYKTQVVGGGGGGGGGGTNYYIKVRAGDNKYMHLKVFKSLGGGGGGGGGEDLVLTGYQVDKNKDDELTGFAEAAAKEAAAKEAAAKEAAAKEAAAKEAAAKMIPGGLSEAKPATPEIQEIVDKVKPQLEEKTGETYGKLEAVQYKTQVVGGGGGGGGGGTNYYIKVRAGDNKYMHLKVFKSLGGGGGGGGGEDLVLTGYQVDKNKDDELTGFAEAAAKEAAAKEAAAKEAAAKEAAAKEAAAKMIPGGLSEAKPATPEIQEIVDKVKPQLEEKTGETYGKLEAVQYKTQVVGGGGGGGGGGTNYYIKVRAGDNKYMHLKVFKSLGGGGGGGGGEDLVLTGYQVDKNKDDELTGFAEAAAKEAAAKEAAAKEAAAKEAAAKEAAAKMIPRGLSEAKPATPEIQEIVDKVKPQLEEKTGETYGKLEAVQYKTQVLANFFQRRWPGSTNYYIKVRAGDNKYMHLKVFNGPWKFRNTDRGADRVLTGYQVDKNKDDELTGF

SEQ ID NO: 702 - protein, 679 aa, Artificial Sequence
IPGGLSEAKPATPEIQEIVDKVKPQLEEKTGETYGKLEAVQYKTQVVGGGGGGGGGGTNYYIKVRAGDNKYMHLKVFKSLGGGGGGGGGEDLVLTGYQVDKNKDDELTGFAEAAAKEAAAKEAAAKEAAAKEAAAKEAAAKMIPGGLSEAKPATPEIQEIVDKVKPQLEEKTGETYGKLEAVQYKTQVVGGGGGGGGGGTNYYIKVRAGDNKYMHLKVFKSLGGGGGGGGGEDLVLTGYQVDKNKDDELTGFAEAAAKEAAAKEAAAKEAAAKEAAAKEAAAKMIPRGLSEAKPATPEIQEIVDKVKPQLEEKTGETYGKLEAVQYKTQVLANFFQRRWPGSTNYYIKVRAGDNKYMHLKVFNGPWKFRNTDRGADRVLTGYQVDKNKDDELTGFAEAAAKEAAAKEAAAKEAAAKEAAAKEAAAKMIPGGLSEAKPATPEIQEIVDKVKPQLEEKTGETYGKLEAVQYKTQVVGGGGGGGGGGTNYYIKVRAGDNKYMHLKVFKSLGGGGGGGGGEDLVLTGYQVDKNKDDELTGFAEAAAKEAAAKEAAAKEAAAKEAAAKEAAAKMIPGGLSEAKPATPEIQEIVDKVKPQLEEKTGETYGKLEAVQYKTQVVGGGGGGGGGGTNYYIKVRAGDNKYMHLKVFKSLGGGGGGGGGEDLVLTGYQVDKNKDDELTGF

SEQ ID NO: 703 - DNA, 753 bp, Artificial Sequence
  source 1..753: mol_type = genomic DNA
atccctggcggactgtcggaagccaagccggccactccggaaatccaggagattgtggataaggtcaagcctcagctggaggaaaagacgggcgaaacttacgggaagctcgaggccgtgcaatacaagacccaggtcgtgcactattacgtgcattacaacgaccaggggaccaactactacattaaggtccgcgctggagacaacaagtatatgcacctgaaagtgttcaagtcgctgtggggggagaacctcttcgcgaagtgggaggaccttgtgctcaccgggtaccaagtggacaagaacaaggacgacgagctgacaggcttcggcggaggaggttccggaggaggcggatccggtggaggcggttcaggcggtggaggaagcggaggcggaggatccggaggcggtggtagcatgattcccggagggttgtccgaagcgaaaccagccacccccgagatccaggaaatcgtggacaaggtcaaaccgcagctggaagagaaaaccggcgaaacctacggaaagctggaagcggtgcagtacaagactcaagtggtgcactactacgtgcactacaacgatcagggcaccaattactacatcaaagtccgggccggcgataacaagtacatgcacctcaaggtctttaagtccctctggggcgaaaacctgttcgccaaatgggaggatctggtgctgactggctaccaagtcgacaagaataaggatgacgagttgaccgggttc

SEQ ID NO: 704 - DNA, 1176 bp, Artificial Sequence
  source 1..1176: mol_type = genomic DNA
attcccggcggactgtcagaagccaaaccggccactccggagatccaggagatcgtggacaaggtcaagccacagctggaggaaaagaccggcgaaacctacgggaagttggaggctgtgcagtacaagacccaggttgtgcactattacgtccactataacgaccaaggcaccaactactatatcaaggtccgagcgggcgataacaaatacatgcacctgaaggtctttaagtccctctggggagaaaacctttttgcgaagtgggaggacctcgtgctcaccggataccaagtggacaagaataaggacgacgaactgactggattcggagggggcggttcaggaggagggggatcagggggaggaggaagcggcggaggaggatccggaggaggcggaagcggtggtggcggatccatgattccgggaggcctttccgaggccaagcctgccacccccgaaatccaagagattgtggataaggtcaaacctcagctggaagaaaagacgggggagacttacggcaaactggaagccgtgcagtataagacccaagtggtgcactactacgtgcactacaacgatcaggggaccaattactacattaaggtccgcgctggagacaacaagtacatgcatctcaaggtattcaagtcgctgtggggcgaaaacctcttcgcgaaatgggaggacttggtgctgaccgggtaccaagtcgataagaacaaggacgatgaacttactgggttcggaggcggaggttcgggtggaggcggttccggtggaggagggtccggtggtggaggatcgggtggcggtggatcgggaggcggtggttccatgatccctggaggcctgtccgaagcaaagccggccaccccagaaatccaggaaatcgtggataaagtcaagccccagttggaggagaaaaccggagagacatacgggaagctggaggcggtgcaatacaagactcaagtggtccattattacgtgcattacaacgaccagggcactaactactacatcaaagtccgggccggggataacaagtatatgcacctcaaggtgttcaagagcctctggggggagaacctgttcgccaaatgggaagatctggtgttgaccggctaccaggtcgacaagaacaaagacgacgagctgacggggttc

SEQ ID NO: 705 - DNA, 753 bp, Artificial Sequence
  source 1..753: mol_type = genomic DNA
atccctggtggcctgtccgaagccaagcctgctacgcccgagatccaggagattgtggacaaagtcaagccgcagctcgaggaaaagaccggcgaaacctacggcaaactcgaagccgtgcagtacaagactcaagtggtgcatcacgcgtacgccgctgtgtacgtgggcacaaactactacatcaaagtccgggccggcgataacaaatacatgcatctgaaagtgttcaagtcgctgccgtactggtacagaaagtacccagacgaggacttggtgctgactgggtaccaggtcgacaagaacaaggatgacgagcttaccggcttcggtggtggaggatccggcggaggaggatcgggaggaggcggttccggaggaggaggcagcggtggaggaggaagcggagggggtggaagcatgattcctggggggctctcagaagcaaagcctgccaccccggaaattcaggagatcgtggataaggtcaagccccagctggaggagaaaactggcgaaacttacgggaagctggaagcggtgcaatacaagacccaggtcgtgcaccatgcctacgccgccgtctacgtggggaccaactattacatcaaggtccgcgcgggagataacaagtacatgcacctgaaggtctttaagtccctcccctactggtaccggaagtatcccgatgaggacctggtgctgaccggctatcaagtggacaagaataaggacgacgagctgaccggtttc

SEQ ID NO: 706 - DNA, 1176 bp, Artificial Sequence
  source 1..1176: mol_type = genomic DNA
attcccggaggactctccgaggccaaaccggccaccccggaaatccaggagatcgtggataaggtcaagccccagctggaggaaaagaccggagagacttacgggaagcttgaggccgtccagtacaagacccaggtggtgcaccatgcgtacgccgcggtctacgtcgggaccaactactacattaaggtccgcgctggcgataacaagtatatgcacttaaaggtgttcaaatccctgccatattggtacaggaagtaccccgacgaagatctggtgctcaccggctaccaggtcgataagaataaggacgacgaactgaccggcttcggaggaggtggaagcggcggtggaggatccggcggaggaggaagcggaggcggtggatccggtggaggagggtctggtggagggggctccatgattcctggaggcctgtccgaagccaagcccgccactcccgaaattcaagaaatcgtggacaaggtcaaaccgcagctggaagaaaagactggagaaacctacggaaagctcgaggcggtgcagtacaaaacccaagtggtgcatcatgcctacgccgccgtctacgtgggcacgaactactatatcaaagtcagagccggcgacaacaagtacatgcacctgaaagtgttcaagtcactgccgtactggtacagaaagtacccggacgaggacctggtgctgaccgggtaccaggtggacaaaaacaaggacgatgaactcaccgggtttggaggaggcggaagcggtggtggtggctccggaggaggaggctcaggaggcggaggatcgggagggggaggttccggagggggtggatcgatgatccctggcggtctgtccgaggctaagccagccacccctgagatccaggaaattgtggacaaagtcaagccgcagctcgaggagaaaaccggcgaaacttacggaaagttggaggccgtgcaatacaagactcaggtcgtgcaccacgcatacgcggctgtgtacgtggggactaactattacatcaaggttcgcgccggagacaacaaatacatgcatctgaaggtctttaagtccctcccctactggtaccggaagtaccctgacgaggacttggtgctgactgggtaccaagtggataagaacaaggatgacgagctgacagggttc

SEQ ID NO: 707 - DNA, 1182 bp, Artificial Sequence
  source 1..1182: mol_type = genomic DNA
atccctggagggctgtccgaggccaagcctgctacgccggaaattcaagaaatcgtcgataaggttaagccacagctcgaagagaaaactggggaaacatacggcaaacttgaggcggttcagtacaaaactcaggtcgtgcactactacgtgcactacaacgatcaagggaccaactactatatcaaggtccgcgcgggagacaacaaatacatgcatctcaaagtgttcaaatcgctgtggggcgagaaccttttcgcgaagtgggaggatttggtgctgactggatatcaggtcgataaaaacaaggatgacgagcttactggctttgccgaggccgctgctaaggaagcagccgcgaaagaagccgccgccaaggaagctgcagccaaggaggcggcagcaaaggaggccgcagccaagatgattcccggaggcctctcagaagccaaaccagccactcctgagattcaggaaattgtcgacaaggtcaagccgcagctggaagagaagactggcgaaacctacgggaagctagaggcggtccagtacaagacccaagtcgtccattactatgtacattacaacgaccagggaaccaattactacattaaagtgcgggccggagataataagtatatgcatcttaaggtgtttaagtcgttgtggggcgaaaacctgtttgccaagtgggaagatcttgtgctcaccggttaccaagtggacaagaacaaggacgacgagctgaccgggttcgctgaagctgccgcgaaggaagccgctgcgaaggaggctgccgcaaaggaagcggccgctaaggaggcagccgccaaagaggccgccgcgaagatgatacctggcggactgtcggaggcgaaaccggccacccctgaaatccaggagattgtggacaaggtgaaaccccaactcgaggaaaaaaccggcgaaacgtacggtaaactcgaagccgtgcagtataagacccaggtcgtacactactatgtgcactataacgatcagggaacgaactactacatcaaggtcagagctggagacaataagtacatgcacctcaaggttttcaagtcgttatggggagaaaacctcttcgcgaaatgggaggatctcgtgctgaccggctaccaggtggacaaaaataaggatgatgaactcaccggtttc

SEQ ID NO: 708 - DNA, 1182 bp, Artificial Sequence
  source 1..1182: mol_type = genomic DNA
atccctggcggactgagcgaggccaagcctgccactccggagatccaggaaatcgtggacaaagtcaagccccagctggaggaaaagactggcgaaacttacggaaagctggaagccgtgcaatacaagacccaagtggtgttcacctatcaaatttcgtacaccgtcgggaccaattactacatcaaagtgcgggccggggataacaaatacatgcacttgaaagtgtttaagtcgctgcggtggaggtaccctgcccgcaagcctgaagatctggtgctcaccggttaccaagtcgacaagaacaaggatgacgagctcaccggcttcgccgaagcagccgctaaagaggccgccgccaaagaagccgccgctaaggaagcagcagcgaaggaggctgccgcgaaagaggcggccgccaagatgattcccggcggattgtccgaagccaagccggctacccccgaaatccaggagatcgtcgacaaggtcaagccacagctcgaagagaaaacgggagagacttacgggaagctggaggcagtccagtataagactcaggtcgtgttcacgtaccaaatctcctacactgtggggactaactactatatcaaagtccgagccggcgacaacaagtacatgcacctcaaggtgttcaagagcttgcgctggcggtaccctgctcggaagccagaagatcttgtgctgactgggtaccaggtcgataagaacaaagacgacgagttgaccggtttcgccgaggcagctgcaaaggaagctgccgccaaggaggcagcggccaaggaagccgctgcgaaggaagcggcggcaaaggaggccgcggcaaagatgatcccgggaggcctgtcagaagccaaacccgcgacccctgagattcaggaaattgtggataaggtcaaaccgcagctggaagaaaagaccggcgaaacctacggaaagttggaggcggtgcagtacaagacacaggttgtgtttacctaccaaatttcctacaccgtgggaaccaactattacatcaaggtccgcgcgggagataacaagtatatgcaccttaaagtgttcaagtccctgagatggagatacccagccagaaagccggaggacctggtgctgaccggctaccaagtggacaaaaacaaggacgacgagctgactggtttc

SEQ ID NO: 709 - DNA, 1182 bp, Artificial Sequence
  source 1..1182: mol_type = genomic DNA
atcccgggaggactgtcggaagcgaagccggccactccagagatccaagaaattgtggacaaggtcaagccccagctcgaggaaaagactggggaaacctacggaaagctcgaggctgtgcagtataagacccaagtggtgcatattccggcgctgaaggtgcacgccggaaccaattactacatcaaagtccgggccggagacaataagtacatgcatctcaaagtgtttaagtccctgccatactggtaccggcacgaccaggaggaggatctcgtgctgaccggctatcaggtcgataagaacaaggacgacgaactgactggtttcgctgaggctgcggcaaaggaggccgccgctaaggaggcggcagcgaaggaagctgcggccaaggaggcagccgcgaaggaggctgccgcgaagatgattcccggtggactgtcagaagccaagccagccactcccgaaatccaggaaatcgtggataaggtcaaaccccagctggaagaaaagaccggagagacttacgggaagttggaggccgtgcagtacaagacccaggtcgtgcacattccggccctgaaagtgcacgcgggtaccaactactacattaaggttcgcgctggagacaacaagtatatgcatctgaaagtgttcaagtccctcccctactggtatcgccacgaccaagaggaagatctggtgctgactggctaccaagtggacaaaaacaaggatgatgaactgaccggcttcgccgaagccgcagcaaaggaagccgccgccaaagaggccgctgctaaggaagcggcggccaaagaagcggccgccaaggaagcagcggccaagatgatccccgggggattgagcgaggccaagcctgccacccctgagatccaggagatcgtggacaaagtcaagccgcagcttgaagagaaaaccggcgaaacatacgggaagctggaggccgtccagtacaaaacccaggtggtgcacatcccggcgctcaaggtccacgccggcactaactactatatcaaggtccgcgccggagataacaaatacatgcacctgaaggtgttcaagagcctcccgtactggtacagacacgatcaggaagaggacctcgtgcttaccgggtaccaggtcgacaagaacaaagacgacgagctgacgggcttc

SEQ ID NO: 710 - DNA, 1182 bp, Artificial Sequence
  source 1..1182: mol_type = genomic DNA
atccctggaggcctgagcgaagccaagcctgccactccggagattcaggagatcgtggacaaagtcaagccccagctggaggaaaagacaggagagacttatggaaagctggaagccgtgcagtataagacccaagtggtgcaccatgcctacgccgccgtctacgtgggaaccaactactacatcaaggttcgcgccggggataacaagtacatgcacctcaaggtgttcaagtccctgccatactggtacagaaagtaccctgatgaggacctggtgctgaccgggtaccaggtcgacaagaataaggacgatgagctgactggctttgccgaagcggcagccaaggaggctgcggcgaaggaagctgccgcgaaagaggcggccgctaaggaagcagctgcaaaggaagcggccgcaaagatgattcccggtggactctccgaagcgaagcctgctaccccggagatccaggagattgtggacaaggtcaaaccgcagctcgaagaaaagaccggggaaacttacgggaagctggaggccgtgcaatacaaaacccaggtggtacaccacgcgtacgccgctgtgtacgtcggcaccaactattacattaaggtccgcgcaggagacaacaagtatatgcacctgaaggtctttaagagcctgccgtactggtaccggaagtacccggacgaggacctcgtgctcaccggctaccaagtggataagaacaaagatgacgagctcacgggtttcgctgaagcagccgccaaggaagccgccgccaaagaggccgccgcaaaggaggcggcggccaaagaagccgcggctaaggaggccgcagccaagatgatccctggtggcctgtcggaggccaaacccgccactcccgaaatccaggaaatcgtggataaggtcaagccgcagctggaagagaaaaccggcgaaacctacggaaagctcgaagcggtgcagtacaagacccaggtcgtgcaccacgcctacgctgcggtgtacgtggggaccaattactatatcaaagtccgggccggcgataacaaatacatgcatctgaaagtgttcaaatcccttccatattggtacaggaagtaccccgacgaggacttggtgcttaccggctatcaagtggacaagaacaaggacgacgaactgactggattc

SEQ ID NO: 711 - DNA, 1173 bp, Artificial Sequence
  source 1..1173: mol_type = genomic DNA
atccccggtggactgtccgaagcaaagccagcgactcccgaaatccaggaaattgtggataaggttaagccccagctggaagaaaagactggagaaacctacggaaagctcgaggccgtgcagtacaaaacccaggtggtgtacgatgaactgtaccacgagaaagccggtactaattactacattaaggtccgcgcaggagacaacaagtatatgcacctcaaagtgtttaagagcctggagtataagttccgcaacctggaagaggacttggtgcttactggataccaagtcgacaaaaacaaggacgacgaactgaccgggttcgccgaagcagcggctaaggaggccgcagctaaggaagccgccgccaaagaagccgcggcgaaagaagcggccgcgaaggaagctgccgcgaagatgattccgggcggtctgtcagaagccaagccggctaccccggaaattcaggaaatcgtggacaaggtcaagccgcagctcgaggaaaagaccggagagacttacgggaagctggaggccgtccagtacaagacccaagtggtgtatgacgaactctaccacgaaaaggccgggacgaactactacatcaaagtcagggccggagataacaagtacatgcacctgaaggtgttcaagtccctggagtacaagttccggaaccttgaggaggacctggtgctgaccggctaccaagtggacaagaacaaggatgatgagctgacagggtttgccgaggctgctgcgaaggaggcggctgccaaggaagcggcggcaaaagaggccgccgcaaaggaggcagcggccaaagaggcagccgccaagatgatccccggcggattgtccgaggccaagccagccacccctgagatccaggagattgtggacaaagtcaagcctcagctcgaagagaaaaccggcgaaacttacggaaagttggaagctgtgcagtataagacccaggtcgtgtacgacgagctgtaccatgagaaggccggcaccaactactatatcaaagtccgggccggcgataacaaatacatgcatctgaaagtgttcaaatcgctcgaatacaagttcagaaaccttgaagaggaccttgtgctcaccgggtaccaggtcgacaagaataaggatgacgaattgactggattc

SEQ ID NO: 712 - DNA, 1182 bp, Artificial Sequence
  source 1..1182: mol_type = genomic DNA
attcctggaggcctgagcgaagccaagcccgccactcctgaaatccaagaaatcgtggacaaggtcaagccacagctggaagagaaaaccggggaaacttacgggaagctggaggccgtccagtacaagacacaagtcgtggtcgaccaagtctggtccgagaatgccggaaccaactactacatcaaggtccgggccggagataacaagtatatgcacctgaaagtgttcaagtcactcccgtacctttggaggaagcacgcggtcgaggacctggtgctgaccgggtaccaggtcgataagaacaaagacgacgaactcaccggattcgcggaagcagccgctaaggaagctgcagcgaaagaagcggccgcgaaggaagcagcggccaaagaggccgccgccaaagaagccgcggcgaagatgatcccgggaggactgtcggaagcgaagccagccacccccgaaatccaggagatcgtggataaggtcaaaccgcagctggaggagaaaactggcgaaacctacggaaagttggaggccgtgcagtataagacccaggtcgtggtggaccaagtgtggtccgaaaacgccggcactaactattacatcaaagtcagagccggcgacaacaagtacatgcatctgaaggtgttcaagagcctcccctacttgtggcgcaagcacgccgtagaggatctcgtgctgacgggctaccaagtggacaagaacaaggacgacgagcttaccggcttcgccgaagccgcagcaaaggaggcggccgcaaaggaagcggcagccaaggaggccgctgctaaggaggctgccgccaaggaagccgctgccaagatgattcccggtggactgtccgaggccaagcctgcgacccctgagattcaggaaatcgtcgacaaagtcaagccccagttggaagaaaagactggagagacttacggaaagctcgaggcggtgcagtacaaaacccaagtggtggtggatcaagtctggagcgagaacgcgggcaccaattactacattaaggtccgcgcaggagacaacaaatacatgcacctcaaggtctttaagtccctgccgtacctgtggcggaagcatgccgtggaggacctcgtgttgaccggttaccaggttgacaaaaacaaggatgatgagctgactggattc

SEQ ID NO: 713 - DNA, 1182 bp, Artificial Sequence
  source 1..1182: mol_type = genomic DNA
attccgggcggactctctgaggccaagcccgccactcctgagattcaggagattgtggataaggtcaaaccgcagctcgaagaaaaaaccggagagacttacggaaaactggaggcggtccagtacaaaacccaagtcgtgggcgactcctattgggaatatgtgtcggggaccaactactacatcaaagtccgcgccggagataacaaatacatgcacctcaaagtgttcaagagcttgccttaccgctggaggcctgaccacgcggaggatctggtgctcaccgggtaccaggtcgacaaaaacaaggacgacgagctgactggctttgccgaagctgccgcaaaagaggctgccgctaaggaggcggccgcgaaagaggcagcagccaaggaggccgctgccaaagaggccgcagccaagatgatcccgggtggactgtccgaggccaaacccgcgacccctgagatccaggaaatcgtggacaaggtcaagcctcagctggaagaaaagactggcgaaacctacggaaagctggaagctgtgcagtacaagacccaggtcgtgggagactcatactgggaatacgtgtccggtaccaactattacattaaggtccgcgcgggagataataagtacatgcatctgaaggtgttcaagtccctgccgtaccggtggaggccggatcatgccgaggacctggtcctcaccggataccaagtggataagaacaaggatgacgaactgaccggcttcgccgaagcagccgcaaaggaagcagcggctaaggaagctgcggccaaagaagccgccgcgaaggaagcggccgccaaggaagccgcggcgaagatgattcctggcggtctgtccgaagctaagcccgctaccccggaaatccaagagatcgtggataaagtcaagccccaactcgaggaaaagaccggagaaacttacgggaagctcgaagccgtgcagtataagactcaagtggtcggggactcgtactgggagtacgtcagcggcactaactactatatcaaagttcgggccggcgacaacaagtatatgcaccttaaagtgtttaagagcctgccctaccgatggcggcccgatcatgcggaggacttggtgctgacgggataccaggtggacaagaataaggacgatgagctgaccggattc

SEQ ID NO: 714 - DNA, 1182 bp, Artificial Sequence
  source 1..1182: mol_type = genomic DNA
atccctggtggcctgtccgaagccaagcctgcgacccctgagatccaagagattgtggacaaagtcaagccgcagctggaagaaaagaccggggaaacctacggcaaactggaggccgtacagtacaagacccaggtcgtgcttgacggcctgtaccatgtcaactccggtacaaactactacatcaaggtccgagccggagacaacaaatacatgcatctcaaagtgttcaagagcctgttctactattaccggtccgaaccgactgaggacctggtgctcacgggttaccaggtcgacaaaaacaaggacgacgaactgaccggttttgccgaagccgcagccaaggaagctgcggccaaagaagccgccgcaaaggaagcagccgccaaggaggctgccgcgaaggaagccgcggcgaagatgatcccgggaggactctcagaggccaaacccgccaccccggaaatccaggagatcgtggacaaggtcaagccacagctggaggaaaagactggagagacttacggaaagctcgaggccgtgcagtacaaaacccaagtggtgctggacggcctttatcacgtgaacagcggcaccaactactatatcaaggttcgcgcgggagacaataagtacatgcacctgaaggtgttcaagtccctgttctattactaccgctcggagccaaccgaggatttggtgctgaccgggtatcaagtggataagaacaaggatgacgagctgaccggcttcgctgaggccgcagcaaaggaggccgccgccaaagaggccgcggctaaggaggcagccgctaaggaagcggccgcgaaagaagcggcggccaagatgattcccggcggactgtcagaagctaagccggccacccctgaaattcaggaaatcgtggataaggtcaaaccccagttggaggagaaaaccggcgaaacttacgggaagctcgaagccgtgcaatacaagactcaggtcgtcctggacgggctgtaccacgtgaactccggcaccaattactacattaaggtccgcgccggagataacaagtatatgcatctgaaagtgtttaagtccctcttctactactaccggtcggagcctactgaggatctggtgctgactgggtaccaagtggacaagaacaaagacgacgagctcaccggattc

SEQ ID NO: 715 - DNA, 1182 bp, Artificial Sequence
  source 1..1182: mol_type = genomic DNA
attcccggaggcctctcagaggccaagcctgccacccccgaaattcaggaaatcgtggataaggtcaagccgcagctggaggagaaaaccggggaaacctacggaaagctggaagcggtgcaatacaaaacccaggtcgtcaagacttgggaggatactgtggtcgccggtaccaattactatatcaaggtccgcgctggcgataacaaatatatgcacctgaaggtgttcaagtccctcgagtacctgtatcggcctctgaaccccgaggacctggtgctgactggataccaggtcgacaagaacaaggacgatgaactgacggggttcgctgaagctgccgccaaggaggctgcggcaaaggaagcagccgcgaaggaggcagcggccaaggaagctgcggccaaagaggccgcggcgaagatgatcccgggtggactctccgaagccaagccagccaccccggaaatccaagagatcgtggacaaggtcaaaccgcagcttgaggaaaagaccggcgaaacttacgggaagttggaagccgtgcagtacaagacccaagtcgtgaaaacctgggaagatacagtggtggcaggcaccaactactacatcaaagtccgcgccggagacaacaaatacatgcatctgaaagtgttcaagagcctggaatacctttaccggccgctgaatcccgaggatttggtgctcactggctaccaagtggacaagaataaggacgacgaactcaccggcttcgccgaagccgctgctaaggaagcggctgcgaaggaagccgccgcaaaggaggcggccgctaaggaggccgccgccaaagaagcggccgccaagatgattcctggtggcctgtcggaggcgaaaccggccacccctgagattcaggagatcgtcgacaaagtgaagccacagctggaagaaaagactggcgaaacctatgggaagcttgaggcagtgcagtataagactcaagtggtcaagacctgggaggacactgtggtggccggaactaattactacattaaggtccgggccggagataacaagtacatgcacctcaaagtgtttaagtccctggaatacttgtacagaccactgaaccctgaggacctcgtgctgaccgggtaccaggttgataagaacaaagacgacgagcttactggattc

SEQ ID NO: 716 - DNA, 1599 bp, Artificial Sequence
  source 1..1599: mol_type = genomic DNA
atccctgggggactcagcgaggctaagcctgcgactcccgaaatccaagagatcgtggacaaagtgaagccgcaactggaagaaaagaccggagaaacttacgggaaactggaggcagtgcaatacaagacacaagtggtccactattacgtccactacaatgatcagggcaccaattattacattaaggtgcgagccggcgataacaaatatatgcacctgaaggtctttaagtccctgtggggagagaatctgttcgcaaagtgggaggacctcgtgcttactggttaccaggtagacaagaataaggacgatgagctgactggtttcggaggcggtggtagcggagggggtggaagcggaggagggggaagtggtggcggtggatcaggcggagggggatcagggggaggagggtccatgatccctggagggctgtccgaggccaagcctgctacgccggaaattcaagaaatcgtcgataaggttaagccacagctcgaagagaaaactggggaaacatacggcaaacttgaggcggttcagtacaaaactcaggtcgtgcactactacgtgcactacaacgatcaagggaccaactactatatcaaggtccgcgcgggagacaacaaatacatgcatctcaaagtgttcaaatcgctgtggggcgagaaccttttcgcgaagtgggaggatttggtgctgactggatatcaggtcgataaaaacaaggatgacgagcttactggctttggcggaggcggatcaggaggaggtggcagcggtggaggaggttccggtggaggcggttccggaggaggaggctcaggagggggaggctccatgattcccggaggcctctcagaagccaaaccagccactcctgagattcaggaaattgtcgacaaggtcaagccgcagctggaagagaagactggcgaaacctacgggaagctagaggcggtccagtacaagacccaagtcgtccattactatgtacattacaacgaccagggaaccaattactacattaaagtgcgggccggagataataagtatatgcatcttaaggtgtttaagtcgttgtggggcgaaaacctgtttgccaagtgggaagatcttgtgctcaccggttaccaagtggacaagaacaaggacgacgagctgaccgggttcggaggaggcggaagcggtggtggaggatcgggaggcggaggatccggtggtggcggatctggcggtggaggttctggggggggaggatccatgatacctggcggactgtcggaggcgaaaccggccacccctgaaatccaggagattgtggacaaggtgaaaccccaactcgaggaaaaaaccggcgaaacgtacggtaaactcgaagccgtgcagtataagacccaggtcgtacactactatgtgcactataacgatcagggaacgaactactacatcaaggtcagagctggagacaataagtacatgcacctcaaggttttcaagtcgttatggggagaaaacctcttcgcgaaatgggaggatctcgtgctgaccggctaccaggtggacaaaaataaggatgatgaactcaccggtttc

SEQ ID NO: 717 - DNA, 1608 bp, Artificial Sequence
  source 1..1608: mol_type = genomic DNA
atccctgggggactcagcgaggctaagcctgcgactcccgaaatccaagagatcgtggacaaagtgaagccgcaactggaagaaaagaccggagaaacttacgggaaactggaggcagtgcaatacaagacacaagtggtccactattacgtccactacaatgatcagggcaccaattattacattaaggtgcgagccggcgataacaaatatatgcacctgaaggtctttaagtccctgtggggagagaatctgttcgcaaagtgggaggacctcgtgcttactggttaccaggtagacaagaataaggacgatgagctgactggtttcgccgaagccgcagcaaaagaggccgccgcgaaagaagccgctgctaaggaggcggccgcaaaggaggccgcggcaaaagaagcggcggccaaaatgatccctggagggctgtccgaggccaagcctgctacgccggaaattcaagaaatcgtcgataaggttaagccacagctcgaagagaaaactggggaaacatacggcaaacttgaggcggttcagtacaaaactcaggtcgtgcactactacgtgcactacaacgatcaagggaccaactactatatcaaggtccgcgcgggagacaacaaatacatgcatctcaaagtgttcaaatcgctgtggggcgagaaccttttcgcgaagtgggaggatttggtgctgactggatatcaggtcgataaaaacaaggatgacgagcttactggctttgctgaggctgccgccaaggaggctgcggcgaaggaagcagcagcgaaagaggcagccgccaaagaagctgcagcgaaggaggcagcagccaagatgattcccggaggcctctcagaagccaaaccagccactcctgagattcaggaaattgtcgacaaggtcaagccgcagctggaagagaagactggcgaaacctacgggaagctagaggcggtccagtacaagacccaagtcgtccattactatgtacattacaacgaccagggaaccaattactacattaaagtgcgggccggagataataagtatatgcatcttaaggtgtttaagtcgttgtggggcgaaaacctgtttgccaagtgggaagatcttgtgctcaccggttaccaagtggacaagaacaaggacgacgagctgaccgggttcgctgaagctgcggccaaagaggcggcggcaaaggaagcggccgctaaagaagcagcggccaaggaagctgccgctaaggaagccgcggcgaagatgatacctggcggactgtcggaggcgaaaccggccacccctgaaatccaggagattgtggacaaggtgaaaccccaactcgaggaaaaaaccggcgaaacgtacggtaaactcgaagccgtgcagtataagacccaggtcgtacactactatgtgcactataacgatcagggaacgaactactacatcaaggtcagagctggagacaataagtacatgcacctcaaggttttcaagtcgttatggggagaaaacctcttcgcgaaatgggaggatctcgtgctgaccggctaccaggtggacaaaaataaggatgatgaactcaccggtttc

SEQ ID NO: 718 - DNA, 1602 bp, Artificial Sequence
  source 1..1602: mol_type = genomic DNA
atccctggagggctgtccgaggccaagcctgctacgccggaaattcaagaaatcgtcgataaggttaagccacagctcgaagagaaaactggggaaacatacggcaaacttgaggcggttcagtacaaaactcaggtcgtgcactactacgtgcactacaacgatcaagggaccaactactatatcaaggtccgcgcgggagacaacaaatacatgcatctcaaagtgttcaaatcgctgtggggcgagaaccttttcgcgaagtgggaggatttggtgctgactggatatcaggtcgataaaaacaaggatgacgagcttactggctttggaggaggagggtccggtggaggaggctctggtggaggcggaagcggcggaggaggatcgggtggcggaggaagcggtggtggaggctccatgattcccggaggcctctcagaagccaaaccagccactcctgagattcaggaaattgtcgacaaggtcaagccgcagctggaagagaagactggcgaaacctacgggaagctagaggcggtccagtacaagacccaagtcgtccattactatgtacattacaacgaccagggaaccaattactacattaaagtgcgggccggagataataagtatatgcatcttaaggtgtttaagtcgttgtggggcgaaaacctgtttgccaagtgggaagatcttgtgctcaccggttaccaagtggacaagaacaaggacgacgagctgaccgggttcggaggaggcggatcgggaggtggaggatccggtggcggtggaagcggaggtggcggatctgggggagggggatcaggaggcggcggatccatgatacctggcggactgtcggaggcgaaaccggccacccctgaaatccaggagattgtggacaaggtgaaaccccaactcgaggaaaaaaccggcgaaacgtacggtaaactcgaagccgtgcagtataagacccaggtcgtacactactatgtgcactataacgatcagggaacgaactactacatcaaggtcagagctggagacaataagtacatgcacctcaaggttttcaagtcgttatggggagaaaacctcttcgcgaaatgggaggatctcgtgctgaccggctaccaggtggacaaaaataaggatgatgaactcaccggtttcggaggcggaggatcaggcggagggggttcaggagggggtggctcaggaggagggggtagtggaggcggtggatccggaggaggtggcagcatgatcccacggggtctgtccgaagccaagccagccaccccagagatccaagaaatagtggataaggtgaagccccagcttgaggaaaagactggagagacttacggaaagctcgaggctgtccaatacaaaacacaggtgctggcgaacttcttccaaaggagatggccaggcagtactaactattacatcaaagtgcgcgcaggagataacaaatatatgcacttgaaggtgttcaatggaccgtggaagttccggaacaccgacagaggcgccgacagggtcttgaccgggtaccaagtcgataagaacaaagacgacgaactgaccggtttc

SEQ ID NO: 719 - DNA, 2025 bp, Artificial Sequence
  source 1..2025: mol_type = genomic DNA
atccctgggggactcagcgaggctaagcctgcgactcccgaaatccaagagatcgtggacaaagtgaagccgcaactggaagaaaagaccggagaaacttacgggaaactggaggcagtgcaatacaagacacaagtggtccactattacgtccactacaatgatcagggcaccaattattacattaaggtgcgagccggcgataacaagtatatgcacctgaaggtctttaagtccctgtggggagagaatctgttcgcaaagtgggaggacctcgtgcttactggttaccaggtagacaagaataaggacgatgagctgactggtttcgggggcggaggatctgggggtggaggaagcggtggtggaggctcgggtggaggagggtctgggggaggaggttcaggcggcggaggttccatgatccctggagggctgtccgaggccaagcctgctacgccggaaattcaagaaatcgtcgataaggttaagccacagctcgaagagaaaactggggaaacatacggcaaacttgaggcggttcagtacaaaactcaggtcgtgcactactacgtgcactacaacgatcaagggaccaactactatatcaaggtccgcgcgggagacaacaaatacatgcatctcaaagtgttcaaatcgctgtggggcgagaaccttttcgcgaagtgggaggatttggtgctgactggatatcaggtcgataaaaacaaggatgacgagcttactggctttggaggcggtggatcgggagggggtggttcgggaggaggaggctcaggcggaggaggatcaggaggcggcggaagtggaggcggaggctccatgattcccggaggcctctcagaagccaaaccagccactcctgagattcaggaaattgtcgacaaggtcaagccgcagctggaagagaagactggcgaaacctacgggaagctagaggcggtccagtacaagacccaagtcgtccattactatgtacattacaacgaccagggaaccaattactacattaaagtgcgggccggagataataagtatatgcatcttaaggtgtttaagtcgttgtggggcgaaaacctgtttgccaagtgggaagatcttgtgctcaccggttaccaagtggacaagaacaaggacgacgagctgaccgggttcggaggaggcggatcagggggtggtggttccggcggaggtggatccggaggaggtggaagcgggggaggtggttcaggagggggcggatccatgatacctggcggactgtcggaggcgaaaccggccacccctgaaatccaggagattgtggacaaggtgaaaccccaactcgaggaaaaaaccggcgaaacgtacggtaaactcgaagccgtgcagtataagacccaggtcgtacactactatgtgcactataacgatcagggaacgaactactacatcaaggtcagagctggagacaataagtacatgcacctcaaggttttcaagtcgttatggggagaaaacctcttcgcgaaatgggaggatctcgtgctgaccggctaccaggtggacaaaaataaggatgatgaactcaccggtttcggcggtggaggatcgggcggtggtggtagcggagggggaggatccggtggagggggtagcggtggaggcggttccggtggtggcggaagcatgatcccacggggtctgtccgaagccaagccagccaccccagagatccaagaaatagtggataaggtgaagccccagcttgaggaaaagactggagagacttacggaaagctcgaggctgtccaatacaaaacacaggtgctggcgaacttcttccaaaggagatggccaggcagtactaactattacatcaaagtgcgcgcaggagataacaaatatatgcacttgaaggtgttcaatggaccgtggaagttccggaacaccgacagaggcgccgacagggtcttgaccgggtaccaagtcgataagaacaaagacgacgaactgaccggtttc

SEQ ID NO: 720 - DNA, 1611 bp, Artificial Sequence
  source 1..1611: mol_type = genomic DNA
atccctggagggctgtccgaggccaagcctgctacgccggaaattcaagaaatcgtcgataaggttaagccacagctcgaagagaaaactggggaaacatacggcaaacttgaggcggttcagtacaaaactcaggtcgtgcactactacgtgcactacaacgatcaagggaccaactactatatcaaggtccgcgcgggagacaacaaatacatgcatctcaaagtgttcaaatcgctgtggggcgagaaccttttcgcgaagtgggaggatttggtgctgactggatatcaggtcgataaaaacaaggatgacgagcttactggctttgccgaggctgcagccaaagaagccgcggcgaaggaagcggcggcaaaggaggcagccgcaaaggaagctgccgctaaagaggccgccgcaaagatgattcccggaggcctctcagaagccaaaccagccactcctgagattcaggaaattgtcgacaaggtcaagccgcagctggaagagaagactggcgaaacctacgggaagctagaggcggtccagtacaagacccaagtcgtccattactatgtacattacaacgaccagggaaccaattactacattaaagtgcgggccggagataataagtatatgcatcttaaggtgtttaagtcgttgtggggcgaaaacctgtttgccaagtgggaagatcttgtgctcaccggttaccaagtggacaagaacaaggacgacgagctgaccgggttcgctgaggctgccgccaaggaagccgcagcgaaggaggccgctgcgaaagaagcggcagccaaggaggcggctgccaaagaggcggccgcgaagatgatacctggcggactgtcggaggcgaaaccggccacccctgaaatccaggagattgtggacaaggtgaaaccccaactcgaggaaaaaaccggcgaaacgtacggtaaactcgaagccgtgcagtataagacccaggtcgtacactactatgtgcactataacgatcagggaacgaactactacatcaaggtcagagctggagacaataagtacatgcacctcaaggttttcaagtcgttatggggagaaaacctcttcgcgaaatgggaggatctcgtgctgaccggctaccaggtggacaaaaataaggatgatgaactcaccggtttcgctgaagcagcggcgaaagaggcagcggccaaggaagccgctgccaaggaagccgccgctaaggaggctgcggctaaggaagcagccgccaagatgatcccacggggtctgtccgaagccaagccagccaccccagagatccaagaaatagtggataaggtgaagccccagcttgaggaaaagactggagagacttacggaaagctcgaggctgtccaatacaaaacacaggtgctggcgaacttcttccaaaggagatggccaggcagtactaactattacatcaaagtgcgcgcaggagataacaaatatatgcacttgaaggtgttcaatggaccgtggaagttccggaacaccgacagaggcgccgacagggtcttgaccgggtaccaagtcgataagaacaaagacgacgaactgaccggattc

SEQ ID NO: 721 - DNA, 2037 bp, Artificial Sequence
  source 1..2037: mol_type = genomic DNA
atccctgggggactcagcgaggctaagcctgcgactcccgaaatccaagagatcgtggacaaagtgaagccgcaactggaagaaaagaccggagaaacttacgggaaactggaggcagtgcaatacaagacacaagtggtccactattacgtccactacaatgatcagggcaccaattattacattaaggtgcgagccggcgataacaagtatatgcacctgaaggtctttaagtccctgtggggagagaatctgttcgcaaagtgggaggacctcgtgcttactggttaccaggtagacaagaataaggacgatgagctgactggtttcgccgaagctgcagcgaaagaggcagctgcgaaagaagcggcagccaaagaagccgctgccaaggaggctgccgccaaagaggcggccgccaaaatgatccctggagggctgtccgaggccaagcctgctacgccggaaattcaagaaatcgtcgataaggttaagccacagctcgaagagaaaactggggaaacatacggcaaacttgaggcggttcagtacaaaactcaggtcgtgcactactacgtgcactacaacgatcaagggaccaactactatatcaaggtccgcgcgggagacaacaaatacatgcatctcaaagtgttcaaatcgctgtggggcgagaaccttttcgcgaagtgggaggatttggtgctgactggatatcaggtcgataaaaacaaggatgacgagcttactggctttgccgaagccgcagcgaaggaagcagccgcgaaggaggcagcggcaaaagaggccgcggctaaagaagctgccgcaaaggaggccgccgcaaagatgattcccggaggcctctcagaagccaaaccagccactcctgagattcaggaaattgtcgacaaggtcaagccgcagctggaagagaagactggcgaaacctacgggaagctagaggcggtccagtacaagacccaagtcgtccattactatgtacattacaacgaccagggaaccaattactacattaaagtgcgggccggagataataagtatatgcatcttaaggtgtttaagtcgttgtggggcgaaaacctgtttgccaagtgggaagatcttgtgctcaccggttaccaagtggacaagaacaaggacgacgagctgaccgggttcgctgaggcagccgcaaaagaagcagcagcaaaggaggccgccgccaaggaagcggcggcaaaggaagctgctgctaaggaggcggctgccaagatgatacctggcggactgtcggaggcgaaaccggccacccctgaaatccaggagattgtggacaaggtgaaaccccaactcgaggaaaaaaccggcgaaacgtacggtaaactcgaagccgtgcagtataagacccaggtcgtacactactatgtgcactataacgatcagggaacgaactactacatcaaggtcagagctggagacaataagtacatgcacctcaaggttttcaagtcgttatggggagaaaacctcttcgcgaaatgggaggatctcgtgctgaccggctaccaggtggacaaaaataaggatgatgaactcaccggtttcgctgaagcggccgctaaagaggctgcggctaaggaagccgcggcgaaggaagcagcggccaaggaggctgctgcaaaggaggccgccgctaagatgatcccacggggtctgtccgaagccaagccagccaccccagagatccaagaaatagtggataaggtgaagccccagcttgaggaaaagactggagagacttacggaaagctcgaggctgtccaatacaaaacacaggtgctggcgaacttcttccaaaggagatggccaggcagtactaactattacatcaaagtgcgcgcaggagataacaaatatatgcacttgaaggtgttcaatggaccgtggaagttccggaacaccgacagaggcgccgacagggtcttgaccgggtaccaagtcgataagaacaaagacgacgaactgaccggattc

SEQ ID NO: 722 - DNA, 1698 bp, Artificial Sequence
  source 1..1698: mol_type = genomic DNA
atacctggcggtctgagcgaagcaaagccggccactcctgaaattcaggaaatcgtggacaaggttaagccccagctcgaggaaaagaccggcgaaacctatggcaaactggaagcggtgcagtacaagactcaggtcgtgcactattacgtgcactataacgaccaaggcactaactattacatcaaggtccgagcgggagacaacaagtacatgcacctgaaagtgtttaagagcctgtggggggaaaacctcttcgccaaatgggaagatctggtgctcaccgggtaccaggtcgacaagaacaaagacgacgagctgaccgggttcgctgaggcagcggcaaaagaagccgcggctaaagaggctgccgccaaggaagccgccgcaaaggaggccgctgccaaagaggccgccgccaagatgattcccgggggactttcggaagccaagcctgccacaccggagatccaagagattgtggacaaagtgaagcctcagctcgaagaaaagactggagagacttatggaaagctggaggccgtccagtacaaaacccaagtcgtgcattactacgtgcattacaacgatcaggggactaactactatatcaaagtgcgcgccggggataacaaatatatgcatcttaaggtgtttaagtccctctggggcgaaaacttgttcgcgaaatgggaggacttggtgcttactggataccaagtcgacaaaaacaaggatgatgaactgacgggattcgccgaagccgctgctaaggaggcagccgcgaaagaagcggccgctaaggaagcggcggccaaagaagctgcggcgaaggaagctgccgcgaagatgatcccgggaggactgagcgaggccaagccagcaaccccggagattcaagaaatcgtcgacaaggtcaagccccagttggaagagaaaaccggggaaacctacggcaaactcgaagccgtgcagtataagactcaagtggtgcactactacgtccactacaacgaccagggcaccaactactacattaaggtccgcgctggtgacaacaaatacatgcatctgaaggtctttaagtcgctgtggggagagaacctgttcgcgaagtgggaggacctggtgctgaccggctaccaagtggacaagaataaggatgacgagctcaccggcttcggaggaggagggtccggtggtggaggttcgggagggggtggttccggagggggaggttccggtggaggcggaagtggcggaggaggatccggcggtggtggatccggtggcggtggatcaggaggcggaggctcaggaggtggcggaagcggaggagggggttcaggaggaggcggctccatgattccgaggggtctgtcagaggctaagcccgcgacccctgaaatccaggagatcgtggataaggtcaaaccgcagctggaggagaaaactggggagacttacgggaagctcgaggccgtgcaatacaagacccaagtgctcgccaacttcttccagcggagatggcccggaagcacgaattactacatcaaagtccgggccggagataataagtatatgcacttgaaggtgttcaacgggccctggaagttccggaacaccgatagaggcgcagatcgcgtgctgactggctaccaggtggacaaaaataaggacgacgaactgaccggtttc

SEQ ID NO: 723 - DNA, 1602 bp, Artificial Sequence
  source 1..1602: mol_type = genomic DNA
atccctggaggcctgagcgaggccaagccagctaccccggagattcaggaaatcgtggacaaggtcaaaccgcagctcgaggaaaagactggagaaacctatggcaaactcgaagcggtccagtacaagactcaagtggtgcactactacgtgcattacaatgaccagggcacgaactactacatcaaagtccgggctggcgacaacaagtatatgcatctaaaggtctttaagtccctctggggcgaaaacctgttcgccaaatgggaagatctggtgctcactgggtaccaagtcgataagaacaaagacgacgaactcaccgggttcggaggagggggttccggtggaggtggcagcggaggtggtggctcaatgattccgggaggactgtcggaagctaagccggccactcccgaaattcaagagatcgtggataaggttaaaccccagctcgaagaaaagaccggggaaacttatggaaagctcgaagccgtgcagtacaaaacccaagtcgtgcattactacgtccactataacgatcaggggaccaactactatatcaaggtccgcgccggagataataagtacatgcatctgaaggtgttcaagtcgctctggggggaaaaccttttcgcgaaatgggaggatctcgtgctgaccgggtaccaggtcgacaagaacaaggatgacgagctgaccggcttcggtggaggaggaagcggcggaggtggaagcggtggtggcggatccatgatccccggaggcctttccgaagcgaagcctgccacccctgagatccaagagattgtggacaaagtcaagccacagctggaggagaaaaccggagaaacttacggaaagctggaggccgtgcaatataagacccaggtcgtgcactattacgtgcactacaacgaccagggaactaactattacatcaaggtcagagcgggagataacaagtacatgcacctgaaagtgtttaagtcgctgtggggagagaatctgttcgctaagtgggaggacctggtgctgactggctaccaggtggacaagaataaggacgatgagcttaccggattcggagggggaggctctggaggaggcggctcaggaggtggaggatcggggggtggaggttccggcggaggaggatcagggggcggaggaagtggtggaggcggttcgggaggaggtggatctggcggaggcggatcaggaggaggagggagtggcggtggtggatcaggcggtggagggtccatgattcctcggggactgagcgaagccaagcccgcgactccggaaatccaggagatcgtcgataaggtcaagccccagcttgaagaaaaaaccggcgaaacctacgggaagctcgaggccgtccaatacaagacacaagtgctggccaacttcttccaacggcgctggccaggatccacgaattactacattaaggtccgagccggcgataacaaatacatgcacttgaaagtgttcaacggaccttggaagttcaggaacactgaccggggcgcagacagagtgcttaccggctaccaagtggacaaaaacaaggacgacgagttgactggattc

SEQ ID NO: 724 - DNA, 1605 bp, Artificial Sequence
  source 1..1605: mol_type = genomic DNA
attccgggaggccttagcgaagcgaagcctgcgacgccagagatccaggaaattgtggacaaagtgaagccccaactggaggagaaaaccggagaaacctatggaaagctggaagcggtgcagtacaagacccaagtggtgcattactacgtgcactataacgatcaggggactaattactacattaaggtccgggctggggataacaagtatatgcaccttaaggtattcaagtcactgtggggggagaacctgtttgctaagtgggaggacctggtgctgaccggttaccaggtggacaaaaataaggacgacgaactgactgggttcggtggcggaggttcgggagggggaggaagcggaggcggaggatccatgattccgggtggactctccgaggccaagcctgccactcccgaaatccaggagatcgtggacaaggtcaagcctcagctggaggaaaagactggagaaacatacgggaaactggaagccgtgcagtataagacccaggtggtgcactattacgtacactacaacgaccagggcaccaactactacatcaaagtccgggccggcgataataagtacatgcacctgaaggtgttcaagtccctctggggcgaaaacctgttcgcgaagtgggaagatctcgtgctcaccgggtaccaagtggacaagaacaaggatgacgagctgaccggctttggcggaggaggctcaggagggggtggtagcggaggagggggttccatgatccccggaggtctgagcgaagccaagcccgcaacaccggagatccaagagatcgtcgacaaggttaagccgcagctggaagaaaagaccggcgaaacctacggcaaactggaggccgtgcaatacaaaacccaggtcgtgcactactacgtccactacaatgaccaaggcactaattattacatcaaggtccgcgctggcgataacaaatatatgcatctgaaagtgtttaagtcgctgtggggagagaacctcttcgccaaatgggaggacttggtgttgaccggctaccaggtcgacaaaaacaaggacgatgagcttaccggctttgccgaagccgcggcaaaggaggccgccgcgaaagaagcggcggccaaagaagccgccgctaaggaggcggccgctaaagaggcggcagccaaagaggctgccgccaaggaagctgcggctaaggaagcagcggcgaaggaggctgctgccaaggaggcagccgcgaaggaagcggccgccaagatgatccctaggggcctgtccgaagctaagccagccacccctgagattcaggaaatcgtggataaagtcaagccacaactggaagagaaaactggggaaacttacgggaagctcgaagccgtccagtacaaaactcaagtgctggccaacttcttccaacggagatggccgggatccaccaactattacataaaagtccgcgccggagacaacaaatacatgcatctcaaggtctttaacgggccgtggaagttccgcaacactgaccggggagcagacagagtgctgactggttaccaagtcgacaagaataaggatgatgagctgacgggattc

SEQ ID NO: 725 - DNA, 1608 bp, Artificial Sequence
  source 1..1608: mol_type = genomic DNA
atccctggagggctcagcgaggccaaacccgccactcctgagattcaggagatcgtggataaggtcaaaccgcagctcgaggagaaaacgggcgaaacttacgggaagctggaagccgtgcagtataagacccaagtggtgcattactacgtccattacaacgatcagggcaccaattactacattaaggtccgggctggtgacaacaaatacatgcatctgaaggtctttaagtcgctctggggggaaaacctcttcgcgaagtgggaagatctggtccttaccggataccaagtggacaagaacaaagatgacgagttgaccgggtttgccgaggcggcagctaaggaggcagccgcgaaggaagcggccgcgaagatgatccctggcggactgtccgaagccaagcctgcgacccctgaaattcaggaaatcgtggacaaagtcaagccccagttggaagaaaagaccggcgaaacatacggaaagctagaggcagtgcagtacaagacccaggtcgtgcactactatgtgcactacaacgaccagggtactaactactatatcaaggttcgcgcgggagacaacaagtatatgcatctcaaagtgttcaagagcctgtggggcgaaaacctgttcgccaaatgggaggacctggtgctgaccggctaccaggtggataagaacaaggacgacgagctgaccgggttcgctgaagccgcagccaaggaggctgccgccaaggaagccgccgcaaagatgattccgggaggattgtccgaagcgaagccggccactccagagatccaagaaattgtggacaaggttaaaccgcaactggaggaaaagactggcgaaacctatggaaagctcgaggccgtccagtacaaaactcaggtcgtacactactacgtgcactataacgaccaagggaccaattattacatcaaggtccgcgccggagataacaaatatatgcacctcaaggtgttcaagtcgctgtggggggagaacctgtttgccaagtgggaggatcttgtgctgacggggtaccaggttgacaagaataaggacgatgaacttaccggctttggagggggtggtagcggaggcggtggttccggtggtggcggaagcggaggaggaggctccggtggaggaggatcaggaggcggaggatcgggtggcggaggttctggcggaggaggttccggagggggaggaagtggcggtggaggttcgggcggtggtggatcagggggaggcggatccatgatcccccgaggactgagcgaggctaagccagcgaccccggaaatccaagagattgtcgacaaggtcaagccgcagctggaagagaaaaccggggaaacctacggcaaactggaagcggtgcaatacaagactcaggtgctcgcaaacttcttccaacggcgctggcctggatccaccaactactacatcaaagtccgggccggggataacaagtacatgcacctgaaagtgtttaacggcccgtggaagttccggaacaccgacagaggagccgacagagtgctgactggataccaggtcgacaaaaacaaagacgacgaactgactggcttc

SEQ ID NO: 726 - DNA, 1611 bp, Artificial Sequence
  source 1..1611: mol_type = genomic DNA
attccgggtggactgtccgaggccaagccagccacccccgaaatccaggaaattgtggacaaggtcaagccacagctggaggaaaagaccggcgaaacctatggaaagctcgaggcagtgcagtataagacccaggtggtccactactatgtgcactacaatgaccaagggaccaactattacatcaaagtccgcgccggagacaacaagtacatgcatctgaaggttttcaagtccctttggggcgaaaacctgtttgccaaatgggaggacttggtgctgacggggtaccaagtggataagaacaaagatgacgaactcactgggttcgccgaagcagccgctaaggaggcggccgccaaagaggcggctgccaagatgatcccggggggtctttcggaagcgaagcctgcaacccccgagatccaagagatcgtggacaaagtcaagccccaactggaagagaaaactggagagacttacgggaagctcgaagccgtgcagtacaagactcaggtcgtgcactactacgtccactacaacgatcagggcaccaattactacatcaaggtccgggccggagataataagtatatgcatctcaaggtgttcaagtcgttgtggggagagaacctcttcgcgaagtgggaggatctcgtgctgactggttatcaagtggacaagaacaaggatgacgagctgaccggattcgctgaagcggcagccaaagaagccgcggcgaaggaagccgccgcgaagatgattcccggaggcctgtcagaggctaagcctgccactccggaaattcaggagatcgtcgacaaggttaagccgcagctggaagaaaaaaccggggaaacctacggaaagctggaagcggtgcaatacaagacccaagtggtgcattactacgtgcactataacgaccagggtacaaactactatatcaaagtcagagcgggagataacaaatacatgcaccttaaggtctttaagtcactgtggggggagaacctgttcgctaagtgggaagatctggtgctcaccgggtaccaggtcgacaaaaacaaggacgacgagctcaccggctttgccgaagccgctgcaaaggaagccgcagccaaggaggctgcggcaaaagaagcagcggcgaaagaggctgccgcaaaagaggccgcggcaaaggaggcagcggctaaagaagctgccgccaaggaagcagcagctaaggaagctgcagcgaaggaggccgctgcgaaagaagcggccgcgaaaatgattccgagaggcctgagcgaagccaagccggccactcctgagattcaggaaatcgtggataaagtgaagcctcagttggaagaaaagactggcgaaacttacggaaagttggaagccgtacagtacaaaacccaggtcctggccaacttctttcaacgccgctggcctggatccaccaactactacataaaagtgcgggccggcgataacaagtatatgcacctgaaagtgttcaacggaccgtggaagttccggaacactgacaggggtgccgacagagtcctgaccggataccaggtggataaaaacaaagacgacgaactgactggattc

SEQ ID NO: 727 - DNA, 1611 bp, Artificial Sequence
  source 1..1611: mol_type = genomic DNA
atccctgggggactctccgaagcgaagcctgccacccccgaaatccaggaaatcgtggacaaagtcaagccacagttggaggagaaaactggagagacttacggcaaactggaagccgtgcagtataagacccaggtcgtgggtggagggggaggtggaggagggggtggaaccaattactacatcaaagtgcgggccggcgataacaagtacatgcatttgaaggtgttcaagtcactaggcggaggcggaggaggaggtggtggagaagatctggtgctcacgggataccaggtggacaagaataaggacgacgagcttactggattcgcggaagctgctgcaaaggaagctgcagcgaaggaagccgccgcgaaggaggctgctgccaaagaggctgccgctaaggaggcagcggccaagatgatccctggaggcctctccgaggctaagccggctactccagagattcaagagatcgtcgacaaagtgaagccccagctggaagaaaagactggggaaacttacgggaagctggaggccgtgcaatacaaaactcaagtcgttggggggggaggaggtggtggtgggggagggaccaactactacataaaggtccgcgcaggagataataagtacatgcacctcaaagtgtttaagtcactgggtggcggtggtggaggaggcggtggagaggacctcgtgctgacgggctaccaggtcgataagaacaaagacgacgaactgactggcttcgccgaagctgcggcaaaggaggccgcagccaaggaggcggcagctaaagaggccgctgcaaaagaagccgcggccaaagaagcggcggcgaagatgattcctggggggctctcagaggccaagccggcaacccctgagattcaggaaattgtggataaggtcaaaccgcagctggaggaaaagaccggggaaacctacgggaagttggaggcagtgcagtacaaaacacaagtggtcggtggaggtgggggtggaggcgggggaggtactaattactatatcaaggtccgagctggcgacaacaagtatatgcacctgaaggtctttaagtccttgggcggtggaggaggtggtggcggaggagaggacttggtgttgactgggtaccaagtggataaaaacaaggatgacgagctgactggtttcgctgaggcagccgcaaaggaagctgccgcaaaagaggcggctgccaaggaagcggccgcgaaagaagcagcggctaaggaagcagccgccaaaatgatcccgagagggctgtccgaagccaagcccgcgactcctgagatccaggagattgtggacaaggtcaagcctcagcttgaagagaaaaccggggagacttatgggaagctcgaggccgtccagtacaagacccaagtgctcgccaacttcttccaacggagatggcccggctcgaccaactattacattaaggtcagagccggagacaacaaatacatgcatctgaaagtgttcaacggcccgtggaagttccggaacaccgaccgcggagcagacagggtcctgaccggatatcaggtcgacaagaacaaggacgatgagctcaccggattc

SEQ ID NO: 728 - DNA, 2037 bp, Artificial Sequence
  source 1..2037: mol_type = genomic DNA
atccctggaggcctctccgaggctaagccggccactccagagattcaagagatcgtcgacaaagtcaagccccagctggaagaaaagactggggaaacttacgggaagctggaggcggtgcaatacaaaactcaggtcgtcggaggcggaggaggaggtggtggcggagggaccaactactatataaaggtccgcgcgggagataataagtacatgcacctcaaagtgtttaagtcactgggtggcggtggtggaggaggcggtggagaggacctcgtgctgacgggataccaggtcgataagaacaaagatgacgaactgactggattcgccgaagctgcggcaaaggaggccgcagccaaggaggcagcggctaaggaagcagctgcaaaggaggccgcagccaaggaagcggccgcgaagatgattcctggggggctctcagaggcaaagccggcgacccctgaaattcaggaaattgtggataaggtcaaacctcagctggaggaaaaaaccggggaaacctatgggaagttggaagccgtgcagtacaaaacacaggtggtcgggggaggtggaggtggaggcggcggtggaactaattactatatcaaggtccgagctggcgacaacaagtatatgcacctgaaggttttcaagagcttgggcggtggaggaggtggtggcggaggagaggacttagtgctgactgggtaccaagtcgataaaaacaaggatgacgagctgactggtttcgctgaggcagccgcaaaggaagctgccgcgaaagaggcggctgccaaggaagctgccgcaaaagaagcagcggccaaggaagcagccgctaagatgatacccagaggcctgtccgaagccaagcccgccactcctgagatccaggagattgtggacaaggtcaagcctcaacttgaagagaaaaccggagagacttatgggaagctcgaggccgtccagtacaagacacaagtcctggccaacttcttccaacggagatggcccggatcgaccaattactacatcaaagtccgcgccggagacaacaaatacatgcatctgaaagtgttcaacggcccgtggaagttccgcaacaccgaccggggagcagacagggtgctcactggctaccaagtggacaagaataaggatgatgaactgaccggctttgctgaggctgcggcgaaggaagctgccgctaaagaagccgccgccaaggaagccgctgcgaaggaggctgccgccaaagaagcggcggccaagatgatccctggcggactgtccgaggccaagcctgcaacccccgagattcaggagatcgtggacaaagtgaagccgcagctcgaggaaaagaccggagaaacttatggaaagctggaagccgtacagtataagacccaggtcgtgggtggcggcggaggtggaggagggggtggcaccaactattacatcaaggttcgcgccggcgataacaaatatatgcatttgaaggtctttaagtcgttgggaggtggcgggggtggaggaggaggggaggacctggtgctgaccggctaccaggtggacaaaaacaaagacgacgaactcaccgggttcgctgaagcggctgcaaaagaggccgcggctaaagaggcagctgccaaagaggctgcagcgaaggaggctgctgctaaggaggcggccgccaaaatgatcccgggaggcctgtcagaagcgaagccagccaccccggaaattcaagaaatcgtggataaagttaagcctcagctcgaagaaaaaacgggcgaaacctacggcaaacttgaagccgtccaatacaagacccaagtggtcggaggtgggggtggtggtggtgggggaggaacgaactactacattaaggtccgggccggagataacaagtacatgcacttgaaggtgttcaagtcccttggtggagggggaggaggaggaggcggagaagatctcgtcctgaccggatatcaggtcgacaagaacaaggacgatgagctgaccggattc

SEQ ID NO: 729 - protein, 554 aa, Artificial Sequence
IPGGLSEAKPATPEIQEIVDKVKPQLEEKTGETYGKLEAVQYKTQVVFQYVFSDEDGTNYYIKVRAGDNKYMHLKVFKSLFRWQRGNPEDLVLTGYQVDKNKDDELTGFGGGGSGGGGSGGGGSGGGGSGGGGSGGGGSMIPGGLSEAKPATPEIQEIVDKVKPQLEEKTGETYGKLEAVQYKTQVVFQYVFSDEDGTNYYIKVRAGDNKYMHLKVFKSLFRWQRGNPEDLVLTGYQVDKNKDDELTGFGGGGSGGGGSGGGGSGGGGSGGGGSGGGGSMIPGGLSEAKPATPEIQEIVDKVKPQLEEKTGETYGKLEAVQYKTQVVFQYVFSDEDGTNYYIKVRAGDNKYMHLKVFKSLFRWQRGNPEDLVLTGYQVDKNKDDELTGFGGGGSGGGGSGGGGSGGGGSGGGGSGGGGSMIPRGLSEAKPATPEIQEIVDKVKPQLEEKTGETYGKLEAVQYKTQVLANFFQRRWPGSTNYYIKVRAGDNKYMHLKVFNGPWKFRNTDRGADRVLTGYQVDKNKDDELTGFAAAGEQKLISEEDLGAAHHHHHH

SEQ ID NO: 730 - protein, 557 aa, Artificial Sequence
IPGGLSEAKPATPEIQEIVDKVKPQLEEKTGETYGKLEAVQYKTQVVFQYVFSDEDGTNYYIKVRAGDNKYMHLKVFKSLFRWQRGNPEDLVLTGYQVDKNKDDELTGFAEAAAKEAAAKEAAAKEAAAKEAAAKEAAAKMIPGGLSEAKPATPEIQEIVDKVKPQLEEKTGETYGKLEAVQYKTQVVFQYVFSDEDGTNYYIKVRAGDNKYMHLKVFKSLFRWQRGNPEDLVLTGYQVDKNKDDELTGFAEAAAKEAAAKEAAAKEAAAKEAAAKEAAAKMIPGGLSEAKPATPEIQEIVDKVKPQLEEKTGETYGKLEAVQYKTQVVFQYVFSDEDGTNYYIKVRAGDNKYMHLKVFKSLFRWQRGNPEDLVLTGYQVDKNKDDELTGFAEAAAKEAAAKEAAAKEAAAKEAAAKEAAAKMIPRGLSEAKPATPEIQEIVDKVKPQLEEKTGETYGKLEAVQYKTQVLANFFQRRWPGSTNYYIKVRAGDNKYMHLKVFNGPWKFRNTDRGADRVLTGYQVDKNKDDELTGFAAAGEQKLISEEDLGAAHHHHHH